European Patent Specification EP 4 038 388 B1, published May 27, 2026. Title: Microbial compositions for improving the efficacy of anticancer treatments based on immune checkpoint inhibitors and/or tyrosine kinase inhibitors and markers of responsiveness to such treatments. Applicant: Institut Gustave Roussy. The sequence listing filed with the application follows.

SEQUENCE LISTING (248 sequences)

SEQ ID NO: 1 - DNA, 3225 bp, Alistipes senegalensis
gtgggtgcggctcaggatgtccgagcctatgagggtgcgattacgcttccgacctatctcctggatccggcggaaaaggccccgatctttgaacgggactggtcctaccagcgcgccaaaagaagtgtctatccctatccgctcaatgacaatatgacccgtaagaagaaggatgtgacctacgattgtctctatatggagaacgagtatgtgaagttgtgcgtactcccggagatcggaggccggttgttgtatgccgtcgacaagaccaacggttacgacatcttttaccggaacagcgtggtcaagccggccaatgtgggaatgaccggagcgtggatcagtggtggcgtagagtggaatgccttccaccatcaccgccagaccagccatattccgtgtgactggcggattgtcgataatcgcgacggctcgaagacgatctggcttggcgagactgagtatcgccatcggatgcagtgggcgatcggaatcacgctccgtccggggaaatcctatatggagatcagtggacgtttgatcaattccactcagaataacaattcgatgctttattggtcgaatgtatcgacgctggtcgacgagaattaccagatttgttttccgcagagcacggagttcgtgacgttccattgtaaaaactggtttgcacactggcccgttacgcatgaacccttcaacgatatggacttctacaagaatggtgtggatgcaagctggtggaaaaaccattacatgagcaactcgatgttcatccatgaccagaaggaggattttgtggccggatatgaccacggccgtcatgctggcacgatgctagtcggcaatcacaacatcatcaagggtggcaagttctggctgtggggccccaattccgagtgggacacccggattcttactgatacgtcgggccattattgcgagttgatggtgggggcctactccgacaaccagcctgattacaattggagtttcccctacgagagcaaggaattcacccattactggtatggtatccgggacatgggtggcgtgaaggccggtagccgccacgctgcgttgaacctggaccgcctgtcgtcggaccgggttctggtgggggccaatgctacggaaaaatatgcgaaactgacccttgaactgcgccatggggatgaagttctttacacccgcagcggtgcaatgtctcctgccgaaccgatggttgatacggttgccgtggcaagcggggtggcagatcacgaactgacattggtcctgaaggacgagaatggaaactggatgctctcctatacgccggtccgcaaggatgcgaactctccgctgcccgagatcgttgagccgccgttgctgcctcatcagatcgaaaacacggaggagtgttttctcgtggggcttcggaacctgcagttccacaacccgttcgtcaatccggttgattattttgaggaggtgctccgccgggatccctcggacagccggaccaataccgtgctgggctcctactatcggatgaggggcgaatacgacaaggctgcgaagtatcttcggacggcgattcggcgtctgacgaaggattatacccgcccgaaggatgtcgaggcgctgtataatctgggactgattcttcagatacagggcaagcgcgaggctgcctacgatacattgtatcgggcgacttggaattatacgtataattcggcggccaatacgcaactggcccggatgtattcggaggagaagcgctggggcatggctctggagcggctcgatgaggcaatcgcctacaatggccgtaactatacggcgctgaatctgaaaggttcggtcctgaagagcctgggccgggatgcggaggcgcggcaatgtttcgaccgcgtgcttgccgacgatccgatcaatgcctatgcgctgcatgaaaccgcttcgcacgacgacttccggcgctttatgcgcgaacagccggaatcctacctcgaactggccattcagtattggcacaatggattcacagatacggccgtcaatctgttgaaggagatcgatgcccgcgtgccgtatccgaccgtgaagatgtatctgggctatctgaccggtgaggatcgctattttggcgaggccttgtcgctgccggtcggttactgcgcgccgttccggcttgagacggtccccgttctggagaaggctaagtcggtttgctcggactcttcgctgccctattattacctcggcaatctgtattacaacattcagcccgacaatgccatccgggagtgggaaaagtgtgtggcgatacagccggacaacgatctcgcctggcggaacctcggctgggcccattggctgcatacgaaagattacgccaagtcggccgactgttatcggaaagccatcgagttgaatcccgatgcggcgctttacctggaggagtgcgatcaggtgctggaagccctggggactcccgttcaggaacgctatgatctgctcaagagccaccatgcaacagccgagaaacgctattatcctttggcgcaggaggtcataacgggtacctatgtcggggattacgactatgtgctggatcttctggaccggtgctatttcccgacgcgggaaggggtggccaacttccatgacaactttgtggatgcgttgatcctggccggcgaggagaagatagcggaaggtaaggtcgaacaggccgtgacgctttacaagaaggcgtttacctatccggagaatcatcaggtgttcctcgtggacgagcgggccacgcacgatgcgcagatcaactattgtctcggagaggcttacgccgcgcttggccaggatgccgaggcggaaaagtattggaaactagccgccgaacaggattatgaactgaagggaagcaaggatttccgctactggacgggccttgcgctggagcgtctgggccggaaagcggaggcggaggccatcttctcggcgctggttgccgatggcgaggctgccgttgtcacacagcacgttaatttctacggagctgaaggaactacgggcgtgacggtcgatattatcaactcggcggcctattatacccaggcactcggtcatctgggactcggacatagggggaaggcgaaacgtctctttgccgaagtgcagcgcctgaagccggatcacctctgggcaaacgagttcatgaagcagtttgaaaaatag

SEQ ID NO: 2 - DNA, 3120 bp, Alistipes senegalensis
atgatgaaaggaatcatatacgctgcggccgtgtcgtcgttcgtgctggccgcatgcacctcctgcacgcacgacggcctgcccggcgcggaggttccggacgacggctgcatcgaaatccgtttcgacgccgatattccgccgatgcccgtggtcgccacccgctcggtcgatcccgacggcacgggcgtgcagaacatgacgctcttctgtttcgacagctacggacttttcgtcgcaacgacgcaggcgacgctggcgccgacatcggacgacctgcatgaaggcacgttcacggcccgcgtgccgcagaatacgcgcctgatccatttcctgggcaaccagaacatgctgggatttcaggaacgggatttctacaacaagtcggaggcgcaggtgatggccgcgctcgaaggctcctcgggcatgatgatctactgggcccgtttcgcctgtgccgaggacgatccgcgctccgtcgccgagcagctgaaagcgcagggcgggatagagctcgtccgcaaccatgcgctgatctcggtggacaaccccgcgggcaacggcagtctggacgtgaccgggttcgtcgtctgcaataccagcgcgttcggcaccgtggcgccctatcaccccgagcagggattcgtatggccggggacggagcctttcgtgacgctgccgaaaaatacgtcggtgatgagcgacatcctcgacgtgacgaccgacatgcggcaatatgtcttcgagtgcgagaatacggccgacaaacccgtcagtgtgatcctgcgcggacaccgccccggtgaaaccgaggccgacgacctttattaccgcgtgatgctgatcgatgcgcagggcgaacagctgctcatccgccgcaaccaccattacattctccatatcgagggcgaactttcctacgggcagcgctcgttcggcgaagcgctcgatgctgccgcgacgaacaacgtctggatctcgatccgggacaatatcgacgaggtttcggacggcacctttaccctgaaagtcgatcggacgagctatgtgctggaccagagcaacgaggggcggcagtattcgcttcgctacacgctccggaggaacgacggatcggcggtttcggaggccgacaaaccgtcggtgacgtggctcgacggcaacaacgtggcggggcagaatgtcggcaattcgttcgtcgtcgggagcgacggcgtggggaacggcgaactcaccgtggtgctgcgcgaaatgggcggcagcgaaaagctcgaagggacgctgctggtcaaaaaggggcttttgcagcgcaagatcaagatcatcctcatcaaaacgcagtcgttccggcccgcatgggtggcgtcgcaggtgttcggcacaccctctgccggagagagcggaggcacgtacggcgaacatgtgacgttgatgttcaccgttccggagacatgtccggcggagctgtttccgctgcgggtgctgatcggcgtcgaggatctcgatgtccgcgcggcggccggcatgtcgctgccggtgatccgccgcggcgaggatggcttcggagagaatatcctcgacgaaaagggggagccgatcgaatacaagttcgtctatacggccgtacagccgggcgtgcagcgggtgtatttccgcacgatcctgccgcagagcggttccggagcgaagaccaaggtttcggtcgaagccggatacttcgccacgcaggagaaggaggtgacctataccggcctccgatatgtgatcgaggtcgccggattgaacgaatatacggccagacccgacgacgatttcgccgacgacgagaagatcttctaccggctggtgccgcagaagaagggcgctttcgtccagttcaccatgcatctgcacgataattcagcggaaacatcgtccggcggcgattacggcgaattcgtcaacgccacggccgacgacgagtttctgatctattcgcagtatctcgaccacattcccgacggagaggagcccgacggcgttacgttcgactgcacgttctcgcccgtcaacgaggatatgtggacggagaatggccgcatgtatctcttttacccgcgcgcgggcggcgatacgccgcagtcggggacgggcatctattcgatttacctgcgaaccaaccgtccgcagagtgccgaggtcgtccgcatagcctccaatatttcgggcgagaagtcgttgaaagatgtcgcccgggactatgccggccgcggttatcgttcgacttcgttcgagctggccaactacaaccccttccgttttgcggcacgcatagacggtgcgggcggggatgcctccggaagcgacgcggagccggtgacggaattgacgtggaattatgagaatccggccgaaacgaacatcgacatcgagttcgacgtgaccagtttccggggttcggacgaccggtcggccgatcctttcggcgagacgttcgaggtctatatcgacgcgccgatgctgaccgtggacgaatcgcggctggccgagtgcaatctgacgcccgataaactcaaagcggaccctgaggtcgaggggcgtttcgtttatacggtcgatgcctcgcgcgaggaggagcgcaaattcggtgtcgcagacgcgctgatccccgatacgacgccggccgctgccggaagccctgcgccttcacagtcgggagagcgcaagcggctgccgttcaagacgaactgtgtggtgagcgccggcgacatcaccctttcgtcgaacgaggagaaagtcgtcttcttccggaagaccttccgtgtggcgaacgagtcggtcacggggcggatcacctacgatccgggcaccggggcgattcccgtgccgcgcaatgcgttcgtgtcgttcatacagtcgggaacggggagccgcatcgggtcgatgaccgtgacggcggacggccgctacgagttgcggttgcgcaaggagtatgaccccgggtggttcgatcgcatcgaactccgctatacgaaggacggcgcggtttaccggaaccggatcgacgagaacaatccgctgacgctggcccgtctggtgcagtcgcccgatatagtattggtgaatgtggccgctgattga

SEQ ID NO: 3 - DNA, 3063 bp, Alistipes senegalensis
atggcacagaatgaaatacataagatcataacgatagagttcaaaaattcggaacttatcgacaaaatgcgagaggcgcagaatgctataaaggcactcaataccgaaaccaaatatctgaaagaggacctgaatgagtatcgccagcagctcaaatccggagctatctcgcaagaccagtttgatcggatgatgattaagaccaagaacgagataatcaaaaacgatcaggctgtaattaaatacaaatcggatattaaagcgtacactcgtgaacttcaatccaatatccgccaagataaggagaaggtcggttccctgaatcaactgcggtcgtccgtaaagtctttgactgcggaatacaataatttgagcgccgcagagcgaggaggagtccgggggaaagaaatcgtgcggcagattcagaaaacaacggccgagatcggcaggcaggaaaatgcactccgtaattatcatatcggcgtcggtaattacgccggaggcattcagaaagcgtttgttaagatcggggcggcgtggatggctattcgctcggcgtttagcctctttcggaatagctttaacacgattaaagatttcgagcaggccaatgctaatctcggtaccatcttgggtgctactaacgaggagatggataaactacgagaatcagcacttgaactggggcggacaactgaatacacggcctcacaagttacacagttgcaaactgaattggcaaaattgggattcggtccgaaatccattcaggcgatgcaacaaccgattttgaatttcgcaacagccgtaggtgcaaaactttcggatgccgcaaaattggccggtgcgactttgcgaatttttggattgagtgcccatcaaaccgaagatgccttagatgtcctcgctttgtctactaataaatcggccctttcgtttgaatacttgaatacggcgttatcaatcgttggtcctgttgccaagacgttcggattctccgtgcgtgatgtaacggcccttctcgggtcattggcaaatagtggattcgatgcttccagtgcagcgacagcaaccagaaatattttattaaatcttgctgatattaatggcaaactggcgaagtctctcaacggtccggttaagtcattgccggagttgatcgacggattaaaaaagctacgtgcacggggcattgacctcgccggaacacttgaactaaccgataaacggagcgttgcggcatttaatactttcttaaatggtgctgatgatgtgaaggaattacatgatgcgttgcaagatgtagatggagcagctaaaagcattgccgaagaacgattaaatactgttgagggatcaatcaaactattgcaaagcgcctgggaaggacttgtgctgtcattttacaatagcaaaggcacgattaagtccgttattgatatactgacgaatgggatagaggggatcagcaatttgctaaatccggatgcccaaaagaacaaacaaaaaaatcttttcctcgatgaatttatgaatgtatattctgccgaaggagaagatgcgctgaatcggaatattcaaatcgggttgaaatattggggcgatcaatatgaagaggcccggaaacgctatgccggaagcggaggtctttttggtaaatccgaatttgatattaccgaaacgatgtataaggcatttatcgctgctggaaatgaagctctcgacaatgtgcagaaactcaaaaaagaacaagaaggtttagcggcacagacagaagataatggtgagaaaatcactacgataactgaaaaagagttgaaagcacgccagcaagccgccaagacacagctcgatttagagaagcaattatcaaaatccattcttgaacttagacaagcgagccttgaaaaagacctggaactttcccggcttcgcttttcgtgggaacgccaagagctggaaaacaaactcaaatacgacaaaacgctgactgcggaatcccgggaggctataaaccagctgatcctgaatatggaggaacgcaggtataaggaggaatccgaaatccgccagcgttggagcgataaggagttcgaggaagaagcccgcaatgcggagaacaggatcaagatgcggatcaaagtccaggaagagatggacaaactatctcttgcgcaagtaaaaaacaggaactatgcaggattgatcggggacgacaaggatgcacggattaaagcgcagcaggccgttgcaaatgaagaattgcgtattgctcaaagtaaatatgacgctatttcacaaatggatgaggagcaatggagtgcgcaatacggttctattcaagcctatgagatggcccgactggatgcagaaaacaatgtgcaagatgcaattaagaaaacgaccgacctgtctatcgcctcgcaaaatcaggcaataaaagtgcaactggacgaactggcggccgcctcctcgttagttgggagtctaagaggtttattcggggcgttgggcgatgatcttgaggcattcgccattgcagagcaggcattggccgtggcgcaaatcatcatcgacgctcaaaaagcaacaatggaagcgatggttgcatcattccaactcggacctattgcgggacctatatggtttgcaacacagaaaggaattataacagcgcaggcggcaatcgcatcggcgacaacgcttgcacaagccatcccttcgttcttctcggaaggcggccttgtcacgggcccgggcaccggaacttcggacagcatccccgcaatgttatccaacggcgaagctgtgatgaccgcccaggctgtcaacgactggggcgcaatgctctcggccatgaacgtggcaagcggcggaaacgccatccaagtatcgaatcttccccagcgcaacgacggaatgaaggggatggagcgcatgatggaacgggccctgatgaatatgccggcgcccattgtttcggtggttgacatcaacaaagggcagaagcgggtcaaggttcaaaacagcctcggaaaattaggtcgaaaaaaatacgaataa

SEQ ID NO: 4 - DNA, 3060 bp, Alistipes senegalensis
atgttcgttaccgcagcggcccagcaaaaccgccaggacgcggtcaaaggcactgtcctcgacgacaaacaagcgcccgccgtaggagcgaccatcgtggtaaaaggtacgaaccggggaacgatcgccgacgggcaaggaaaattctcgattgaagcctcctcacgagataccctgcaaatcagtctgatcggataccttccccaggagataccggtaggcagccaggccgaagtgaccgtctggctgaaagagaacctgctttcaatcgaagacgtggtcgtggtcggcttcggtgtccagcgaaaagagaccgtaaccggtgccatcaacagcatcggctccaaagagatcctgcgttcgccgacagccaacgtcactaacgcgctggcaggcaagatggccggtctgaccgccgtacagcgcggaggagagccaggcaaggacggagccacattcaaaatccgcggcatcggaacgctgaacgaaggcagcgaatccgccccgcttatcctgatcgacggcatcgaacgcacctccctggacgtaatcgacccgaacgagatcgaaaccatcaatatcctgaaagacgcttccgccaccgcggtatatggagtccggggagcgaacggagtcattctcgtcacgaccaagacaggccagcccggacgcgcccaggtcacgctgacatccaatttcggatggcagtcctataccatgatgcccgaactggtcaacgcttacgaatgggcgaccctttacaacgaagggctcgcacacgaaaacagcaccaaggcgccgttcccgcaggaagcgctcgatgcctggaagaaccacacgaacccggtactctatccggacgtagactgggtggacaaactgctccgcaaatcggcccctcagcaacagtataacgtcaacgtaagcggcggaagcgaccggaccaaatatttcgtctccttcggaatgctccatcaagaaggcatttacaaggagtacgacatcgacggcgtggacttctccgtcaatccggattaccgcagattcaacctgcgcgccaatctggacatcgacgtgatgaagggcatgacgctcggactccggctcggtaccatcttcacggacggcaactacccgaacgcatccacttccaatattttcgactatctgttgcgcacggtcccgggtggaggtccgggtctgatcaacggcaagctcgttacgggttattcgggcgacgatccgctcgaaaactacgagcgcagagtatccaatccgattttcgacatcctcgaacaggggtatcaggaatacaacaccagtacctacaacctgagcgcagacctgaactacgacctcggattcctcgtcaaagggctgtcggtacggggcaaagtcgcctacgacgactacggcacccaccgggtagcatacacgacgggaagcattccgcaatacacggtcgtggtggacaacgactacgaagacggataccgcctcgtcaaggcttccgacgaaacggccttcggcgccaaggagtcttacagcacccgttaccgtaatgtatacctggaaggcggcatcagttatgccggccagttcggccgccacagcgtcaccgccctggccctctacaaccagcgggtacaagacaatccctcgttccaatacgacctgcccaaaggcctgctgggattcgtaggacgcatcacctacaatttcgacaaccgctatctggccgaattcaacgccggctataacggttcggaaaacttcgccgaaggcaaacgattcggcttcttccccgcattctccctgggctggattctgaccgaagagaaattcataccccgcaacaaatttctgacctacgccaaaatccgcgggtcatacggagaagtcggaaacgaccaaatcggcggcgaccgctatctctacctgcctccgacattcgtatacggttcgaacggctacaacttcggaacattcgggcagaattcgcagtactatcccgcctccgccgagggaagcgtcggcaactccgacgtgacctgggaaagggccaagaaagccaatatcggactcgacctgaaaatgttcgacaaccagttgagtttcacgggagactatttctgggaaaaacgcgacaacatcctctgggattacggaaccgtcccctcgatcgtgggtacgactctttcggccgcgaacctgggccgggtggacaacaaaggtttcgaactcgaactgggctggaattccaaagtccggaacttcgagtattggatttccggcgtattctcctatgccaaaaacaagatcgtctacatggacgaagccaagcaagcctatccctatctggcgcaaacgggttactccgtgggccagtacaaaggctacatcaacgaagggttcatcaacacggatgccgacctcgaaaaccagcccgcacacggctggggcggcgaccggtgggccaaaggcgagctgaatttcatcgacatcaacggcgacggcatcgtcgatacgaacgaccgtgtaacaatcgggtacggctcctatcccgaaatcacgttcggcgtgaacctcggattccaatggaaagggttcgaagtcagcgccttgttacaaggagccgcaaacgtctcgctctacctgaaacagagcgccgtctgcccgctgtattacacccggagcgcccagaaatggcacatgggccgctggaccgaagagcggtatctcgccggagagaagatcacctatccgcgcattctgtccgacaacatttcgtctccctcgttcctcgaccagaatccgctctctacgttctggctctacgacgcttcctacctgcgcctgcgcaacctggaaatcgcctacacgctgaaatcgaaaacgctcaaaaactcgggcatctcctccatccggctctatgtcagcggcaccaacctgttcacaatcacaggcatggataatttcgacccggaagcgccctccggcatcggaagtttctacccgatgcagaaagtctataatgtaggtgtcaaacttgttttctaa

SEQ ID NO: 5 - DNA, 2937 bp, Alistipes senegalensis
atgaacaaagtaagcaaagacgacgtattgcaggccaccgaaggcggcaagacggttatcctcgattattaccccgcgtcccgggacggattcgagcggcgccggaatttcaggctccggccggacgaccggaacccttcgtgcaccgtgttcaaccgcgacggcatctggttcctgcaagacaagggcggcggcgataccaaggcccgcacggccatctcgatcgtcatggaggaagagcgcctaacatacccgcaggcgatcgagttcatcgcgtcgaaatacgctcctcacctgcttgccggggcctcggcggtttccgtacagccggagcccgggcgggccgaaacggccccgcaggacgccatgaccgtacaacgccgcaagggtggaaaattctccaaatgggaactcgatctgctcggacatcagatcacgcaggaggtgtgcaacgaactccgcctggtaccgctggactcctacatcacccgcaaaaacgaaaaggggaagagctggaagatctcggccacggagaactatccgatcttctactacgattacgggacatggggacggctctaccagccgctgtcggcccagctccgtttcatgttcgtcggagagaagcccgccgacttcattttcggcgactcatggttcctcaaagcgttcgatggttccaagcgtcggacgcccgacatctcggatgtcggggaagaggaggaagagacgccggaacagggcgacgacgacgatccggaagatgagggcgatatggactccgcaaacgcctcgccccggcaggagcaatgcgacgcaatcatcctctgttcgggaggttccgacgccctgaatgtccggaacgcctgcatcaataccggccgggccggatggcatgtcgcatggctgaactccgaaacggccgaccttccccgggccgacatgttccacctccggcagatagccaaagaggtctacattctctacgatcaggacagcacgggagtcgccaacgccttccggcacgccatgaaatacctcgacctccggatcatccgcctcccggacgacctcaaacgcttcaagacccgcaaaggaggagcctgcaaggatgccaaggacctcttcatgcactaccgaaagcctgcggcacaagacccctacaaaatcttcagcaacctgctccgggtatccggatcgctgaaattctgggtgcgtttcaaagaccgccgcggcaaggagtgtttcgacatcaacaacgagcagctctactccttcctgcaagcgagcggatactatcgcatcgaatcctcggccacgagcaagggattcaccttctgctacatccgggacaacatcgtccgcctgatcgacgagcaggccatcgcgtcggaatgcaatgccgagttgatccgctatctctatgctcatcccgagtactactcgcaggcgctggccaacgccatccaccgaagcaaccaggtgaagctcggatcgctggagaagctgcggatgatcgcaccgaatttccgttatttcggggcgaatttcgaccatgtgctattcaagaacaagatcatccgcatcgaccgggacggcctgcacgaaattcgtccgcaggactggccctacttcgagtacagcaacaagattctcgaccacgaaatacaactggacaggaacggtgtgcttccgttcgacatcgtggaaacgccggccgcccttgcgatacggaaagaaatgcagggccttaatccccggtcccctatttataagcaaatgcaagctgcgcttgacacgttgacagggacggcgaggttcaagctgcgcatcaaccgccccgatttctctttcctgcggtacatctacaacaccgggcgcgtgcattggcgcaaggaggagatgggacagcccctcaccgacgaagagcgcgccgagcaggatctgcacttcatgtcaaaggtcatggcactcggatacctgctgaccaaatacaaatcggcagccgaggcaaaggcggtctacgccatggagacggagatctccgacgagggccagcacaagggaggaaccggaaagtcgctcttcctgggcagcatcgagcagatgcgcaaccagcttttcatcaatgggcaggagctccgccccgacaagatggagttcctattccagggggttgtcaagggggtgacggacacgatctacttcgacgacgtgaacaagtcgatcgacctccaccgcttcatgccggcgatcaccaacaagatcaccatcaacgccaagtatgccgcggccgtaacgctcgaatacgccgagtccccgaaaatatccttttcgagcaaccatgccatccgggagttcgacaactccctccggcgacggatatggttcacggcattctccgactactaccactcggcagacccggccgccaagctttcgctgcggaacccggccacggagttcgggaagaatctgatccaggactacacgcccgaggagatgaacgaattttacattttcatgcttacatgtatgcacgtatacatcaagcatcaggtcgcgctccagccgccgatgcacgacatcgagcagcgcaacatccagcgtcagatcggcgacgacttcatctactgggccgaagagtatttcgccgcagacggacgccgagacaccttcctcaataaaaccgaggtattcgaggcatacaaggaatcgctccccaagcgggcacaggacagtgtgaagatgcagaccttcaaaggccgcctcatccagttctgcgagtacaagggatgggagttcaaccccgacgagatgctgcaaaccgaatccgaccggaagcggaacgagatccaccgaaaagagcagggtgtcgatgtctactacttctacattcggacggccgaagaggacggggaggagaagattttttag

SEQ ID NO: 6 - DNA, 2754 bp, Alistipes senegalensis
ttgctgtttgcggggtgtctgttatctgcctccgcccggcagaacgaaggttttccggtcgtaggtgctcccgataccataagtctcggctacgggatcggtgtcgaccgggatcggagcgcctggacacaggcgggagtgggccgcgaagtgctggacaatgcgccgcagattgatgcggccaaagccctttacggacgaatcgccggactgaatgtttatcagggagtcggcacgacggccgataacatcgcttcgctgtcgattcacggacaggctccgctggtacttgtcgatggtttcccgcgggatcttaagaatcttacggtacaggagatcgaatcggtcgtcgtgctgaaggacgccgcagcggttgcactctacggtgtgcgcggtgcgaatggggtcgtgatggtctccacgcggcggggaacgcccggcaagctgaaagtgggtgtcggctatcagtacggcgtcagcacgcaatttcgcgcaccggaatttgccgatgcctttacctatgcccgttcgctcaacgaggcgcttacgaatgacggcctttcgcttcgttacaatgcctacgaactgaatgcgttccgcagcggaaaacatccgtcgtattatccgaatgttgattggtggaatgaagtctacaacaccacagcgtcgaatcatcgcctcaatcttacattcgatggagggtcgcgcaagtttcgttattatacggccgtggattatatgcacgaccggggcttttttcgcagcaatgaaaacgaatcccggtacaaaaccgatccgacggatgttcgcttgaacattcgggccaacatcgatgtggacataacccgttcgacgcggatgcggctgaacgtgatgggcaagatcgctgagacaaaccgtgccaattacggagatatttacaacatcctttataacacgccttcggctgcttttcccatacgatacgatgacgacggcctttacggcggtacgagtatttacggggccaataatccggtagctttgttgatggacagcggcaattaccggcagaccatcggaatgcttttgggggatttgtcgttacggcagaatcttgatgcgctgacccccggcctctcggcagaggtgtcggtggctttcgacaatgtcggctccatgttcgatcaggcgacgaagacttatcgttataaggatgcgcaggcctccgtttctacggacggaacgctgatcacccatccggccgtttacggcaaggattcggaagttgtcggccacagtcagaatttctactcgttatacatgcggtccgatttgcaggctaaaatcggttatgaccgttgttggagccaacatcatgtgcaggcggccgtgatttacgatcagcaggcctacacggccaacggtcggaataactcggttcgtcggcaatcggttctcgctacagtcggctacacgttcgacaatcgctatacggtgaatgtcgtcggcaattattcgggttcggcctatctgcccgagggcgatgcgttccacttttatccggcggtaaacgccgcctgggtcctttccgaagaacccttcctgcgaaacgcaaagcagctcgatctgctcaaattatccgcttcttacggcatttcggggtgggacgggaatctgtcgcacgaactgtggcgtcagtcgttcgggaatacgaatgcgcacggttactatttttccaacaacgtcgcggcctattccggtttggcagaagggaatctcgcggccgaagggcttgtccccgaggagtcccgccgggtaaccgtggggctcgatctgcgttcgttcggtaatcgtttcacggcttccgtcgagggatttttcgagcggcgcagccatatcctgatctcttccggggccaccgtgtcgggtatcatcggcatcggcgtggggctgcaaccggccggcgagcatgagtaccggggattcgacgcctcgattgcctggaacgaccgccgcaaggatttctcctacggagtttacgccaacgcctcctatctggacagcgaggtgatcgtcgacggtcaggagtatcagccctatgattatctctaccaccggggcaaccgggtggggcaaagttacgggctggaggtcgtcggcattttccaaagccagatggagatcaacgaaagtcccgtacagacgttctcgacggtgcgtcccggcgatttcaaataccgtgaccagaacggcgacaaccggatcgacgatctggatatggtccggatgcacggatcgagtgttccccgtttctatttcggcttcgggttccatgccggttacaaagggatcgaactgtctgccgattttcagggcatgacggggcgcacggtcaatctgctcgactgtccgctctacaaaccgctgatcggcaacggtaacatttcgcaaacgctgctcgatcacgagatcccgtggtcgcccgaacgtgcttcggaggcgaccatgccgcgactgacaaccctgtcgaatgcgaacaactaccggaacaattcgtattggtatcgggacggttccttcatcaaactgcgtaacctgaccgttgcctatacgctgcccaaacggattcttcgcttcgcggatatgaagatttatctgcaaggtacgaacctcttcagtctggacaatctgaaaaccgttgatcccgaacagttgggggctgcgtatccttcggtgcggtcgtactgggcaggcgtgaagttcaatttttaa

SEQ ID NO: 7 - DNA, 2547 bp, Alistipes senegalensis
gtgcttcccggcagcggcatccgattttacggtgcgtactgtcgggactttacccccccctccattccagacggtgctaaaaatcccggcgtggcgggcgctttcatcggcgggatcggcgaccggatcgttttggccggcggctcgaacttcgctcagggcgcgccctggaacggcgatgcgaagcaattcgaagatgcgatttacttgcttactccctccggaggtacttataaatgcgaattggttgccgatgcgaaattgcccgcaggcattgcccacggttgtgccgcggtggctggccgtagcctctactgttttggtgggctgactgccgaaggggagtcgcgcgcggtctatgtgctgacgcttgccggaaattcggtgtgtgtcgctgcggcgggagtgttgccggaggatttccgacctgcggctgcgctggcttataaggatgagatttacattcatggtgtgaaagacggtgccaacgctttctggcggttctcgcccgtgagcgggaaatggaccgaactcgcggcgtgtcccggtgcggttcgttcggcaggtcctgcttttgtggaccagcacaacggacgcgaaaatgccatgtacttgatcggcggtcgtcacgaaaagggcggggaattgcagttgtattccgacgtttgggagtatttgccggtgcatgacaggtggcaggccaagggtgacgtgacgatcggcggcaagccggtggtggtgatgtatgccgctgcggtgccttacggatcgggtcatgtgctggtgttcggcggtgacgacggccgggagttgcagcaccgtgctgcgcttgaacgggcgatcggcggggcggcgacgtctcaggaagcggatagtctgcgcggacagctgcgtgaagcgttcatggggcatgaagggttttcgaaagaattgctggcttatcacgccattaccaatacatgggtgtcgctcggtgaggctcaaacgggctttccggccgtatcgacggctgtgattgcgggcggcggaatcgttattccgtcgggcgagatacgtcccggcgtgcgtacgcccgacgtacagatcgtgacgattcacgagccggtggagttcggctggggcaactattccgtaattattgcctatctgctggttatgatgggtatcggcgtctatttcgtccgcaagaacaatacgactgaccagttcttcaagggcggagcgaaaataccttggtgggcggctggtatcagcatctttgcgacggcacttagtgcgatcactttcatctcgatccctgcgaaggcctacggcgccgactggggcatgttcatgttcaacatgaccatcctgatgatcgtgccgatcgtcatccactactatctgcctttctttcgtaaactcaacgtggcttcggcctatcagtatctggagcagcggttcagttcgtcggtacgctatctggcttcggtgttcttttgtttcttcatgtttgcccgaatagctatcgtgctcttcctgccgtcgctggcgctgaatgcggtgactggaattgacgtttatgtctgcatcttgctgatggggctggtgaccatcgcttattgtacgatgggaggcatcgaagcagttgtctgggccgatgttgtgcagagtgtgattctcgtaggcggtgcgcttgtgtcgcttgtattcctgatcagtggcatagagggcggattctcaggcatgatcgatgttgccatgaccgacgacaagttcaatattctgaacttcgctttcgacttgacgcagccggtcttttgggtgacgttggtgggtggtctggctaatcagctgttggcctacacaagcgatcaatcggtgatccagcgctacattacggtcaaggatacggccggaacgaaaaaggggttgtggctcaacggattcctgagtatcccgattgccgtgatcttcttcatgatcggtacggcgctttatgttttcttcaagcagcagcccgaattgctaagcattgggatgtccaatacggactcgattttcccgcatttcatcatgtgccgtctgccggtaggtattgcggggctgctgattgctgcgatcttctcggcagctatgtccaccctttcggctaatatcaactctacagcgacggtgctgacagaggatttctaccgccgcttccgaaaaggtgcgacggacaaacaggcgatgggcttcgctcgattgtcgggtatcgtcgtgggtggcttggggttgctgatggccatcctgctcgctacgttcgacattgcgtcgttgtgggatcagttcaacttttttcttggcctgctgaccagcggtttgggcggcttgttcatgatgggtatcttcaccgagcggatcggcacgcggagcgcctttgctggatttatcggcagtatcgtcatactgctgatcatcaatagctattcgactgtttcgttcctgctctacggatttatcgggttggcttcgtgtttcctgatcggttatctttcaagttttgttttcgggcgcggcaaataa

SEQ ID NO: 8 - DNA, 2475 bp, Alistipes senegalensis
atgtttcatatgattgtaaggaaaattttcagtttattgtccctcgtcctctcatgcgcagcgatggggcagacgattacacccgaaatagaaaagcgtgcccttgagttggttgcgcaaatgacactcgaagaaaaacttgcctatatcggtggctacaacggtttttttattcggcccattccccggttggggattccggagatacgtatggccgatggcccccaaggggttcgcaacgacactcacagtacgatgtatccatgcggtatcgcggctgccgcgacatggaaccgggaattggcccggacttacggccattcactcggtcaggacgcccgggcacggggtgtccatatcatgcttggccccggggtgaatatctatcgctcgccgctttgtggacgcaattacgaatattatggcgaggatccctttctgacgtccgaaacggccgtggcgtatatcgaaggtatgcaggcggccggtgtaatggcgacgatcaagcatttttgcggcaataatcaggagtggaaccgtcataacgtttcttccgatattgatgagcggacgcttcacgaaatctacctgccggcgtttcgcaaagctgtacagaaagcccgagtcggcgctgtgatgtcgagctataatccggttaacagcatacataccaccgaaagccgcgaactgattatcggcgtactgcgggaaaagtggaattttaagggtatctacatgtccgactggactgcgacctattctactgtcggagcagccaataacggtttggaccttgagatgtcgtggggccagttcatgaatccggataaattgcgtacggccttggcgacgggaactgtgacggaggagacgatcgatgaaaaatgccgtcatatcgtgcagacgctcatagctttcgggttcttcgatcgggagcagcgggattggtcgatccccgaaaaaaatcccgtctcttcggaaacggcgctcgccgtggcgcgcgaagccgtagtattgcttaaaaacgatggcgatatgctgcctttctctcgaaagatacggaatgtggttgtgatggggcccaatgcgactaatatccctacgggcggaggcagcggatttgttatgccctttgaaaccgtatctgtggcagaggggattcgcaatgcagataagcgcatccgcatgaaggtattggcacctgaactgtctgtggatttaacggcttgggggtgtttctttacgccggatggcaaacccggattgcgaggggaatttttcgccaatccgaaacttgaagggaacgccgtcggaacggtcgatgccactgcaatcgactttttctggcagaatgctccgatggagggtgtgcctgctacgcagttctcggcacgttggacgggaacgttcattccgtcggttacggggcaggcagtctttcagatcagcggtgatgacggttaccgactttatatcgacgatcgggagattattgccgattggtacgaccattttatcacaatgaagcgcgcatcggtggatgtcgaggcgggcaaaagctacaaggtgcgtttggaatattacaatgcctgggattccgggactctccggatgtgcagcgcttgtcattcgcctattttaccgcagcaggagatcgaatcggctgatgccgtcatctattgtgccggcttcgactcttcgaccgaaggcgagaattgcgatcgtccgttctcgctgccgcaacagcagttgaaggagattgccgaagcggcgatgctcaatcctaatctgattgtggtggtcaatgccggcggcggggttgatttcacaccaatagtcgataaggcgcgtgccgtgcttatggcctggtatccgggacaagaaggcggtcgtgcgattgccgagatcctgaccggtcggatcaatcccagcgggcgtcttccgattacggtagagcgtcgggcggaggataatccgacgtttgacagctatcgtgcgaacgttgctcaggtttacaacagcccgctacgagtcagttatgacgaaggcgttttcgttggatacagaggatacgatcgggcgggcaccgaaccgatgtacccgttcggctacggactctcctatacgactttcgattatgcgaatctgaagatggaacgactggatgacgggaatgtcgtggtatcattcgaggtgacgaatactggtcgtttcgctggttccgaggtggcgcaactttatgttggtgatgaggtggccagtgttcctcgccctgaaaaagagttgaagggatatgaaaaggtgcggctcgaacccggtgaaacgaaaagtgtggagattcgtctgtcaccggacgcctttgctttttacgatatgaaccgccatgatttcgtggtcgaaccgggtgatttcacgatttcggtcggcgcttcatcgcgggatattcgattgagcgaaaagattcggatcgactga

SEQ ID NO: 9 - DNA, 2412 bp, Alistipes senegalensis
atgcgatggatcgtgacgctgatgatgctgttgtcggtgctgtgcgacacgacgcccgcggcggcccgcaagcggcgcgcgacggctcccgaaccgcgtaagacggcttacgaacggcttttcgccggtaagaatccccgaacggtgcagggattgttcaccctgcatctgctcgacggggatgtctatttcgaggtgcccgattcgatgctcggacgtgacctgctgctgggggttacggtgctgtcggtcagcgacggcgaggagtcgtcggtcgggatgcagccttcgcgtccgcgccatgtcgttttccagcgaaccgattcgcttttgcagattgccgcactcgacagccgttcgcgcagcgacgatccggcgatcgggcgggcgctggccgcgagccggcagccctccgtgatcgcgtcgtttcccatcgaggcggttacgcccgacagcagcggcgtcgtggtgcgtgcgacatcgttcttccggaacggcgagagttacctttcgcccaaggacccgaagagttacagcagccgcgacggattcgtcctgcggagttacgaataccgttctgaagcctcctggatacgcgatatagcggcctttagcgacaatgtctcggtggtgagcgagctctcctacgaagtctcgtcctacgctttcggcgtgatttctcggggcgatcccgagctcttcacggcggccgtgcggacatcgttcctgctgctgcccgaaccgatgacgacggtccgtgaagcggatctgcgcgtgggcacctccacgtcgcgttacgtcgaatacagcgccgaccggcagggcgccgaagtccgttattacgcctcccggtggcgggtggatgccgggcgtcccatcgtcttctatctcgacgagcgttttccggcggcgtggaaaccctatatcgaacggggcatactgctctggaacgatgccttcgagcggatcggtcttccgcgggccatcgaggtgcggcgtgtctcggcggaggggctgcccgacgtgaacgacattcgctattcggccgtacgctacgttccttcgccggcccgcgatctgcggttcaacgcctggaccgatccgcggacgggagagattctgagcgccaacatctacatcagccataatatcgggccgcagatccagaccgaacggcttcttcagacgggagccgccgatccccgggcgcggcggctggaactcgacgaggcgcttttcggcgagagcctgtcggcgaaggtggcccgttatacgggtttttgcctggggctgctgcctaacatgggggcttcgcagacagtgccgctcgattcgctgcgcagcgcgcattatacggccgcgaacggactttcggcctcgattctcgacgagctgccgttgaactatgcggcgcgtcccgaagatttccggaacggtgtgaaactctgtcagacatcgctggggccgtacgattaccgcgccgtcgagtggctttacggcgacggggcggtgagcgacgatccgtcgtgccgttttctgcgggaacagccggaaaaattcgcgctcgatccccgggcccgggcctcggatctgggcgacgatccgctgcgggcggccgatgccgggctggcgaatcttgccgttgttctgcgccatgtctcggagtggatcgacgacgaggatgtcgattatgcctaccgttcggccttccccgagtcggtttcgttctattgcaatgcgttgttcggctccgtgatcgcccgcttgggcggagtgcggatcaacgaacgctatgccggagatgcgggccggagtttcgagccgcttcccgccgggacgcagcgggaggcgatgcggtggctgctgtcgcggctcgacgatctgcaatggctcgacagccgttcgctgatcgtgggggaggggctcaaccccggaatcgcggatttcatccgtacggagaccttcgaccggattctgggaagcctggaccgcattgcgctctgcgcttcgttgaccgacggggaggcttacacgcgcgcggaggcgctggacgacctctcggcctatctttgggacaatgcggacccggcggacgaactcgtcaagcagccgttgcaactgcgattcctgaatcggttgctggcccttgccgaacaggctgcgggccggaaatcgaagctgcgttcggactatttcgccgaggctgtgacggcggagaattccgcaggcttcgctccgcttgccggggtttcctacctcacgcggcccgaggacggccatctgctctacggcgtgctgctcgactgccgggatcggattgcggccgcccggaatcggagcgcctcgccgcagatgcggggacactacgcattgttgctgcgtcgggtgacgcactttcttgaaaacaagtga

SEQ ID NO: 10 - DNA, 2214 bp, Alistipes senegalensis
atgctttcggcggcagtgctcttcctcgccgcctgtgaatcgacggatgagaaggacggcgggagatattcgctcggaacgacctgccggattctcgaaagcagaggcaatttcaccagcttcattaaggcgctcgaccgcagcggttaccgcaggcttgtggacggcggcggactcgtgacggtttttgcacccgacgacgatgctttcgacagttatctcgaaggcaggtacggaacgtcggacgtagatcaggttcccgttgaggagctcacgctgctcgtaggctgccacatgatccagttcgcctacacgacggaggatttcctctctttctcgatgacctcttcggaggacgggacggatgcgggcgacggctcctgttacaagtacaagacgtatgggcgtgccgccatcgaggattataccgacccggtgacccggcggaaggtgaagctcttctcccgggagaagtacatgcccgtcttctcgacccggatgttcgccaagcgggggatttccgatgcggagggcgactaccgcaaattctttcccgacgtgaactggcagggttcggacgaccgcctttatgcgggcaacgccgccgtgatcgaaagcggcattcctaccgacaacggttatctctacatcgtcgataaggtgatggagccttcgcgcaccatatataaagagttgtcggacaattcggggaccggagccggttattcgctctgcaagggccttttcgaccggatcagcctttacaagtacgacgcgtccgtgtcgaagaactacgctgcgtcgtcgggcgactcgcttttctatttctaccactggaaagagcccagccgtacggccgagattccggaaatcgccagcgaatggacctatcacgacgagagcggcgtggtcttcgaccgtccgctgcgttattcggtcaactgtttcctgccggacgacgaggtgctggaagagtatatgaaggagtatttcagcgagtacggcacgcagacctcggacgatttcctgagcctgattcccaaaaacgccatataccatttcctgcgggcccatgtctacgggagccaggatctgatcctgccttcggagctcgaccggcgtccggtggccggcgtgaacggcgagcagttccgtgtttcgtcgtcggagctgcgcagcgtgacctactgctcgaacggcgtcatttacgggatgaacaaagtgttcgaaccggctgtcttcacctacctgacggccccgttgttccgctatcctcagttttcgttctacgcgcgggctttcaacacgaagaacatgtacaatcagacggtcgatcccaacaaccgcttcacgctcttcatccagaacgatcaggacctggccacggccggttattcgtcgagcgagggaaccgggacgaacggcgactatgcgttccgcagcaggtccggtgcgatgaacgccaaccaggtgtcgaatctggtgatgtcccagttcgtctacggaactcttcccgagctggcggaaaccgacgacctgcgttatttcatcgccaaggacgagaagacctatttttatataaaggataaggcgctttacgactattcgggccgggagctggtcgtcaaggcgacgttcgataccgaaaacggaacggtctaccagatcgaccgggtgattcccgcccgcgtcggagcctactccgagaccggtaagctgcccgaatacgagcagttcaaggccctgatgatcacggcgggcctgggcaacaacagcggcggtctggtcaccccgatcgccgacggactggtcttcttcccgaccaacgaggcggttatcgccgccaaggcggcgggaatgatccccgaggtggtcgatggcgacgtgacggagctgcggaaatatctccagtactatttcgtgccgctgaagaaaaacaagctcaactattacctgctgccgggtctcggtcccgagggagcgacggaggagccctattcgggaacctacgtcacgctgtcggagtaccagaacgaggtcgatgccaagacgatggctatcgcgtggaatcccgagaatcccgagtcgctgacgattaccgacatggccggcaactccatcacgacggaacccggggtgatcaatctgcgcaccaactgtgcgacctattccatcaccacctgcttcgattatcgcacgatgtacggaaactaa

SEQ ID NO: 11 - DNA, 2034 bp, Alistipes senegalensis
atgagtgcgttacgctggtttttggacgaaccgaatcgttttacagcccaagacttcaccgtaactctatggaagagtataaatgatataggggataaatggttagatgtgtccaatgatgaagaaatacacattgaggattggtttaatatcgtgccatctatggatgtgtgggtaaagatagattcatcggaaaaatatcgcgtaataaaccttttgccatctcttacttggaatggtgaaaaggtaggggccagattgcgattccaaccgaaagaagtgaaaaatttgtatgcggcatatataatggcaaaacgaaatgtaaacgccattaaggaaaagcatggaaatgaaagcattgatatatatcccaaaaatctgacagattttatttctcatcgcaataatctacaaacttattttgaactggtgtgttaccttcttgacgaggaacaagatatttcagaatataaagagtctgtttatgaaattgaaaatccgtttaagaaacttattaaaattaactgcatagaggctcttcgtgaattttccgatcccgatggaaacggagacaatattattgacactttatccagacagcttcaagaatattataaaaagcaggtagatccaagagaaaatatcagggagaatgattatagtttgctaaaagctattgatgaaaccaataaggtttttgatgagaatttaatgaaaagtttcgcctccattattgacgagttggaggaatttaattatccgggatttcaaaatccgaaaatagaaatccatagttattcaaatccggcatcttcaataggccatgattctgccgttcaatttattatgccgggagaagagggattacgcatccctgagaaatataatggattgggttatcgtaatcttttatccatgtattttaagttgattcagtttagagaatcgtggttacatttaagcgatcgtcgtactgatggcaaacaagaaatagaacctatacatttagtgttgattgaagagccggaagctcatcttcatgcacaagcgcaacaaatttttatccgtaaagcgattgacggattgaccaatgtgcagtttctaaaagacaattcgcagttttctacgcaattgatcgtttctactcactctacgcatatttctaatgaggtgaatatgtgttgtatgagatatttcaaacgaatacaaaagactaaggaccatattcctattagcaaggtaattaacatgcgtgatacctttggagaggacaaggaaaccgaacgttttgttacaagatacctccaattaatgcactatgatgtattctttgcagatgccattatactgatagagggtgccgcggaaaaaatacttttgccgcaattcgtacgcaaaatggaactgggatcgagatttgtgtcgattatagaaattaatggaagtcacgcatttcggttcaaacctctaatagataggcttgaagtattgacattgattatctccgatatcgatgccaaaggtaaatatacggatgaagcaggaaagccgaggtcgaaagccgaacttccggaagtcggtaaaaatcaagaaacgagcaacaacacattgattgactggcttcctcaaaggaaaatgattgatgaattgctcacgttggaatctgacaagaaagagaacgcccatatacgcattgcttatccatgcggtatgaaaataaaatataaagaagatacgaaagaaattgatgtatatccttatacatttgaagacgcattgattttctcaaatatcgagttgtttcgtcaggaaaaattaggaaatatgggagctgttacgacaataagtaatttattgaagagcaatgcagatttgctgtcattccataaaaagttatttgaaaaactcgaaaacaagaaaattacaaaggcggaacttgctattaatctgctttttgctgagcaatttggaaatttagtcgctcctccatatattcaagaaggattaagatggttaaaatctaaattggactga

SEQ ID NO: 12 - DNA, 1911 bp, Alistipes senegalensis
gtggattatctcgacgtggtccccgacaacattgcgacgctcgacattgcgttcaacaaccgttccagcgcggaacgttacctcacgacgtgttattcctacgtaccgctctacggcgaccaggattggaatcctggactcaccgcagggaacgagatctggtactattcgatggacgacaatgtttatgtccagaatctctgggcattcgggattgccaatggattgcagaacatcgtaactccgctcaacaactattgggacggggaagagcgcggaatgccgctcttccaggctatacgcgactgcaacatcttcatcgaatacgtttccgaccgtaaccgggtggcggggttgtacgaaaccgaacgccgccggtggctcgccgaagcaaaggtgctcaaggccttcttccactactacctgtttcagctttacggcccgattccgattatcgacaagagcctgcccatcgatgcgtcagtcgaagaggtacgggtgtcgcgcaacaaagtggacgatgtggtagactacatcgtccggacgatcgacgaatgttataccgacctgccgaaagtgatacagatggaggccgtcgaactcggccgtctgacccaggctgcggcgctggccatcaaagccaagacgctggtgctggcggcgagcccattgttcaacggcaataccgattatgccaacttcctcgaccacgatcacaagccgtttatcagccaggaacaaagcacggagaaatgggagcgtgcagcggaagcctgccgggacgcaatccggtcggcagtggacgacggaaagcacgacctgtacgatttctcactcgatgcgacgtacccaatgccggacgaactgctgtacggtatgaacacccgccaggccgttactgaacgattcaataaagaactgatatggagcgtcggtacacagtcgacattcgacctgcaaatcaatgtgatgccgctgattacacccggcacgaacaatatcaacgcgtccaatgcgaacagttattgcaaggcaaactatgcacctacgctggcagtcgccgaacgcttctattcttcgaacggcgtgccgatcgaagaggacaaggtctggaacgatccggccaacgattactacaaccgccgttaccaaacgcagagcacaaacggttacagcgaatacctattcaagcagaattacgagacggcgatcctgcacttcaatcgggaaccccgtttctacggttcgctcggattcgacggctcgacgtggtacggcaacggttggaaaaatccggacgatgtggatacgcgcaattacgtggaggcaaagaagaaccagcgggcaggccagactaagatgggcatctattcgattacgggctattatgcgaagaaactcatctattacgacaatacttacggatcttcggtttcagtccgggagtattctttcccgatcatccggctcgccgatctctacctgctctacgccgaggcgatgaacgaagccaacatcgacaagaacgtccccgacgatgtatatatctatgtgaacaaggtacgcgcccgctcggggctgaaaggggttgtggagtcgtggcagaactattccatgaatccttcgaagcccttgacttcgctcgggatgcgcgagatcatccggcgcgaacgttccatcgaactcgcattggaaggacagcattacttcgacgtgagacgctggaaaacggccgtaaaagagttcaacaaacctgtgagcggctggtcggtggaccaggagaccgtcgaagggtattacaatgtaaggaatattttcaaccaacggttctatcaacgggattatctctggccgataaaagagtacgatctggtgattaaccccaacctggttcagaccaaaggatggtag

SEQ ID NO: 13 - DNA, 6441 bp, Clostridium boltae
gtgaataagaataaattagtgaaaagaactttggccattgtactatcagcagcaatggtatttacaaatattggccattccccgactgttgcgtatgcagccagcggaaacagtgtggacttcatggtatcaggaacggattttgttgctgctattgaagacatgattcattcaggagcagagccattaaaacaagaggagctggattttaccaatggaaaggcagaaaagtactatcagtttttctttgatggggaggacccggtatatgagttctatccggaatttgatggtcaggatatggaggcagaagtaagggtttttgtccgccttccggaagcagcggatgatacatattcccttactggtgaggaagagattatatttctatatattaacaatagtgaggataccataagctgctcaacaacaatcttaatgtcagatggcagtgaaaagaggacaaaaagggttacagtcaaggactatgaaactgcgtttggtgataacagaattgagtataaatccaatacatctgccacgggccagacagaggctgaaatacctgaatccgatgcagcagaaattgagaaacccggaacagatgcaccgatggtggaaacacctgaaaccagtatggaagagtccggggtgacagaaccagagacaggatctgggattcctgaccaggaaacagaggaaaaggaaaacgaagctgttgagacggatgaagtgatagaagataccgagccggaaatcgttgaaaagtcagagccagagacgcagtctcctgatgtatcggaagagggaaaaacacaggctgatagtcccgtggcttcccgtatcaggcatgcagttcctgtcgtggcggcagtggatacaggagaagaaaattctacgattgaacccagtgttgataagcagcaggaggatacagaaacaggtggaacccatgatgattcagaaaaacatagtaatgataaggacaatgaaactgtaggcagcgtacctaaggaatcctctgcagaggcagagtctgaaacggagtcattgacagaggaaagcgggaagcagacagaagcgtctgccgatgaaaccggagaagaaacagctgcagttgagtcatctgaacctgcaacagatattcagaccccttcagaggaaagccggacagagacatctgaggagactcagacagagacatccgaggagactcagccagtagaatcagaacccgtccaggttacggaaacccaggaaagccagatttcgacagagacggaaagcatcccggtgagttctattggtaatggtgatcttgtggggatggacggatgcagcactgcaaaggcatatgtaacaacactgaagaaattgaaagtattagatgaggtggacggataccgtgtcacatatgagattacccccgaagacaaggcggcaattgtagataagtgtgacagggttaaagcaggagaaagcgttacctttggtgtagaggaacaagagggttttcgtgttgggcaggtagaggcaaatggagatgtggtggaatccgcatacagtgaggaaaacatcgtatggtttactctggagtatgtagaggaagacttggaaatccttataacgatggttccggatggtacatctatgccttttaacaaaacgatctcaatggatgatggtatggatattaccatatccgctttgccgggtgttcttcctgaaaatacggaggttacagccgaaattgtaacatcacaagttgaggaggcaatcaggtctgaccagtcagaagagggacgggaaattatagctgctcctgcttatgatattaacctgtgtctggatggagaaaagctggatgatgaaatctggaacaggaatggtgctgttacggtaagtttttcaggccctcttatggaccaactgattcaggagtcacagatggcccaggttctctgggtaaaggatgagaacaacagcacagaagtaatggaaggcagttataaggatattacccgggagggtacaactgaagatctaagttttgaaaccagtcattttacgacgtttgctgctgtctttgctgtagcgccggatatatctaatgtatttaatattgatgaacatggactgatggatgaggattttcctaaacttgttgtccgggataaagacgaaaatacacttgatattgagattacagaacaggaagatggggccaggagggttaccttgaaagatggaaaacctcttccaaggaacataagcacctggtttgagatttcctacgattttaagaatagttcagaccctttttttgaaacttacagtgtacagaagggagaccattttacatatcagttcccgtcaaatattttatatgacaaaaagcagactgttgtaaaagatatcaatggaggagaagctgtcattggaacggcatccatcaatgcagagggttacatggatgttgaaataacagctgaaaatgtaggccagaattatcgcggcacggcagaagccggtggtaaactggatttggaaaaggttttagaggaaaaaaatgaaatcactctggtgggtgacgaagtggagtacattatggaactggtgccggctccggtgcaggaaaattactctgtaaaagtagtcaaaggacccaagagcggaaagtggacagaccaggatatcaggtatgatgagaataggcttccttcagctttgcagtaccatgtaaccgtgacagctgatgcgcagaacagcggcccaataaccaatgtaaaagtaagcgataccttggggaacaccaaaaacggaacgattgtatttgacaagacccaggaaatcaaatttgaatccaataatcaggatactgttatagacaatgttactttcggcggcatgagcaatgggggaaagaccataggtatccaactgaatacaaaggatggaatgccggcctctatgatgcctggagagtctgttagtttatcttattgggtaaagcttggagccggtgcttggagcggtcagaataccgggaattcttcaaaagagatgtccgcatccctgtttttggaacttaagaatacagttaatgtgacagcggataaaaaagtatcgggcagtgacagcactacatttaagaggaccatagaatgcgttaccaagagtggaattgtacattataattatgagatagatggtaagactgagccggttgtcattgagtatcatgtttttgtaaatcccaggctgattaatatgaccggatggacgattgaggataagctggataaaaatcaaaagtatctgggaaatgtagaagttattgcttatactggcaaaaatggaacctcacttgggaaagtggatgacattgaaccaataatttctaagaatccccaaacatggaaatatgtcattgaaaatccaggaaaatattactatgatttcaaatactttaccactcctaatgaagcaacagaaagcaatctcagtaacgaaataaagataacatggccaggcggaggttctggaggcataggcggaagtaccggtgtcggattcctgtacaacacctataccatgacaaagaagaacttaagcagcaacatgaaatccagcaataacattaattccggcggggtatatgagcctgtcaataatacagccggaaatgttgggtggggggatgaatttggcacaatccgctggcagagcgtgcttaccccatatgcagacgggcagacgaaaggcgccacgattccagcgggcactgtctataaagattctctcagcgtaattaagtggggaaataaaaataaggaagatgctgcccgtgcaaatatgcatacattcaaggatgatggcagctttaaggcttcctttgttctgaaagacggtaatggcagggctatatctccggatgatgggacctatacattatcatttgatgaaaaacttggaaaccgtggattcagcgtagtgttttcaaaagatgtcccaggaccggttgtcattgagtatgagtccttcgtggatttagagatgttggaaaatgtgggggtttttgataaagacggaacaaaagataatctgcggttcaaaaatgtaggtgagatgacaatcaatgggacaacatggaagagcgctacctctcagccatattacatcgaagattatatttcaaagaactgggtaaaaaatgatacgaaagcaggcaccatcacatggaatctgaatatcaacaagggatatgggaatgatgcaccccaaaatctggggcgtttcacggttgatgttattgagtatataccggaaggactaactctggaccatattaaattccagagcatgaactatacgctgaaaccagaaaagggagattacgatatagatggaaataaagtgaccatccaccttaacacggttgctagaaacttttctggttacaagatgagcaaacatattaacctaaacatcataaccaaggttacagatccatctataaagagttttacaaacagcgcccagatggttattgatggaaatatgcttcataaagtatcagctacgactggttttgataagagcttcctgaaaaaaggaatggcatacagccgcgacacggcgccgtatgctgaatatacaattctggtcaaccagccaggggcagatatcagcaatggtaccctgaccgtaattgataccttaggagtacccgggaaaatggcatatgttccggacagctttaaggtaacaaatgcagaaaacgggacacctatagaagaagcgaatatcagggtgggaaaagacagttttggcaatgacagttttgagatttccaatcttccgaacaaaacgcccattaagattttttataaggtaatgattacaggagctataaatgaaaccgttgatacgaagaacacagcatccctgctctacagcagagaaggtataattaccgaaaccattgagcgcagcgtcactattgtaaaagccgcctttacaggaggaggaaaattttctataaaactatacaaggtggatcagaataaacagccgctgacaggagctgcctttacgctgagcaaagtatcagaagtgggaagcccggatttagaatatgtgggagagtttaccccggtaattgattctgggaatccgcaggcaggcgcagcagtgctgataacgggactggagaaggggcagctgtattatctggaggagactacggtgccggaaggatatcagaaggcagaaggggagtattttatcattccggatagggagaatggtattggggtgccggatggagcgatagccatagaaaatgccggaacacctcatgtagtagagaacattaagaattccggtacattaaagctgaccaaagatgtaaacggcagggaatcaggcagtgattttgagaccgatttctactttacagtctatggtggagaccgatactacgatagggatggatcctacgccgacctgaggactgtaaaacttcactatgattccaggattgcggataacagcctcatactgtcgctgcctattggagaatatgtggtgaaagaagtggcagacgcagaggggacgcctattaacggtgataatttctattataatgtacagataaatggtgaggacaggaatgaagcggtcatagctattgaaaaagaacagcaggcggaatgtctggtaaagaatctatatgaagcagatggaaatctccaattcactgccatgaagacaatggaaggaaggcctttggaagaaggggaatttactttccgcatatacgagggagacacgctgaaagcggaagctcaaaatggactaaacggagttatcctgtttccggagattaactacaaagccaatgatgcgggcagacatacctacacaatcatggaacagaagggtacattgacaggtgttgactatgatgatactgtttatactgtgacggtagaggttacggacaatcatgacagaacagtgagtgcagaaatagtaaatatccagaggtctgatggtgctgaggcagaggtgatacagtttaataatgtttaccatgagaatccagaaaccacaccggatccgtctccaaatccaaacccatctccttctccgggagggagtactggaggaggcggcggtacttccaatactgggggtggacggtaccagccttctgatggcggaccaggagttacaatcagtattaccccggaagaggttcctatggctcagattcccagccaaccagactctctgattacgattttggatgacgatgtaccgctggcaccactgccaaagacaggtgatatgtcagttgatcattatatgctgactgtgatatcaatgttactgacagggatttatctagcgttgacgaaaagaaaaaaggaatga

SEQ ID NO: 14 - DNA, 3714 bp, Clostridium boltae
atggatttgattcgtgattttaaggacccgggaagggaatacagcgtgctggccttctggttcttaaacggggaactgaaaaaggaacgtctggcctggcagattggccagatggtggaaaaaggcgtgtacgggggcttcatgcaccccagggcctaccttaagactccttatctggaggatgagtggtgggacgctgtcggggtttgtgtggaggagtccaggaaacagggatttgccccctggctctacgacgagtatgcctggcccagcggcaccgcaggtagtacctttgaatatggattccaaaagccttccaggatactgtcccggggaagggacaacatggcaaagggactctgggcggtgaaaaaagatgccgggaatagggaatgcggaaatgaaggtgccggaaatgagggcggcggaagtcagggcggcggaaatcagggcgccgccaccccggatgccgccaccccggaggataagggacaaagcggcgccaatccgtcatcaatgccgtaccgtgtggtgaaaagagatggttttatctatgagttttatgaaaaagtatttgaaaaggccgtggactatctgaatcccgaaaccattgcttccttcataaaactgacccatgaggaatacagaaagcggtggggggaggattttggtaaactgataccgggtatctttttcgacgaaatctacatgatgggaaatcccctgccctggacggaccggctgccaggacggttccgggagacatatggttatgacatcctggacgagcttccctctcttgtggacggcgcgtctgagcgggacaaacaggtgcgaaaggattatttctccctcgtaaccgccatgtatgaggaagcatttttcaggcagatatcagactggtgcgggaaatacggtcttaagctgacaggccacacagaggagtttttgtgggaacatcccagaaggcagggcgattattttaagaccatgcgccatctcatggtgccgggctctgactgtcacgattaccggtaccggtatcccagaaggattacatactgcgagcccaagtattctgtgtccgtggccagaatatatggaaaagagagggctatgtcggaagccctgggaggcgcgggatggaactgcaccatggaggaatttaaaaagggaatcaatactctggccgccatgggaaccggaatgttcatcctccatggattctactacgagtgtgagcaccagggttcccagagtgactggcccaccagttttttctatcagaatccttactgggactattttaagatatttgccgattacataaggcgtctatccttcatgaacagccagggaaatcctgtggtggattatgccatcctgtatcccataggggacatggatgaaaatatggagaacggagaggaaaatccctcaggccaggccataaacaacggattccaccaggccctcaactgtatgattgagcaccagctggacacggatatggtggacgaggaatccattttaaatgctcatatatgtgacggaaagctgtgcctggggcagcagcgttttaaagtgctcctccttccggaagggggaagcctgatggaagaaaccgtggaaaagctggaagcatggacaaagaccggaggcagcgtcctgttttacaggaccggtctggctgacgaataccggtccggcggggacagggctggcggggacaaggctggcggggacaaggctggcggggaccggtccggcgaaaacaggtctgacaggaactggcctggcggggacagggcgaacggatgcagagtaaacggatgcagcgtaaacggatactggaacacggtcctcagggaaaatgtacacagcatcagccgtattccggaagcagcagctgcactggctgcgccgtccgcatccgtgatttacggaaatcccggagacatctttttgaatcatagaatggcagggaatgttgactattatctggtggccaacagcagcgatgagaggcgaaacctggtgctgtctttcagccatgcttctacaccggtccttttggatattgaaaaaggggacatggtgcaggctgtatacactcaggcgggcgccgcccaaatgtgcggaggccgtccgtccggcagcggtgtcctgatttacatggatttggaaccgggagaagctgtctacgtactgtttggtttggaggaagatacaatcagacaggcaaaaccggcccttacgggggatatccggtgggaggaagagtggattacaggaaaatgggattttcttcccctttccccgtccggcccgaatcatggagataaggcatacaatgaagagagtacggttctggaaatcccaatcgcagaattcacctctgatgtaacctccggaacagagaccatccggatctgcaaccaatccggggaggaggggagctgcggccgccatatgagcctttggaacggacggtggattacacgcagacgaagctggaatgaccagctggatgcatcggatctgtatttcagaaagacggtattcctggaacatgtaccagaaaaggcggagttctgcgcggcagcggtggattcctttgagtgctttatcaacgggacaatggtttacaaaggaatcagcaacggagagccggtggtatttggtgataagagccagctgacccagggggagaatattctggcattccatgtaacaaaccgcaacccgcttcatgatgtatatgtctgctccgcagaggagctgcctccagaccggttcatttcccttcttatggaaggaaccatcgttcagggaacaaacgtggaagtggtgaaaagcgacagcacctggattgtaaatgacagtctgattaaagggtgggaacagccggattcggacgggcggtttacggcagccggctttgatgtccgcaaggtcctgaatttcaattatacggggctggagcatgtgtggctgaaagcctgggagaggggaaaaccgcctttgaagccgtggggagaccttccgttatttgggcagaccctgacctatcccagaaagctctggtatacagtcacaatacctgccggagcgtcagttatatatgagcctgttacagccggagcagcggtctgtatgctggacggcaaagaggtgcattgggaaaatggcatacacatactcccggacaatgaacgcattcacatacttaccatacagataacggcaggcggatgcagcgacgggctgaaacagccaatccgcgtaaccatgaaggcagtggctgtcaatctttcggactggcgtatgctgggacttccgtggttctccggaaggtgcaggtatactaacacatggtccgtggagcaactggagggcacgtacatgctggagcttggcggggtaaaccactgtgcccaaatctggatcaacggcaggctggcagatacaaggctgtggcgtccctatagggcggacatcacttccctgctcaggcccggggaaaatgagattaccatattggtatccaacctggcctccaatgaacggcgccacatgctggtggacgaaggaatggccctgggatggaaccggtactggaacgaggacaacatggaccgggacagccggaattatgtgtcaggccttctgggaccggtaaggcttcttcatatgatatccccaaaaccataa

SEQ ID NO: 15 - DNA, 2895 bp, Clostridium boltae
atgaatatctctgttatgataaatgactttataaggcaaaatattcagtctgaggctgaagtgagaagcaaactgattgttcctttattagaactattggagtatcctaaggatttgagagcggaggagttcccagtatatggttatgaaggaagtaaagcattaaaaacaaaagcagcagattttttacaatttacatcaaatcaatttgataaatatagagggaaaactgatttagaagtagactgggtatataaacatagtttgcttgtttttgaggcaaaaaagcctacagaaaaagtattggtaaaaggacaaccagtattttattcagcatggacgaaatcggttgcttacatgatttcaaacggaattaacatagaaggttatatcgtgaatgcaaactattctgatacatgtgtattttcatgcagagttgaagagattcctgaaaaatgggaagagataaatcttttaaactatgatagaattctggaattaaagaaatcatcagatgaaaaggataaatggactaatagagatatttatgaaaaatacaaaaatgcgatgcgggtacattgtacagaagagttatgcatatgcgtagatagaagcttaaaggaatttgcatatgatttaaatattttaaagaatggagaaaataaagattttggcgacatattagataatacatcaaaaataatcacatcagaacctggaggtggaaaatcgtatctgatgtggatgctgatgcgtgagtatctgacaaagtgtaatggggatgaggataaaataccggtaattttagaaggaaggtattatggaaaagtatttaattccatagtagatggaatttatcaagaagttaatttgctgttgccttttttaacaaaagaactaattgaaaaacgtctgcgagaaggtggttttgtaattttatttgatgctatagacgaagtagaacaagattatgatgttttggtatatagtttgcatcaactaaggagaaatacagacaatacaataatcattacatcaagaatgcaaaattataaaggagatttttgttctgagtttgcacattattctctggaaccgttagatgatcataggattgttgatttgttgaagcaatactctcaaggggagatgcagattcaaattcatcaaataccaaaaagattaatggaaattttaagaataccattgtttttaaagatgtttgtttctatatcaaagaaggaggacaaatatagaattccgtctaatcatgcggcattatttcaagagtatattaatgagaaaatgaatgtactttcatgttctctgtatgataaaacgattattaaatcagtgctaggtaattatgcaatgtatagttttgaaaatggggacagtactgaacacttttttgaaattatggataatgcttgcaccgatctaaataaaacaaaaatatacgaaaaaatatggaaaacagggttgatgtctgagggcttacaaggaattaaatattatcataaagcaattcaagagttttttgctgcagtggaattatctacgtgggatagagataagcttaccgcctggctggatagcaatgcattgaaagaaaaatacaatgagatactttgttatttgactggtattatttcaaatcagcaaaaacaaaattatgtattggattacttggaaatacacaatttaaagttatttgtaaaggcacttaaatccagaagaaattttgatgttgttgagatggatttgaattttgaatacgctcagagttattatgcacaaattttaaaaacttatgacagtatagttcaatcctatttttataaaatatgccatgtttttgatgggtacagtataaaaggaaccggaaaaatctgtatccgtggctgtatgaattttacgaaaaaatctatttctatgataatttataatggaacatcggatgccaaaagtttggatattacagtatctgatgaaaacggtgtatatatggcagtagcagatggaaccgagataccaataaattcatcagtatttacggcgggacatttgcatgaacggtattacaatttagagttgttgtcttatgggtttgattcttccagggaaattgcaattgatataataaaaagtcaaatcacagaaatgttagagcaaaaaagcgtgtttgatattgagatagatgtattgctagcggagcgcatagaaaaagaattgaaaaaattgcgaaataggagagaaagtcaaaataacagacaggatttaagcttatattctaatgatataaattatgttattgataaagtaaatgaactggggatatataatcaagatgtagatatgattactactttttgcaaagtattaggacttagaatggataatgcggagagtctcctagatattaaggaggatttgactttggctccaggaagacattcatattggtttgacgaattatattcagatgagcagttagtaaaaaaagttgaaagaatactttccttatcgaatgaagcaatacaaacgataactacgaatattattccggtattatcaacagtaaaacccataaccagaaagataggaattgttcatcgaaaaggtaaattttctggcgttagttatatgagagtggaagtcagggagaatgaagatacgactccaataattgaatttggagaagataatattgatatataccctaaattagatccgtattatgttaataaattaaaagaaattggtaaaagtgaaagtaatgttcttgggtcaagttcagctgttttagatttatattttagggaggacgtatttcatgatcagatttatggagagataaaagatttgtttaaggagttattaggagacatatga

SEQ ID NO: 16 - DNA, 2877 bp, Clostridium boltae
atgcagacaaaggtaaaagggatgaatgggatattgatgatagccgtgcttctcattgtattcctgttccctctggacgtatccgcagcggagacggcttctgccgcgcttgtaggctattatgaagatggcgattacatgtatcataatgcgcagggggagtatgaaggttataacttcgagttcctccaggaagtctcaaaactgagtggactatcttacgaggtagtggattcccccagctggcaggaagcgttccagcttttgattgatggcaggatagacattctgcctgctgtataccgcacggaaggcagaatggatcagatgttatttaccgatgagtccatgtgtacgatttatactaccctcaatgtgcggatggatgataaccgttacaattatgaggattttgacgctttccagggcatgagggtaggcattattaaggggggtgaggatggcgaaagtttcaaacgctactgtgcgcagaacggcgttgcgctcaccatcattgaatatgatgagacgcaggaactgctggacgcgcttgggagcgggaccctggatggtgtggcaattacccacctgggccgcagcagtgtgttccgcagtgttgcgcggtttgccccgaccccaatgtacattgcggtctcgaaacagcgtccggaccttttggctcagattaaccggtccattaatgacattcttctgcgcaatcctgattatcggacggacctttatgacaagtatctctcaccaagctccaatcaggttccggtactaaccaaggaagaagttgaatacatcgaggctgcggatgagccgatacatatttcttacgacccttcgtttgcccctttctcatataaagatgctgaaggcgagttaaacggtattatggcagatatttttgcccggattgcagagaagagcgggctggacttccagtttgaagcctgccctgcagccacggccttacgtgcagtgaaactgggggagacggatgccgtttccgttgtggatggagattatctgtgggatgagcgcaaccatatgaacaccacactgcgtttcctgaatactcccagtgcaatgattacccaggctgaaagaacggagatagaggtgctggctcttccggaggggtatcagctctctgaacatgtcgcccaaaacaatccggaaaaggaaatccaatattacgattctatacaggcgtgttttgatgcagtcctggatggaaaagctcaggcaacttataccaatacccagacggcaaattacataatcagcgcccccaaatatgaaaagcttcatgtcactgcgctgacccagtacccaaacgacctctgtatcggcgtatccaaatctgccgaccccaggttgttctccatattggataaatatatccagtatatgtccaatgaagagattgataccctgctgctgaacaactccgtttctgtccgtcccattaccatggaagcgtttgtacatcagaatatctggttgataacagggcttgtggcagctgtatccggcagcatcatcctgctgctgtgcatcaacctgtttaatatttcccgcagtaagcgccgtatccaggacctgctctaccgggatgagctgacaggtctggataatataaaccgtttttatgtccgggcggaggaactcctggcgacggggaaatatgcggtggtttattgtgacattgaccgtttcaagctgataaacgatacctttggctttgaggagggggatgaagtcctgcgcgcattcgggagtatcttacagaaatcaatggaggacagggagtgctgcgccaggctttcggctgataacttcgtgatgctcaggcattacaaacaatgggaaacgcttgctgctgatttgatgcatatccaggcggtgctgaacaagtggcgtggggagaggggaatcataccttatgagatcgcggtatcctttggtgtttaccaggcggatgccggcgagactaacgacatgaaacagatgcttgactttgcgaactatgccatgcgtagcgctaagacagcggcaggcggaagctgcttcctatatgatgagcagatgcggaataaggccctgtttgaacaggggctggagggaaggctggcctccgcgatggaacagggggaatttgaggcgtattaccagccaaaggtggacatggatacaggcaggattgtgggctgcgaagccctggttcgctggaatcacccggaacaggggcttctgatgccggggtccttcattccattttttgaaaagaagggtcttattgtccgagtggaccttcatatgtttgagcaggtatgccgcacagtacgcagatggctggatgagggacgtcccgctgttacagtctcatgtaatttctcgcagatgcatttcggacatgacgggtttgccggccaggtttctgaaattgctgatcggttccaggttccccatcatctgctggaagtggagattaccgaaagtgcgattgccgatgcacctgagagtgtgtcctccgccctgacggaactgaagatgcgcggatttcagattgccatagatgatttcggctccggatattcctccttggggcagctgcaaaggctgagggcggatgtcctcaaactggaccgcagctttgtatgtgccgggcttcagggaccgcgggagcagattgtcattgaaaatctggtgaacatggcctcggagctggggatggaggtcgtatgcgaaggagtggaaacccaagtacaggtaaaagtactccaggatattggctgccacatcgcccagggctattactattaccgtccgatgcagacagcagcgtttgagcagcttctgggctaa

SEQ ID NO: 17 - DNA, 2520 bp, Clostridium boltae
atgaaccaattgattaaaaaatataggatggttttgtctgcaatatactgcctgatactgccatacagttttgtttcctatggagcagaagcagagtctgtgattcgggtgggatttcccgtgcagtcgggtctgaccatgaaggatgaaaatggcaattatgcgggttatacctatgattatctgaaagagattggacagtacacaggatggacctatgagtttgtggaaccccaaggatccatggatgaacagttgattcaaatgatggatatgctggaacggggggaactggatcttgttggagccatgaataacaacaagcagacttcctctgtttttgattttcccagtgaaaactacggcaacgcgtacagtgtgattgcggtccgggatgatgatgaccgcattgatgaatataatctttctgatttcaagggactgcgcatagcgcttttgaaacaggcagattaccataacgaaaagttttaccagtacgcgaagctcaatggcatccagtatgagatcgtttggtgcgagagggatggggagcaggaggagagggtttattccggtaaggcggacgcattgctgtccgttgatgtatccctgtcccagggattccgtcctgttgctaaattttcgcctactcccttttattttgccaccaccaagggtaataccaaaataatcaatgaactgaaccgggcaatctcctatatcagtgagaataatcccacccttcaaatgaacttgtataataagtatttttcccggtccggaagccagatgcacctcaacagcaaggagcgggaatacatacaggaacatccggtacttaaggtactggtccatgacgggtttggccccatccagtactacgatggaaaaggacaggtgcagggcgtagccagagacctgctcagcagtatagcccaaaaggccggatggacgctggagtatgtttacgcggatgattacagtgaatttgaacaggcgttaaatgaaggcagagccgatgtgattctgtctatcctgtatgattatgatgcagtccaacggagaaatgttcttttaagcaatccatatctggagacagagagtgtgctggtggcccgcgacgggtttgatatgacaaacctgaagggcagggtacaggctgtgtatatgggcatgcgcaaaagcgacgatgaccggacggatgtgcggttctatgattctctggaggaaagtcttaacgcagttgaaaggggagagtgcgattatacatacagcaacagttacactgcctcttattatctgagccgcaaccagtacgagcatgtggctatctatccccaggccggcagtgacagtgtgaaatacagcataggtattttgagaaaggatgataaacagatactggctatcctgaataaaggaatccgttccatagagacgggtgaactggaaaaatacatctacaacaatgcgcagcagaaacaggaagtgactctcaggacctttatcagggataattccgttcccttcattttgtttaccctgttggctgcttccggcctgctggccctgatttatgcccattacagaagccagatgaggatgaagcggcagattgaactggaaaatacccgttaccgctatctctcagacatattgaaggaagtgacctttacgtatgactatggcagtgatgtgctgaccctatcaagggagggcgttgaaatcttcggcacggataaaagcatcgggcagtattcgcggtatcagggaagcagcggacaggaggagggtctcccatctctgtattatctgctggagcagagacaggatgtggatacagagattctgatggtgctgccgaatggggacaccaagtggcaccgtgcagtcataaaagtgattttcgacgggaatcaggctgattctgccatcggacgcttacagaatatccatggcgacaagctggaaagggagagactggagcagcggagcaaacgggacgctctgacggggatttacaatatagcggcagcaaaaatggagatcacccggatgataaacctgcataccggcgcccttgctctggctgtcatagacttagacggctttaaggaaatcaatgaccgttacggccattatacgggggaccaggtgctgattcatacagcaaaagcgctaagggaatctttttgcggggaggctgtcactgcccgtatgggcggagatgaatttatcgtctgtgtaccctatacaggggaaaaccatctggcaaaatgctgcaatgcactgtttgattcactgcaggctaaatgcagggcgtccggataccctgctgcgactgtcagcatcggtatatctataagccgcagggaggacgactataccacgctttatcagagggcggataccctgctctatgaagttaaaaacagcggtaaaaataatttccggatagaagatgaagcgggaaggacttcccggccggacacggaacaggaacatcacacggtacagtaa

SEQ ID NO: 18 - DNA, 2421 bp, Clostridium boltae
atgagagagcgcgggaaaaatctgataagatgcggggctgcttttgcggtgtcctgctgtctgctggcaggaaatgtgtttcctgcggcagccgacacctctgtaagcggagcaaccatgcgtctttcttccagagagggcacggtaaatgtgtcaggaaaaggaggaaaggcggttgcggcctttgataacatgcggctccagagcggatataacctggaaacagaggctgcaagctacgcaggccttgcactggatgacgtaaaggccgtgaagatggatgaactgagcaaaggagagatacggaagaaaggaaagcagctggagctgcttctgtcagaaggaagccttctctgtgatgtaaccgcgcctcttaagggggaggagtccctatccatccgcacctctaccatgataaccggaatccggggaacggtagtatacgcggaagtggttgacagcaatacgagccgcgtctgcgtcctggaggggcaggttcttgtaagaccggtgaatcctgtggagggtgaccggaatgggcagtacatagagaagggccggcaggcacttattatcggtcctgaccgcatggagcggaagggagagatacagacgcttccccttacggaagcagatattgccccttatgtgctttgggaaatccatgagaatgaggagcttgccagaaggctgagagaggcaggttgggatgtggactggatgattgaaaacgcggaacggcttttaagggaagaagaggataaaaactcccaatgggcagagaaggggcagggaacatcaggctctaagcctggcgggaaggatattcacacccctctttataacggaggggattccggttctgattccggaaccggcacacagccgggcagacctacggtggagcttactatgccggtgagtccggaaaccatagaggaaaagctgcggacatctgatgtggttcttcacagcgctgcggacagcaatccccttatcattgataacagcctgaccgtaccggcaggcagccggctggaattagccgggggaatggggctggtggtgggaacgtcggcagcattgcaggtggacggaactttgattgtggacggaaacctggaaaacagaggaactgtaacgaataccagtatgaataccctggatattaaaggagattatgtgggaagcggaacactgaataataaagggagagtggcggcaaatggttcctttatgcaggaaggcggcagcttccaaactatcggacagggccggcttgaggtggagagaaaagctgttattgataatgcagcctttgatttcggtaccggaactacattgtttcacggtgatttgacagtcagaaacgctgacggggaatttggcgataacctgtgtgtggaagggatgctttcattggaagacagcagtattctgataacagggggattttacagcggggggattaccgcagtaaagaaacaagatggagagaatatagcatatgaagagctgaacctggagggaggaaaggttttggctgaacgtggggtcaaaggggtaatctttgcagaaaattataagctgaatgtacaaagcggtatcttggaaaggtcagatgatgggattccttttataaccggcacaggtattttagaaatggatggagaggaatataaaattgaagagttgacagagtccatgtttgagagcgaagagacagagacgggctgggttttaactggtattgtccaggaacaaaaaaaacaggcagaggtgcttacttctatccctcttcaggcagatgctgaaaaactgccggatgtgaatgaggaagagaaagagctacaggagggagagagtttgccggaggaaggagagccggaagagggcggaaaccagccggaggaaggaagtccggaagagggcggaaaccggccggaagaaggagaaccggaagagggcggaaatcagccggaagaaggagaaccggaagagggcggaaaccagccggaagaaggagaaccagatgagggcggaaaccggccggaggaaggagaaccggaagagggcggaagccagccggaggaaggaagttcggaagagggcggaaaccggacggaagaaggagaaccgggagaaggcggaaaccggccggaggaaggaagtccggaagaaagcggaaaccggccggaggaaggaagtccggaagaaggcgccgcaaaccagccggaagaaggaagtcaggaagaaggcgcaaaccagccagaggaaggaagtccggaagaaggcagaaaccagccggaagaaggaagttctgaagaaggcgcaaaccggccagtagaaggaattccggaaaagggcaaaaaccagcctgaaacaggaaaaccggaagagtatggaaatctgccgggataa

SEQ ID NO: 19 - DNA, 2373 bp, Clostridium boltae
gtgaaatatttcgagcatgagagcgctgccacctttgatgaggcagtctccttattaaaagagtccccaaaagggaaaacagtcgtaatggcagggggctccgacctgattggagtgttaaaggaacagattctggaggattatccggaaaaagtggttgaccttaagaccgtcaggggcggggaatacataaagcaggacggggacaccatagaaataggcgccctgacaaaactctgcgacatcgtaaagtcggacctgctcaatgaaaaggctccggttctctctcaggcggcccgctccgtggcaacaccgttaatccgcaatgtggccaccatgggaggcaacatatgccaggatgtgcgctgctggttttaccgctatccccacggcatcggcggcaggatggactgtatgagaaagggcggaaaagagtgctatgccgttatgggagacaaccgttatcattccatattcgggggcatgaaggtacataccacaccgtgttctgtccagtgtccggccaatacggacataccggcttatatggaacggcttcgggaaggtgatgtggagggagcggcccatatccttatggaagccaaccccattcccatgattacatccagggtctgcgcacatacatgccaggagcagtgcaaccgctgcggttccgatgagagcgtgtccatccacggcgtggagcggtatgtgggggattacatactggagcacccggacacattttacagggcgccggaaacagagacaggccataaggtggctttagtgggagccggtccggccggcctaagcgctgcctattatctgaggaaggcgggccatgatgtgacggtctttgataagatggaggagccgggcggcatgctgacctatgccattcccaactacaggctgcccaagtcctatgtgaagcaggtggctgccgcctatgaaaaaatgggaatccgcttccgcctgggctgctgtctgggagaggatatacaggcagaggatctggagaaggagtatgacaatgtgttctatgccaccggcgcctggaaacgtcctgtgctgggatttgacggcgaggagttcacggagttcggcctccagttcctgatggaagtcaaccagtggatgaacaaaaaggaccgccgccatgtactggtggtgggaggcggaaatgtggcaatggacgtggccataaccgccaggcgcctgggcgcagagagcgtcaccctggcctgcctggagtccgagccggagatgccggccagcagggaagagattgcaagggccagggaggagggcattgaaatcatgccgtcctacggcgtatcaaaggcaatctatgagggcagccaggtcacgggaatggagcttatgcgctgtacctccgtcaaggatgagaacgggcgtttcaatccccggtacgaccgggaggagactctcagggtatcggcggactccattctgatggcagcggggcagaaggtggatttgagtttcctgggcgacaaatacggccttgccctggaacggggactgattcaggtggacaaggacacacaggccaccagcaagtccgggatttatgccggaggcgacgccaccacaggaccggccaccgtgatccagggcgtgcgctccgggcgcaacgcggcggaggccattaacaggggctatgcagtcatgcctgagcggcgcagggaagataagtttatccattttgacaccgcaggcgtcaaggaggagcacgcggtaaaggacaaagagctgtctgccgcagagcgggccctggataaggaggacagcttcaccctgaccggggaggaagcggccagggaggccggacggtgcatgaactgcggctgctactccgtcaacgcctcggacatttcaccggtgctcatcctgttagacgcccggattgtgaccacaaagaaaaccgtaagggcggcggacttctttaccacccgcctgaaagcagctgacatgctggatacagacgagctggtgacggctgtccggttcagggtaccggaaggatataccacggcctatgacaaattcagggtccgtgaggcagtggattttgccattgtcagcctggcttacgcatacaggatgaaggacggcctcatagaggatgcgcggatcgttctgggcggcgtggccccggtgcccatggagcggaaaaaggtggaggcgttcttagccggcaggaagccggatgaggcgctggcagaggccgctgctgaactggcagtggaggggaccgcggccatggccaataattcatataagatacaggaggtaagggctcttataaagaagatgattctggatatgggggcggtccaggcataa

SEQ ID NO: 20 - DNA, 1926 bp, Clostridium boltae
atgcctagaatcatattgaaatgccgttacctgaagcatgagaaagcacatctggcgcatctggtccgttacattgccacacgggaaggtgtggagatggcaagggatacccacgaccatctgccggcaaccgccagacaaaaacaactgatcgatgaattactccgggcccttcctgatacgcaggagtcttatgaatatcgtgattatcaggcgaatcctaccatgggtaacgcatcggcgttcattgctatttccattgagcagaatatggacctggtagcaaagaaggaaaattatgtggattatatagccagccgtcccggggtagagaaaagggggacacatggactgtttaccgatgccggtgtgccggtcatactgtcacgagtacaggaagaagtcgccagacatgaagggaacgtatggaccttcatactttccatacggagagaggatgcagtgcgattaggttacgataatgtaaaaaggtgggaagctttgctgcgcggtaagcggatgcagatggcggaggccatgaagatgtcaccagagaatctggtatggtatgcggctttccatcaagcaggacatcatccacatgtccatatgattgcgtacagccgcgaccccggtaaaggattcctgacggaaaaggggattgagcagatgcgcgccatgtacgcaaaagaaatattccatcaggatatgtatgagatgtatcagaatcagacggttcagaggaacgagctggtaagggccagcgcagacccgctgatgaaattattcggacaggatcagggaagatgggaagaaagcagtaaactggagcagttgatgacacagttggcagcggatctgaaacagacaaagggaagaaaagtatatggttacctgcctccaagggtaaagcagcaggtagaccgtattgtgaatgtattgtccaccaaccctgctatagctgaatgttatcaaaaatggtatgaatccagactggagattttacacatctattcagatcagacgccggagccgcccccactttccaagcagaaggaatttaagcaaatcaaaaatatgattatcagggaggccatggaatgggaagcgtatggggaatgtatttctgagcagccgatggatgatgtgagcctgatgattgcggaggatatggagatcatggatggaactgaatttacggatgatgttgtggcagatgatgatatgtcctgtattgtggaatttatagaagatggttatgccaaatggacggacgaatacaggcagacgaggaatattctgtatggaacggatggagaaaagccggacgtaggaacagccaatcagatgatttactccgaagctgaacagggaaatacgtttgcaatgtgtgaccttagacagatgctgcattatgggagaggatgcgaaccggatccggaagtatcccaggcatggtataacagagcattccgcgttttcctaaatgctgaaaccgtaaaggaaactgcttatttggaataccggcttgggaagctgtattatgacgacctgtatatggaaaagaatctgggagcatccgtttactggctgaacctgggagcaggtcatgggaatacgtacgcacagtatctactgggaaagctatacctgtttgaaccaacggtcagggatgatgagagcggcatcttctggctgcagaattgcgcagaccagggtaatccatatgcagtatatcttctggaacataaggatgagtggggaaggatacgactccggtcaggagttatccgcttatttcatcatctgtctgctctgtttaatgaacaggaaaacgaagatcataacaagatgcatgaatggattgaccgcaagagaggacgcaagcttaaggaaaagaagatagcacagggaatccggggatag

SEQ ID NO: 21 - DNA, 1851 bp, Clostridium boltae
atggacagttgggcagagatggaagagcagatcctggaagaactgaatcttcacaggatgaaggctgatgctgaggttttcagcagattggagcgttactccggttcagaggccggggaagcagccgtggattatctggttcaggagctggaagcagcggggattgaatatgaacggcattattatgagcttatgagaagcctgcctgtacaggcttctgttactgtaaagaaatcaggagagcctgatttcaccgtggaggcaatagctgctgtatacagcggtgaagcctatgggcttacaggagaactggtctgggatgagatgtgtaccaagggccaattgaacggtctggaacaagaggaacggttccggacatttaagggaaagattgtcctgacctatgatatcagttttcctttctattatgaagcggcgagggcaggagcactgggcattgtggccatatggcccaaggacattcatcaccacgacaccatgggcggtgtatggggaatgccgggaagcagggacagggatttgtacccttatctgccctatgtgcagatattggggcaggacggcctgaagctgattgagatggttaaggcgggcgctgcagccgtgggaaccgaggcggctaagggagtggaagcagccatgggaaccaaagcagccaaaggtatggctgtgacagctcagatggatgtggccatggacaaccgcatcgtaaggtccagtatgccggtggccaccattccgggcaaaagtgagagctttgtgctcctgagcggccactacgattcctggtatgaggggatgacggacaacggggcagctaacgtgctgatgctggagacagccagggcgctggaaaagtttaaggacaggctgaaccgcaccgtggtgattgcctggtggtccggtcattcggacgggcgttactccggctccacctggttctgcgaccatcactatgagtatttgagaaagcactgcgtggctcacatcaacatggatatctgcggatgcaagggaagcaatgcagtccgtttcgatatgagcggtatggagggagaggcgtttaacgatgaattccttgcatcctataacagccgcaaaccccttgcgtacagggctctggaccgttccagcgaccagaccttctggggaaccatgacccctgtatccattgctccccagttttatatggatgacggacagacgccccagcccccaaagagcagcgatatcttaaggccagcggtcatgccggcggcctttggggtgggcggccccttttactggtggcataccagggaggataccctggataagataggggatgatgtgctggcccgggactgtgagatagctgcaaggctggtgctgcgctatgccatggaaaagccccttcccattgatatgagtggtttcatgagggaaatgcagtcctattttgaggcctttgcagaggaactggacccggacttcgatgtggctccggtactggcatccattgccctgacccgaaaatccgttgagaagctctccgatgccatccgggcatatccaaagcaggatgcggacagcatactcatccggacagcgggagaactggtgcgcttaaaatatacgtattccagcccctacggacatgactatgcagtggagcaccagccctacgcagtgttttcgtccctgttaggagtgcacagggacaatacgcctgaggaccggtatctgatgtcgcagacggatttcatccgccagagaaacaggatgacaggccagcttcatgagatatgcgaggccgttgaattacagctgtaccgctggcaggtacaatag

SEQ ID NO: 22 - DNA, 1836 bp, Clostridium boltae
atgaaaaagggatttataaaacagaaaagcctgtccgtcatggaacggcttatgaatcaaagtctgaccgtaaaaatcagtgtttttatttatttaatcgtaatcattctatttttatttctctcccttttcctttttggcattgttggacgcgcatctgaacggcggctgtcagaggagcactccaaattgctgagggttgcgattcttatgattaacagccgccagcagtatatgatcggtgtggcagactactatgctctgtctcctgatatcaagaatatgatggataccagcaattccggtcttcctgttacaaccatcctggacgagtccaggttcaaaacccccacaatcatcattctcagtactgtgttctacaatgccgaaggcgaggctgtctattatactacaaaggatacctcccgggtgccaatcaatcaaaaaaacaacgatgccttccagaagctggcatcaggacaagccacctatgtatgggactatattgacaacaataacagtgattttatgaagtacgatttttcccccaagctgtgtctttggagagcggtccgggacagcaacgatgtccatatgatcggtgccgtagccgttaccattgactcccgttccctgcttggctttgacgaaaccgcaaaacagctgtctgaaaatctggcaattgtcaactcaagcaaccaggtggtctataaccgttccgatatcgatctgaatgaggatgatatacggctgttatccaacaactcctttggcagcgatgcaggcctttataccgctgagttaagcagcggcaggtacagagtcagttaccaggcaattccttccactgattttgtggcgttcttcctctaccgccatactccgtttgcctttgggattgatgtggtatacagctatatattagccggattgtttctgtatattctcagccttttcccatcaattatattggtttccaaaatgatcacaaaacccctggtaagcctgacaaaatccatccagcagtttgcagaggggcagcagaatgtaaaagttcagtttaaatatacggatgagattggactgctgggaaaagcttttaatgacatggttttggataatgaacgtcttcggatatcagaatacgatttgcgtttaaaaaataaggatgcagagctttccctgatgcaggcgcaaatcaatcctcactttctctacaatatgctcaatgccattcagtggcaggctctcaaaagcggaaacaaagaaatcgccgatattgcctattccatggcacaggtattccggatcagcctgagccgcggcaggagtattatttcagtgaagcaggaacttgatctggtcagctactatttatccctgcagaaataccggctgggtaaaaaaattgactatcatattgattttgatgaggatgtccttgaccgccagattccaaaactgattcttcagcctctggttgagaactccatcgttcatggcatggcaaaggattcttccctcaatctggtcatttctctgtctgttgccctgtcagaggatggaaaattgttacactttgtaattcaggataatggatgtggaattcctccggaaattctccggtatttgcccaatgaggtaatcccggctgcggcggaacagggtcaaagaccaaataaaagcaaccgttttgcggttaaaaacatttatgaccgccttacactggtatatggaagcgatttcactttccgcatccacagtgaacatgggacatccatcgaaattattcttcctgtaaaagagatagatgaaaggagcacctccaatgcttag

SEQ ID NO: 23 - DNA, 1836 bp, Clostridium boltae
atgaagcatcctgaactactaagtctgcacagcgtatcggatctgcggatctctcccggaacaagccgctgcgcgttccttgtccacactccctgtgaagcagaaaataattatgaaacccatctgtatgtcagtgattttaccgtgtcttatcccattgggatgtccggcattaccagctttgcctgggtagatgatgctgcactggcggttgggcgtcccagcgcagatagtacacaattcgcgcttttgtccctgaaggacggttcggaaggaaccgtctggaacatcccctttgacgccagaattgaaggatgggttttgggacagcttctcatctcagcccgccgcccaattaccgaggaaaaggctcaggaggatggatcgtggacaatcctggatgaacttcccatttgggaggacggcgagggataccgtgccaaaatccggcgtcagctttttctttgttcctacggcggccagcctatacgtatttctcctgaggagatggatgtccgtattgtatcagcacattcaaacggtctggcctatgccggatatatcctcgggaaccatgggaggatcgtcaatgagatccgctattgggccggagaagaccggttactccgcaggaactgcggtgatatcagacatcttgccctgggcagcaattatgcttttatctatgctcttgatattgagcgtgagacagactctgctcccgccctgatacaggtttccctggacaccggcaaagctgatcccctgtatgtttccggaattgcggttggcaattacattgtttccgatatcggcctgcaggggaaaattctatgcgcagatggtgatgctctctattttgccgccacaaaggaaggctcctcccagatttataaactgtctgcctcaggcgaaccgctatgcctgacccttgacccaggcagtattgaacagctggacgttcgggcaggacggattgtttttgctggtttgcgcaggggctcctgtcaggaggtctacgtcctggaggatggggaacaaatgatttcacacctacacggtaatgacacgcttcctttttaccctatggtggaaattccctgccatggtattcagggctgggctcttcgggaagaaacagaggaaaagacttgcccggcggttatatttcttcatgatggtcctcagcaggcatttggtaaagtgtaccactttggtatgcagctgcttgcccaaaacggctatgttgtgctgtttgccaacctgcccggcagcatgggctatggcaaagatttttccatgctggacggacacttgggagacgatgactgcaacggtcttatccgtttcctggacgctgctctggatgcctgccctgagatcgatcccagccgtctggctgtgattggcaccggctacggagcttatctggctgcggctgccacgggaaaatgtaaccgcttcggagccgcaatctgtgatggggtcatttccaactgtgtttctatggtatccaccagtgatcatggcattgcctttgccgaaaaacagatgaaagcctgtgcttttaagcaaaccggggaactgtggaaacgttctcctctcagccgcatcgcttccatgaaaacgcccactttgctgcttcacggtgagaacgaccgcagcagccatctttctcagggacagatgctcttcaccgcgctaaagattcatggcgtgccggccagattatgtgtattccccggagaaaaccacagccttgcaagcaagggaacacctctggcccgtgaccgttatcacaccgaaatccttcggtggctgaaaatgtatctataa

SEQ ID NO: 24 - DNA, 1755 bp, Clostridium boltae
atgaaaatagcagtgtggatggaccgtggaaaaatggtcagggcagctatgggagaaatcccctgtgacctgactgtctgcaatatacagctggtcaacatgttttccggggaggtttacccggcccaggtagatatactggacggcatcattgtgcgggtgcgcacagacaatgaatgtccggccctgccttcggaacggatttttgacgggggaggacgttacctgataccggggtttattgactcccatcttcatgtggaaagtaccatgatgattccggagaatttcggaagggccgtacttccctgggggaccactaccattgtcatggatcctcatgagattgcaaatgtgctggggattgaaggggtcagcttcatgctggacaacgcaaagaaaacacccctgcgccagtttgcgctggctccctcctgtgtaccctctgtgcctggagcggagaacagcggggctgtattcggcgaggaggaaattgcccgccttctggaactgccggaggtgctgggaatcgcggaaatcatgaattatgtggatgtatgcaggggggatgaaagaatgagccgcatcatatcccaggggctgaaacggaatctgtatctgcagggccatgccccccgcctggagggagatgcccttgcagcctacttgctggcaggaccggagagcgaccatgaatgccgcagtgcccgggagtgcagggagaaagtcaggcagggcatgcatgtaaaccttaagaccagctctctttccaaccatctgccggatgcactggagggaatcagggaccatcgctggcatgacagtgtttccctgtgcacagatgatgtccacgcaggggtgatttacagagaaggacatctgaaccgggtggtccaaaaggccataggctatggtgcccatccattagacgccatccgttatgccagctataacgctgccagagagtatgggtttgatgaccttggagcgattgccccgggttatgtggcggatatgcagctggtggatgccctggacggccgccggcccagccatgtgttctgcagggggaaacttgtggctgaagagggaaggtatctgggaagtccctacgacggaggactcaagttcaccaataccatgaaactgtcctatctgtccggccccggggatttcaggctgaaagcgcctgcttcccagggagagacgctggtgatatacagcaagtatgacggacccttcaataaggccttttatgagacgctgcctgttgaggacggatacatctgcatcaggcaagatccgaatctggctatggcatgtgtgtgcaaccggcacggactgaaccagaggaccgttgttcccatccggaattttggaattacggaaggagccattgccaccacggtatcccatgactgccataacctgaccatgatataccgggacccggaggatgcatggattgcggcggagaccttaaagagaagcggagggggcatagctgtggttctcaatggaaaggtgctggcaagcctggcccttccggctgccgggctgatgtcccagctgtctgttgacagcctggccccgcaggtggaacaggtggaaaaagcagtgtatgacctttgcgcgggaaagagctcgctgcttaagatgtccacctttgccctggctgccctgccgggagccattatgacggataagggcgtgctggacggacagtcccagacatttatgcctgttttccggtaa

SEQ ID NO: 25 - DNA, 2115 bp, Clostridium clostridioforme
atgaagatgatacggcaggtcctcacagtcctggttctgacaggaatgcttttcagtatgacggcctgtggaaaacaaaccaaaaccgaagcacccgaagcatcctacatcgcgagcttttttgatataccggatacggtggcggatatctcaaggctcctgataaaggataatacagcttatatgtgctgctttgaagaaagtggtatctcctatctggcgtccatgacggttggtgatggtgaatttcaacaactgccattagaagtggaggcatccacttccctgttagattttgcatttgattccaagggcagcacatgggcggtttgcatggatgataccgaccgctatagtcttaagaaatttaatcgggacgggcaggtaatccaaaacattgatttaaacgaggtattggaaaccacaaacgcggccggggccggcagggatttgttcctgagcatcgatgcggagggatatatctgtgttgcggaaaaaagaggaaatacatccgcatatatatttgatgataaagggcagtttttattcccccttacgtatgagggaagtcttctgaacacaataacaacggctgaagggaagattggagtctgcgcatcaacagcgaaccggatggattatgagctgctcacggtggatatgaaaagtcgggactggaataaggataggatttacctgaaagcaaccgcgggtctgtatggagggagcagcaatagcttctaccggtttgattcctccagcctgtatagctacgctgcaggctcacaggaaggcaggcatgttttcaactggtcggacgtgggacttagcgcatcggatgttcacttgggtgaactttcagatggaagattgattgtggtagctgcttcgcccaatcagactacggcatttacgtatgagatggcagtactttctcagggagtggatgagcgaaccgtcctgagtatggtgagcttgaccgcaggaccaggggtcgttcaggcagtttctgaatttaacaagacaaacagccaatacaggattgaacggacggagtattttccatttgagcaaaacgtgtccgacgaggaatgggacagtgcggttgtcaatctgaatacacggattatttctggtgatattccggatattctggatatgagtaatctatcggtccagatttaccatagtaaagggctgttggaagacctttatccgtatatagagaaggacccaatgctccatatggaggactattttgaaaatgtttttaaggccataagccttgatgggaaattaccttatatcacagacggggcagctgtatcaaccatgctggctgatgcagacatcatgaagggaagaaccgggtggacactgcaggatttggagaatgtcctgaacgcttccggatccaattccataagcaatatgtcgggtgcaccttttcttaaagtcatgctccagacggataacagctttgttgactgggcctcgggcaagtgttcctttgattcacctgaattcataaaattactggaatttgccggacggatacaggataacagtaaaaacgtctttggaggagaaaatctaagcggtacttatgcagcagcatatgaaaccatcctcagtatttaccagattacccagtatagggactattatcacggaaacctggaactgctgggccttccaagcagcagcggtgagtatcatgccctcaaacccgaagtgaaaatcggaatatcttcggccagcgggcagaaagacggcgcctgggagtttgtcaggacattattgacagaagagcatcagaagtcctgcagcatgctgccgattcatcaaggcgcctttgatacagtcatgcaggcagcgattgacggaaaatcaatctggacatggctttatgaaaatggaaaggcaacaacggaggatgctcaagtgacaaggcagcttctaagcaatgccgcctatgtggtaaatgacaatcagacgctggaacaaatcatactggaagaagcccgggagtacttttctggggcaaggaatgcaaaggaagcggctgaacgaatccagagccgtgccagcctttatatcaatgagcaaatgtaa

SEQ ID NO: 26 - DNA, 1992 bp, Clostridium clostridioforme
atgcgcttacatattgtagaaaaaatgaatatggttttaaaacagcaaaaaagcatgcttgcttctggagagaaatacaggcctctcatagaaaatcgtgtgcagcgcatagctgtacattctattgttgcgttttttacactgatttttgtatgcacaatcatatcccgtatttcccattcctttacaactgccagcatccatgtagcgaccctgacaagcggggccttaacggaccgggctgaagcagaaggaacgattcaagcagcatctgacaggggcattacgctgccggaggggcttaaggtcgtggcggttaagacaggaaaaggcagtcaggtaaacgcgggtgatgcactgcttgaatttgacgtttcctccattgaagaacaggctaagaaactggaagatgaaatccgtatcctgcaattgaaaatagagctttccggaagtgagggcggcaatgatgtaatcacggcccaacgtaatcttgaggatgccaggcaggcgtatcatcgcttatctgaaaaatatgcccggcaaaacacaagattacaggaagattattcaaagctggaagagaagctggcggctgccgagaccagagatgaaaaggctgtcgctgcaaccaggcaggaccttattgataaagcagaggcggtggttaaggaagcaaaagaaaatctggaggatatcaaagatgcggcagaggaggctatctatgacgccaggagagagcgagatgatgcctcagaccatctggatgcctcaagggaggcgtatcaggagttgttggaggcttataatcaggcggaacgtaatgttaacgatgcgaatcaggcggtgaacgatatcaaggaggcgattgcaaatcaggagcctggagacacctcggattataccgaggagctaaatgcagcaaaagaggagctttccaatgcaaaggaggaattgaaacaggccaaaaaggaactgtcaggagcagactataaaacttcgtcctatgacagtgctgcagataatctggatgccattgaggagcgctgggataacaggatagaaagggccagagataccctcagggatgcaagagcagcgctgacaaaggcaaagaagcgtaccgacttttctgacgaagccgcggtcatagaagcccaggcagcggttgaggccgtaaaggataccttgacagaggtcaggcgtgaatcagaagacaattggtatcagagagaagaagaactttatgaggcacaaagggcgattgaagcagcgcagatagcattggaaaatgcacagaagcagacggatgcgtcacagaaagaagatgaaatcacaaggattacctgcgggtctgaattggctgagaaagaaaaagcatggcaattgctgcgggaaatgttggcccatgatgggcaattgctggctccggcttccggaaccgtattaagtactgtgaaaagaggcgctaaaacagcagcagatgaggaggtagtcacactatcctgtgatgacagaggatttgtttttgaaggagtcctggataaggaatctgcacagcactttatagccggagacaagggggaactttcgtttcaagcggatggaagtacgcagaagatagaggtggcgattaattctgtcagtacatcggatgaggaggataaggtttttgtatctgcaattttacccgagggaagttattcagttggtctgcccgcacagctgtcattgagcaggaaaagcgagacgtatcaaagctgtctgcctattacagcacttagaacagattccagaggtgatcacgtgttggtgattcgcagacagaattctgtgatgggaacagagtgggtcactgcaaggattgatatcaatgtaaaggacagagacagtaaaatgatgagcgttgagagcgcgcttacttactccgaccaggtgataacaagttcaaataaggcgatagcggaaggagacagggttcgtattgaaaactga

SEQ ID NO: 27 - DNA, 1956 bp, Clostridium clostridioforme
atgctattgcctcgggaaaaaagaattctggagatactgtatgcaaaaaagcagggatatacatcttctgaactggctgcagctctgcatatcagcctgcgtacggtaaaaactgatatcaagagaatcagagaggaattagaaaagacgggctgtgagatactcacaaaagcaggaaagggtatatggctgtcctatgacagtcagggaaagaagtacctggacagtcttttgctgggaggtgaatgtgcttcatccatggatccgaaaaccagaaagtattatattgcgcttcaacttttggacagcgatacatatatatccactgaatccatatcaaattccatgtatatcagcaaaggaaccgcgaccaacgacattaatgagttgattcctttctttgagaagcagggtctgacactggaaaaaagggtgaaatatggaatacgccttcttggaaaagagagtcagttgcgcattgcaaaggcatctgtaatccgtaagattgtggtgtaccaggggagccaagtatcccggaagctgcagccattttttgaggatttaaatattgaccatattaatgctatcctacaggaggcagaggagcattttggcttcatcctttcagatgcttcctactcagaactgctgattcattgttccattattgtgagaagaatccggaagggaaaagtgtgcgccatagatgagacggagcttagggcatatagtgaaatgaaggaatggggcatctgcaggtttatagcagatgccctggaaaagagcttttctgtccatatgacggaaggagaccgctcttatcttatgatgaatctgctgggtacaaggatgcaggaacatatcccggcagagacatattcctggggggatgatggagcggactccggacagatactggagcagtgggaggatatactcagacacgccggagatatgtttcgtgagaatctgataggagatgaaacgcttaaaattgccatgtttctgcatctgaaagccatgtttaacagattgcagcaccagattcatctggaaaaccccatgaagcgtatggtacgggaagaactggtatatgagtttgaggtagccacctatgtggccaggctcattaaagaggaattccatgcggatctgggtgaagatgaaatatgtgatatcgcgctctatctgggggccagcctggaacgggaacgggccatgagaaaccgccaaagtcctgtggttaccattgtctgcggttccggaatcggtacttcacagttttttgaggcaaagctaggccggatttttccagagatacaggtgagaaagatagtacctatatcaagggccaggtatgagattggaaaggatacgcaggactttgtgctggcaacggttccgctggagctggagggcatagaggtgcttaatgtatctcccatgctgggagagagggacgcccttctgattgaagagcgaattcatccggagcgcagacagttgctgatatcaggaaaagagaagtatccggccttgtttgcactcatgagcgagcgtatatcaatctttaagtgtgactgtcgctcgctggaagaggtaataagccttatgggtcgccgtctgattcacgagaaatacgtaaaagagggattcattgaatctgtgcttaagagggaggaacttgcccctacatctatcggcgacaagtttgcggttccccatgcctttgagggatatgtgctgaaaacaggagtcggtctgatgacacttaaaaaaccaattgtctggggaaatgaaaaggtgcagattatcatgatgctgtccattgatataagagagcaggagcaattcagggagatattttccgaactggcagcaatcacaaaaaataagtgggccattgaacagattcttaacgctgaacgcatcagtgatattaaaataaggaactaa

SEQ ID NO: 28 - DNA, 1947 bp, Clostridium clostridioforme
atgtcggaagtgaatgaagcgacaatgattgaaaaaacgaaaacagaaatatggattgataaagcggttatcgtgattgcgattattatgagctgttatcaactactggcggcaaatttcaccatgctgtctgcagagcagcatatcaacttacatattgcgttttctcttgcaatcatttttttacaggctattaagttaacacaaacaaaagataaagcgcgcagtgcttttatgattatccttcttgtggcaagtgtagcggctgctacctacatccactttaatacaacaagatttcagatgagcattggcagacagccgtttgataaagtgttctctggagcagtattcttagttgtcattttgattgccactaagatgacatggggttgggtaatcccggttatttccataatcgcgttggcatatggatattttggaaaatatatgcccggtattttttatcactctggtttaagcttttcccgtttgatcacatatgtaacaacaaactttaccggtgtgtacggtatgcttgcatcagtatctgcaaatacgattgtgttatttaccatctttggcggcttgatggaggcatttggagcgatcagcacaatcatggatgctgctatggtggcatctacaaaaattcgttccggcggagcgcaggttgctgtaatttccagtggtctgattggttctatcaccggaagcgtggcagcaaacattaccttgacaggcgccgtatcaatccctctgatgaagaaaagaggatatccctcggagtttgcagcagcatgtgaagcggcagcatcgacaggaggtgcgattcttccgcctgtcatgaacgcggcagctttcattattgcttcatggacaggaattccttacatctacatcgttgcagtcggagttgctcccgcgttactgtattatcttggtattgcgctgagcgtatatattaaagcattaaagctgggagacgagaaagtcaaagcagaactgctcccacagtttcataaagcattcggaaagctggcaatgtttgtcgttccgatcattgttctggtagtattgatggtaatgagctattctccgcagaaagcattattcattgcagtattcacattaattgctatggggcttgctatcgaattgatggacaagagtaatagaagtccaatggactcctttaagaaatttatcacaaaagttctgtctggatttgaatcgggtgcgaagaccgttgcaggtattgcagtatgtatggcaacgatgggatgcgtagtagaaatcctcacatccacaggactgccgtctaaaatttcgcagtttgctttgtcacttgcaggagataatttatttgttctggcaattttagttatgattacctgtttgatttttggtatgggtatgccaagtggttcagcgtacattttggcagcattattaggtgctccggcattaactacattcggaattccgattattgttgctcacttcttcgtattttactttgcggagttatctgcattaacacctccggttgccatcggatgtctggttgcttctggtctggcagatgcaaagttcttgaagacgtgtatcgtatcaatgcgtttggctattggaggatttgttcttcctttcttattcctgtatagaccggcattgcttcttcagggacagtggtatgaaacgatttgggcagttttaatggtaattagtttcatgttttcttttatcattgcggtcgagggcttcttcctgcagaaaacaactgcatttgagagagttattgctttagtcggtgcattgtgctgcctgcttccgatttacgttttagattttgtcggacttgctctggtggcagcattgattgtactgcatgtgattcgctttaataagaataaagtacttgtcagacagggggcagaggtataa

SEQ ID NO: 29 - DNA, 1854 bp, Clostridium clostridioforme
atgcataagagaaaaattaatataagaaaatacaagtatgagatttttttgtatgccgcgtttgttttaataaacagcattccatgcctttttttgactgtgcctgtttttagcgatggattgaatacaatcgcggtaccggcttatataagtggctgtgattggactaaatatctgtatgcagacgggtattattacaaatatggagtgacgattttatatttgccattattttatctgttccgttccccgattgtgctgtatcgggccatgctgctgttgaatgttttagcggcaggggtaattcctgtcatcgcatatagaatatccatggattatttggatatacaaaaaaaggaaaatgcatttctcatagcaggcgtaaccgcctttttgccggcgctaacattgaatataaaatacacatgggcggagaccgttcttctggtctcgccttggatgatcctccttcttcttctgagaatccatgaagataaggatgccgggaaacaggtaagggacagcatcttaattgcgtgttcctctgtatttgcgtatatggcacatcaaagaggcattgtggtggttttggccacgtttctgaccgttgtatacatacgttttgtgcggaaaaaggcaaatctgagaatcggagtttatctgattacagctatggttttgctgattgctgacaggttggtggacgggctggtaaagcagtatgtattcaatgcgggtgtgaacacggtaaacagtacattttccttttgggatgcaaacatgtgggagagattgctgtcctttaccggccttcaaaccataataaagattatatacggctggctatttaatgtgtttaccggcagcggcggtcttgtttgtctggggctgtgtgtcaccttggtctgctgtttcagatacaaatccagtgaagggggatgctgcatccatttgattagtgtattttcccttttatgctttgttggtgcatttgccttgggaggtctttttttcttctctgatatttatctgtattataccggagaaatggttagaagatgcgacaagcttatttatggaagatatctggagtcttccatatcgataccggtgttaatgggcatgtatttttttctggagaaaggctctctttttataaaacgcagaagatatatctttttaatcatgggatcggtatatttattttttcttgttaatatcgcaggcaaggtgaatggggtggttacatggcccaataatacgatgactattaatatattctgcaatctggcccagtgcagacatggatacggtgctatccgtaatctgtcccaggggctgaccgtctatggtgcattggctatcgtaattcttatgtcaatattcgtatttcataaaaagcagagaatggcttgtatgggattgatagctgtttttatttcaatctttgtttggagttcctataatgtgatttaccggatggacaaatatgagatagagaacatggaaatgacaagaaacctggtaaaaggtcttgagcagcttccagaggattacaaagtaatttttttggacgatgagattaccagaagctcctatcagtatatgttccgtgattactatattgtgacaggcagggataataataggacacagataaaagatatgataatcgtctctcccaaaggagtgataaatgaggagttggaccagggagactattttgaattagtggatatggaaacagaaagtccggattaccatttgtatatcaaggggcgggacatgaatcaatggatgaaccaaaatggaatccggacaaaacagctgatatcagggggaaggggacagtga

SEQ ID NO: 30 - DNA, 1689 bp, Clostridium clostridioforme
atgaaacagacttttatgaaactgaatctgtcctgccgtctgtttctgatcattatcgtactttttctgattccctatctgtcccttttttcctgggcttacaggaaagcggagatcattatccgtaccaaagctcagtccctggaaaaagaaaacctaagccagacaagaaatgacattgagaacctttgcttaaacatagccaaggcttctgattacctgatctccctggatcattacggtgtactctatcgtgaatcagaacaaaagggatatgcttatttaaaatgctggcagtacgtagatgaacagatccagaatgcaaataacgccctgttaaactccagtgcagatatcagcgttctttccaaagaccggcttttatactccacactttcttaccagaaattccggtatcaggattttttcagagaacaggtcgtttccactacatatttttcaaatgctcacaaaagttatcgcaattttgaaaatgaccagacttttatttcctatatcagagaacttccatccttctgttctcagtcatattatctggtgatctccattccggcaaacaatttttcaaagcttcttggaactgctgccggaaccatggaactgacggattccgcgggcaataccatctgcggagtccgttcaccccaaaataacgaaagcttccgggaagaaacctccatctccctctccggttggaaattggaagataccatttccacagattttctctacagggacatttaccagctgcgtctgtttacatttgctgtatccttagtattattaatggcatgccttctggtaacattttctgctatttacgctcagttaaggcctcttttaaagctgaaagagcaaatggagctggtgatgtcaggcaatctgaatgcggaagtggccaccaccaattccagagacgagatcagcagtctttctcgtacctttaacaacatggtcaatgaaatcagccacctgatcaatgaaatccaggtcactcagaaaagagaaagtgagctgcgttttgaaatgctcttagcacagatcaatccccactttctctttaataccttaaactctattaaatggatgtcagtggtatccggaacagaccatatcaccacgaccataacctctctcggacgccttcttgagatcagtatgaacaaggttaatgatgtacttccgcttggcgaagaactggaaaatataagaagctatatccagatccaacaggtacggtatccgggacgttttgatgtattttaccatatagatgattcccttttagactgccgcaccttaaaactgatcttgcagcctcttgtggaaaattccattctccacaacattgagcaccgcgattatctttccattgacatttccggtaagctttctgaggatcttattatcctgtgtgtaaaagataacggaaccggtatgacaaaagaacagatggaacagatcttaaagcctaagacacatgcagaaaaaggctatgttttctccggactgggtgtatgcaatgtagaagaacggatccggcttgcatatggccctgattacggattagaatataacagtgacggctattcctatacggaagtaacgatcacttttccccgacaccagaaatcagacccattattacagaaagaagcaaaacaatga

SEQ ID NO: 31 - DNA, 1650 bp, Clostridium clostridioforme
atggcaggaagtgcacgggacattcagatgcgtgagctgaaggacacgatatcagaactgaataagctgattaaaacgctgcagcagacgattgaagctgctaatgcgcgtgaggccgccctgtgccaggaacgggataacctaaaggaacagatggactatctgacaaagcgcctcttcggtgcatccagtgaaaagggcaaatgcgatattcctgggcagctgaatctgtttaatgaagcagaaacagcagaagatccagtggccgcgctctcagaagaagcgcttccctcctgggaagaaccagaagcaaagccccgaaagaagcgcgctgccaacgaggaacgcttaaagggcctgccagttgagcaggtatttcttgacgtaccagaagaggagcgtatctgcggtgtctgcggcaccctaatggaaacaatcggaacggaattcgtacgccgggaactgaagttcattcctgcaaaggtaaaggtcattgagtattacagcgtgaattatggctgcccgaaatgccgcaaggaggctgtcctccctcagatcaaaaaggggaagggtggccgggcgcataggatccatgggatggcgagtacatctaccgtggcatggattatgtaccagaaatatttcaacggcatgcccttgtaccggcaggaacgggattggaaacagtgcggtgcaaacatcagcagaacaaccttcgccaactggattatcgcgaatgcacaggattttttcactcccatgtatgcctacttccgaaagaaactgcttgcacggtcatttgcgatggcggacgaaacgccagtccaggtgctgcacgaaccagggcggcgcgcgcagacacagtcctatatgtggctgttccgcagtggtgaagatgagggtccgccaatcatcctttataaatacgctccaacgcgcgctggagacaatgccgtggaattcctggaagggtacagtggatacctgatgtgtgacgggtacagcggctataataaagtgccggatgcaaagcggaccgcatgctgggcgcacatacgccgatacctgattgatgcgattccaaagggaaagcagcttgattatacccagccatcggttcagggagtcatgtatgtcaaccgtctctttgaaatggaagataaaatccggaagaaacatgccggggactatgaagccatccgaaaggcaagactcgaaaaagagaagcctgttatagatggatttttgtcgtggctggagcagcagaaaccgacacgcggctcccggctggacaaagcgattacctatatccggaacagagaaccgtatctgtccagatatctggaggatggaagatgcagcttttcgaacaatctaagtgagaatgcaatccgcccatttgttgtaggacgtaagggatggctgttcagtgacaccccggcaggagccgaaacgagtgcggtcatctatacgatggtagagaacgcgaaggcaaatggagtaaatgtctaccaatacctaaaactattactggagaagcagccgaataaccgaatgtccggtgaggaattggaacgctttgcaccgtggaatccagaggtgaaagcccttctggattctcgggttaccgatgaacctgaaaatggctga

SEQ ID NO: 32 - DNA, 1500 bp, Clostridium clostridioforme
gtggaatgtaatagaacaaagctcagcagtgtattgtcttatataatgattattgtaaacataacatctgggcttttttttacgccgtggttaatgcatcgtttgggaacttctcagtatgctatatatacattaggcatgtcgattatcagctatttgaccattgagcttggaataagtgaaatagtaaccagaatcagtttaaaatatataatcgaaggcaaccggcaacaggtaaacaggttgatgagtattgcaattagaatttatctgatgattgatatactcattctgatattagcaattgtgatgtacttttttatagattctttttttacaaatttgacactttcagagattgatttatttcgtaatgttttcattatatgtgctgcaacagtaatagtcattttctgggaaattccattcgaaggtttgtatgccgcatatggaaaaatatatgtaaatcgcctcgtgggtttaggatataaattatcatatgttttagttactgtcattagcatttctctttataattcggttattattgtcgtactatgttatgcagtgttgacaattagcacaaaagtatttttgtacctatatataaccagaaaaaataatatagtaattgacttacatacccatgacagagagattactaaaaatttactaggcatgtcaggttggattattattgcaatagtttcaagccgatatttttatgcaattataccgaccctactgggaaggttctcaaattcatttgagataacaacattttctgttgcaagcgctgttgagggctatctattccttttttctaatgctctaaatggaatttttttgccacgcattacgcgaatggcaatgagtaacgatgatgaaggaattaccgacttgttaattagaattggaagaattcaattaatgataatttcttgcataatcatcggaattataggatttggacaggagtttatttctttttgggttggaagtgagtataaaaatgcatatgtttgccttattttaattttaataccatgtattgtacatttgactcagactgtagcattagaggccacatttgcaaaaaatcgaattcgggaaagggctatagtttatgctgttgggactattattagtacagttcttacatgtattttagcacctgaattcggagcaataggagcagcaataggaatatgcgtggcagaactattatgttatgaaataggcatgaactttgtgtataaaaaaatgcttaatattaatataagacacttttttgtacaaacacatttgaagctattaccgccgttaataatatcacttatgacggcttttgtggttaatcaattaatagaagaatcaacaattatagtgtttctaacagaagttggaatatgggcagcgattcatttgattttactgtataccttgggatgcaatacatcagaaaaagatgtgattaaagccatcctgatgtatagatag

SEQ ID NO: 33 - DNA, 1497 bp, Clostridium clostridioforme
atgaaacacatcaaaccactattgctggcaggagtagtttcgtttgcggtaatgggctgtgggaaatcaccggctccgcaggaagaaacatctgtcaaggaaacaattgccgccacggaaaaggaatccgtggccgcgaaggatgaagcccaaacagttaagcttttgaaggcggacgcgctgacggatgatatgcagctggtagacgtccgtgaagaagaacagtatattggctggaatatcggggataaaccagggggacatattgcaggcgccgtggattttccggcaagctggctcagtcagagcccggatacctatgcaatcagaacgacaatggaaaacgaattaaagcgccgcggcattgattccgaaaaaccccttgtcctttacggagatgatactgtaccggaggaaacagcttccatgtatgcggaactgggatttaaggacatctctgttctggaaggcggcttctcatcctatttggaaacaggcggggaagcggcaatgctgccgggattcagcctctatgtatatcccgactgggtacaggcactgatagacggaaaaaagccggatacgtacgagggttccgattataaaattattgaggtctctttaagcagtgaagagggagaatacgaaagcggtcacatccaaggcgcaatcaatataaaagacactttcaaccatgttccggggcttcgtgtactttctgaatatgagaacataccgatggaggaacaactgaaattctggaattgtccggaagattccgtgattcaggaaaatctggaaaaggccggaatcacgcagaataccaccgtgattttatatgccacaacaccggccacttccgccgcgcaccgtgcaggggtcttaatgaaatacgcgggtgttaaggatattcgtttcttaaacggcggaaaaacactttggaaacttcaaaacaggcctctggagacagaatccaatataccggaaaatgtttcctttggaacgaaggttccgtctaatcctgaccttatttatgactatgatgaggaactgggatgtgtaaacgacaatcaggcggtcattgcatccatccgaagctggaaagaatatatcggaaatgtcagtggttatacatacattggcgaggccggggatattgccaaagcgcgttttggttatgccggctcagacccttacagcatggaagatttccggaatattgacaatactatgtttaactacgaaatgattaaggacagatgggtaaaatgggggattgttccagataaacgtatttctttccactgtggtaccgggtggagagcaagcgaaacatattggtattctctggcattgggatatcctgacattcatgtgtatgacggaggctggtatgaatggtccaaaatgcctgacagcccgaagaaagaaccaggagtgcccgcagacgcacctgaacaggagccggcagaatactttataccaaaggaaaagtaa

SEQ ID NO: 34 - DNA, 1392 bp, Clostridium clostridioforme
atgccgttaataggagcagtggcagatgatttgaccggagccaccaccaccggcgtgctgcttgccaggtccaaggcaaggactgccgtttttttcaacgaggaggccgcggagcgggaaggggaggctgagaccctggacgccatactggtgagcagcaacagcagggcgctgccggcggaggaggcatatgaaaaggtaagctccgccacccaggcattaaaacggatgggggtcaggtatttcagcaaacggattgacaccacgttgagaggaggtatcggtactgaaatcaaggccatgatggatgtggttggaggggatgcggtggcagtggtggtgccttccatgccccagtccaggcggattgtggtaggcggcttctcggtgattgacggcattgccctgacaaagacaccggtggcccaggatgtgcgcaccccggtgcatgagagctatgtgccccagctattgagcaggcagacaggggaggagaccggccttgtcacgctgaaaacagtccttttggggcgggaggagatagcccgcgcccttaagtggcagagggagagaggaaaccggatcatagtggtggacgccataaccctggaggatatccaggagatagcccatgcctgcatttcgctggattggaatgtactggcagtggacccgggggcatttacggcaaagctggcatactgcagagggctgaccgaggaagaacggcccaatgttccggaaaagacactggacggcacgggcagaaccgtgctggttgcagccggaagcgccacacctgtgacaaagcggcagctgggaatcctgctggaggaccagcgccatgtacaggtcagtgtggaccccatcccgctgattgacggagcatgggaggccgcagaggaagcggagtcggccgtcaggcgtattatggagctgatggaaggagcgtcagcgcccagggctgtagtgattgagacggcactacacgggccggttctgaacctggcagaggaagacgccaaaaggggatatgcggacggcatgagcgccaaccggattaatgcagggctggggaccattgtgcagaaggtgctggagcgcgctggccgggaacggattgccggattatacaccaccggaggggataccatggtgaatgtctgcttccagctgggggtggagtgtattgaggtgctggattacgtgattgcccagaccgatgtgggacgcatggtggggacataccaggggcttcccatcattgggaagggaggactgacaggatacgacaccattgctgttgacattgtagaccgcttgtttagagaggcagccagggaaatgcagggggatgccgtgaccggcagaccgcaatatcaaatgaaataa

SEQ ID NO: 35 - DNA, 1383 bp, Clostridium clostridioforme
atgatgaagacaatcatcagacaaggcacgattgtgtcaccgagtgaaatttatgaggcggatatactgattgacggagaaaagattgcatgtataggaaggaatctggaatcagaaggagcaaaggtcattgaggccaggggaaaatatgtgattccgggaggtgtggatgtacatacccatatggaccttttggcaggcaattcacgggcggtagatgacttttatgacggtacggtggcggcggcctgcggaggcaccactgccattgtggaccacatgggatttgggccggatggctgcaatcttcattaccagctgaatgaataccatcatctggctgacggaaaggccgtgattgactatggatttcacgggactgcccagcatgtgaaccaggatattctggacgagctggagggaatgatggaagatggagtgtccagcgtgaaggtatacctgacctatgacaggcgcctgaatgacggggaggcccttcaggtcctgaaacgcatgaagaaactgggaggcgtgactgcatttcactgcgagaaccatgaggtggtggaatactatcggagcatgtacagggaacagggctgtaccagtccgtactatcatgccaagagccgtccaaatctggcggaggcggaggctgtggccaggattctcagtctggcgcgtctggcaggcgatgcacctgtttatatcgtacatctgtcctgcaaggaaagcctggaggcggtactggatgcccggaagaaggggcagaagaatatatttgtggagacctgtacacagtacctgacactgacagaagaacggtatatggataaggacggcctgaaatatgtcatgtctccgcccctgcgcaccagggaagactgtgaacggctttgggaagggctggcggctggtgatatacaggtagtggcaacagaccactgtccatttaattacggcatagagaaacagctgggcagggatgactttaccaagtgtcccaacggggcgcccggtgtggaggagaggatgtctgtcatcttctcagaaggcgtgatgaaaaaacgaatcagcttaaaccgttacgttgaggctctgtgtacaaatcctgccaggatatatgggttttatccggagaaaggaattttgcagccaggatcagacggagatttggtaatcattgaccccaataaggagtatgtgctcacccatgaccgtatgcacagcgcggtggattataccgcatacgagggtatgaagctaaagggacagatagagcttgtgatgcagaggggcagcgttgtggcggaagggaatgtatttaagggaaaaagaggcgcaggacggtttattcacagacggccacatgataatgcgtaa

SEQ ID NO: 36 - DNA, 1374 bp, Clostridium clostridioforme
atgaaaatgcgtcgatggaaaccagtagtattttatgtttcgctggcactcgtattgctggtttccttttttggaaaaaaactgattggtgataatcattatgagattaccttagctgctgttttactgtttttttcaatacttaactggattttagaaacagtatcgattgcggttacttcattaactttggtagcacttgtgcccttgagcggtattatgagcttttcagatgcaattgcaggaagttttggaaattcaatttttgctttcttcctaggggtgctacttttgtcatttgcatttaaacacacaaatcttggcaggttgatttctgatattatttttaaaatatttggaagacaacccaagcgggttgtgctggggattatgctgactggagcacttcttgccatgtgggtaacagaggttgcagctgcagcaattgtatttccgattgcattatctatttgggataaagctaaggaacgcgatgactatgcagcaataggaaaagcagtgatgctgggagttgcttggggatgtgcatttggaggcgttgccacaccgatagcaaccggtgcaaacctgattgcagttaattacttggaaacttattgcgggattaagattacatttggtcattggatgatgattgggattccgatttgtttcagtttgattcttgcaggctggtggattttgacgttacctttaaagagcactgtagaattgggaacggatagtgaagcgattgaatttggaagaaaggagagaaagctttcagtgatcttcgccgttgcaattctaggttggatttttggagataaaattggacttggaagtcatcaggtagcaattatttcggcgattgcattgtttttaccgggtattgaagtaatcgactggaagacaggaatcacaaatatcagttggaattcgatctttttgatttcagcaggtgttttgattggcgatgttctgtattcctccggtttagcggaaaagatggcaaatatattttttgttccatccttacttgaaaatggtattttgataagagatatctatattgttatttctgtatctattttaaaaatattattctcaagtaatactgtttcaggagtagtgttggtgccgatcatgctctcggtagcggctgcaaatagcctttctccctggggattggttgcgccgtgtattttttcatcagcattgtccctcattgtggtttcatccagcccagtgaatgttattccgtattcttcaaaagcattttctccgaaggatatggccttgtatgggattgttatgacaattatgactgcgctgattatcggtggatggctaacggtttttggggtgaattaa

SEQ ID NO: 37 - DNA, 5229 bp, Clostridium hathewayi
atgaagagagcagccgcatgtctgcttgcattgtgcctggtcgtacagggaccggcaagtctgatgaccagctttgctgatttcgggcagagaggagtggcgtcaccgtcgaacagcgtatcggcgagtccttctgatgcatggaaagagagtgacagcgacagtaagaatggggaattaaaggtagaaattcgtggagtccttcctgtgcagaaggccgcggaatgggaattgtttctgacaaaggacgaggaactgaccgatcagggttcggtgcagtatgaggccgtggaatcggccggggtctattcctccggcagttacacatttacagaccttccgaaggggaagtatcagcttcaggtgaaggcggtaaatggcggttatgaggactacatacagaaaaatatttcaattaacggtgaccgggcgtcgattctgcttttaaacgactacccggacaaatacggctatgccggggataaaatgcccggtgtaatccggatgggtgatgtgaatggtgacggaacgatcgacagcgatgatatggaggctttcattgacgccattgatgaagcagacggtaatttcgcagattccaggttcgattttaatggagacgggcagatagatcttgtagaccttcagtattttaccatcttctataaaaataagagcaatacaaaggcgactgtaacgaggcaggccctggtggataccgctgctgttgttgcgtcatccagcaatgcgtcgttctccgaggagacgctgaaggaagtatttgccggaaatgacagcgaggcgttgacgcttacagcggagacggcgatcacaccggaaacgccaattgagatcaccgcagacttgggacagagcttaaaggcggaaggatttacaatccagccggttacaggttccggaaacaccatcaaagacggctgggtcacggttgaattggaaggcgaagagaagcctgtcgtattcaggattgagaacggcgtggcggaaagacagacagggacaaggatgcgcgcggcctttagaagcgcgcctgaggattccgccgctggtaagaccattgtcatcgatttgggcaaacaggtggcgatcaagaaggtgacgatcaaagtgacggctgcattagaaaaggaggccactctggtcgagatatccaaggtggaattcttaaatgatatggagagcagaattccggagccggagatgaacatcccggaggacttaaaggctgtggcaggcagcgaatcctttgatttaacctggaagcgcgcggtaaatgtaaccggctatgaggtcgagattaccggtgaggtaaaaggcggagtcaagtctgaggtgctgtcggtatcggacaaccgtttaagcgtaaagtcaataaaaaatgaggacctgataaacggaaaagagtataccgtgcgggtgcagtctgtaaacggggcgtggagaagcggttacagcacggctgtgaaggtgacgccggaagcctccaaacggcctgatccgccggagggaattacggtaaagggcagttaccgcagcctcgatgtgtcctggaaaaagatgaaggatacggatacgtattctctgttttaccgggaatacgatgatgccgacggtaaatacaccagaatcgacaacattgaaaataccagccagatgatccagaatctaaaggatgaaacaaagtacgatatctatctgaccggtacgaacaaaattggggaaagtgcgccttccatgcactacagcggaacgaccgagagcgtcaatgcccccataacgccaaactacaaactgatcaatgtggcaggggagaatggcggaaccgaacatatcaaggcggtaaacaatcacggcggaaatgccgacagtgagtttgcgattgtggacaacgatatggtatctgcgtgggtgcgcaacgactgggatgcgggctgcgtttacccgggagaatcaaaatcaccaacggtgaccctcgacgacagctatacgatggacaccgtggtccttattccggatccggctcagaagtttgcatataccaatgcgaccttcttctactggccggagggaagcagcacacaggtgcaggcagcaggcaccttcagcagaaaaaccagctctaacggaaaagtatattatgaattccagacgaaacagccggtaacgacagaccgggttcaggttagactgacggcaggatacggtgcggccaacagaatcagcattgcggagatgaaattctatcactacgatccgattgagcatgaggtatacgatctgtttgcagacgatatgcacatttctttgaaggaaggggtgactcaggagcttattagcagtctgagggcgcgtctggatgagaaggatgaggtaagcggggaattccatccgaagaaagagattctggagagagaactggatacggcagaacagcttttaacggatgaggctctggctggaattcttaccatagataatcacgtaacgaaaaatgcggacggcaatattacttttaaaggcggattaaacgcctggcagccgcttggcatcacagccatggccggagacacggtgctggtctatgtgggcagcccgtccaggaagactggagacagcacgaatctgcgccttatagcgactcagtatcacggggaatccagcgcatggtcgaacacgatcggcacgctgaaagcgggaatcaatgagataaccatcccccagatcactgccctcgacgtggagcagggaggacagctttacatcgaatataccggtgatcaggatatggagacctacagtgtgagagtcagcggaggaaatcacattccaacgctggatataacgagagcttccgattccaatgcaaagagagccctggtgacgaagtatgtggaagatctggaggccagcacagcggagctggaagcaaaccatgagaaccataaaaaagcgcatgacggagactggagcgctgcgcggaaaaactgtattctgggcgccacggatatcgtaacgagatatatgatgtattccgtttcctcccagcagatactcgccggattatcaggcggaactacggaggaaaaggcggagcagctgtatcaggcgctgacggcggccgatgagatggtaaatctcttctaccagcacaagggactgagcagcgatcctgatgccggagtgaaaaataaactgccggttagccggctgaatctgcgctaccagaggatgtttgcaggcgcatttatgtatgcgggcggactgcatatcggaatcgagtggggatccgtaccgggccttaccaagtccgtaccggtgaagacaacgccggaaggcaaatacgaaagcggccagtactttggctggggcatcgctcatgagatcggccatgaaattaatgaaggcgcatatgccatagccgaaatcaccaataactacttctctgtgctggcgcaggcccgtgatacgaatgacagcgtgcggttccagtatccggaggtttataagaaggtgacgtcgggcgtaacggggcggtcctccaatgtatttacacagctgggattatactggcagcttcatcttgcatacgatatgggcggttataactataaaacgtacgatacgtataaggaacagttcaacaatctgttctttgccagagtagattcctacgtaagaaatccgggatcggcgccgaagccgggcaacgtggcgttaagcgtaagcggagatgtggacaacaagctcatgcgtctggcttgtgcggcggctgaaaagaatattctggagtttttcgaacgctggggtatggtgccggatgagaacacaaggaagtacgcggagcagtttgagaaagagacaagagcgatctggtttgtaaacgatgaggcaagggcttacgtgctggagaacggcaaaaatggttctgtggcagccagcgccacggtcgaggctgacttaagctacaggccgaattccaacgaggtgacaattcatctcggaagccagtcgaagcagccggaggcaatgctgggatacgaaatctaccgttccgaaaccatcaagagccatgtagagaagaaaccggtcggctttgtgaccgcggaccagacagaatttgtcgattccatttctactattaacaacagagttttcacctacgaagtggtaggctacgataagtacttaaatgccacaaaaccggtggtactggagccggttaaagtctcccacggcggtgtgattgataagtcagactggaccgtgaccacaaacatggtctcggcagaggacaaagtggatgaggagataaatccggatgtggtaaccatggaggccatcggaaaggtcatcgacaacgatgcaggaaccacctatacaggaaagacggtagccggaagtaacggaaaagtacctgcggcctctgtcaccattcacttaaacagagaagagaccatcaccggtttcacgtataagctgagtaaggcggataacgcggccggaagtccgatcggcaattttaaagtggagatcagcgataccggcgcagatggttcctggacccaggtcaaggccggaaccttcgccgtagcgcagggacagctggcgaacggcagtcagaccgtctattttaacaagaatgacgacacctggctgtatgcctatgacacctcatacgtaaggattacggcggtggaccagaagggaaccgatatttccatttcggagattgatctgctggggcagaccggagacgacatcgactttggtcagacggattcgattggccttttgaaagaggattaccatgccggacatggagagagcggcgaggccgttattccggcgggctccctcctgttcacaggaacgtataaagggaatccggcgtacaatgtggtcctgctgtatgatgagcagggaaagattgtgggcggtaccgatgcagaaggaaatatattggcagcacagatgatctttgcggaagtgccggagcacggagagctgggcgagaccagcagcggaacgtggatctattacattgaacccgaaaaccttaaaaatgccgctcttccaaaacgtgtgagagcggagctctaccgggtagacaacgcacatgacaacaggggagaacgtcttgtcagcaacactctgtttgtcgatgtgccggagacactgccggagatcgagataaaaacacaggactga

SEQ ID NO: 38 - DNA, 2454 bp, Clostridium hathewayi
atggaattaacgtatcagatcggatatgatgagacaatcagcagatggaatgtgacagccatggggaaagaaccgttccattccccgaagaaaacctttgaggccggagtgaacatggaggaatcttatgttcaggtggtgtatccggtcagggaagcctttttaaaggaagaaaggatcaggaaggcggtccggtatgacggatcatatgaaagtctttattttccatttgagaataacagaattgatttatccacattttttcacacaccccagtacatttacgttcatgcgaaggcgggagtgcgtgtgcaggaagagggatgctatccatttgagatctatacctgcggcggagtccgggtgtgggtgaacggagaggaacaggcctgctatacgccatataccagaaacattgcgggccatacccgggtgaatctttctctgaggaagggactcaatgaaattaaggtttacgcagatgagctggcggaacgggacgtttttttctattttgaactgcggtataagggtgtaacgccagtggaaggcagtgtggaagtgacagagcagcctgagaagatccaaaaagcggagcagattttaaaaagctgttattttgagcaggatatgtacacggaaggagaggtcaggctttgttacgaccggacgcttttagacggcgatacaactgtgtacttgacttcaactccctgtggaaccggaatgcagctctccgaaatagaacatacggtgatgacactgaaaaaagataaggattacctggtggttgcagagacagagaaaagcagtatcaggctttcgcgaatctccgtctgtttgacagtagggggctatgtaataccgcgcaatttatttgtcggtgtgatcccgaaaaaacggattgtactggaaccggctggaacgattggggagaggaagcagcaggctctggaattcctggtaaagaacggtgagatcggttttcagtctgtgattacttcgctggaactcttaaagggctggaatgacaatgcagaaaaagggtttgatatggcatgtaaaaagatcgagcgccatgatgactgtgccgatttcagcctcgccccctttagccttttgatgacccgctataagcatctcctgacaccggaaaagttggaacggatcagagatatggtgctgaacttccggtactggattgatgaaccgggaaatgatgtgatgtggtatttcagcgaaaatcatgcctttctgttccatgtttcccagtatctctggggatctgttttcgagaaagaactatttaccgtcagcggcaggacgggagcagagcagtacgaaatcggaaggaaaagggtgttggaatggtttgacagctttttcagctatgggtatgcggagtggaattcagcaacctacattcctatcgatctgattggctttttcagcctgtacttaagcgctcctgatggggaaatccggcagaaagcagaaaaagcactggattttaccatgcagatcatcggatataactcttttgaaggtgtgatgaataccacctatggaagaatttacgaagaaactatcaagacgcggctccaggttgaaccgaattttgtgagctgggtgtctgccgggcggggcttctgtacctattacggcaatgccacatgtctgtacgcgatcagcgattacgagccggaggactatgaaatggagtgcaggccccagccgggccagggtgtggtgatggaaatggatcagggaatcgcgggagtaaagattcatacttaccggacaggagagtacttaacggcaggagtcagaaggtttaaaccattccgccatggccatcagcagcatctgatgaatgtggtattcggaaaagaacgtccggcgattttctatgttaatcatcccggagagcgggttttcagcggagaaaaccgtcccagctattgggcgggcaacggaacgatgccgtggattgagcggtactgcaatgtaacggttatgctgttcgctatcgatcctgatgaactggtgcattatattcatgcctatacgccggtctatgagtatgaagcgtatgtctgcggcggaaactggttttttgccaaatccggtgacggatatctgggctgctggttttccaacgggtacgagatggctgcatatggtgccaacacgaaaaaagagctgatatcagaaggattgaaccatgctgtgatcgtaaaatgcgggtcgaaggaggaatttggaagcttcgaggtgtttcaggagaatttaaaagagatggatatcgaatgggacggggaccgcagcattgcattcgcagatgtgcagtacggtgaaatgcgggtaagggatgcggaggaatttctggtgaatggtacggcagttggtgtggaaccggttgagggagttcggttccttcgaagggagctgtag

SEQ ID NO: 39 - DNA, 2424 bp, Clostridium hathewayi
atgaaaagaaacagcgatattttcaatcaggtgattcgttttattgtgtatcacgggaagatcattgagaagattttcctggtaaccacaattctctgtgccgtttgtttcccgtttgtgggggtgaattacgatctgagcaaatatctgccggattttgcaccgacaaagcaggcgctggatgtgatggaggcggagtttggttatcccggcatggcgcgtgttatggtaaaagacgtatctctgcaggaggcgaaacgcatccgggaagagatatctgcggttgacggggtagatctggttctcggttctgacgtctcgaccgatgtctacatgggaacaccgtttctgagtgaaagcatgacggaattcatcggcgtcgatttgcttgcaatcgacgattactataaagacgggaacgccctgatggacattgtctttgaagataaagacggggagccgcgtaccaatgcggccatcgaggaaatctaccggatcgtcggtaaggaccggggatgcttttccggaagcgccatatccagcaaggaacgggaggcttcgatcacaagagagatcgccatggcgattgccatgtcaatcgtgattatatggctgatcctgacgctgaccaccacgtcgtggatggagccgtttctctttattttcgtgatgatcgtggcgattgtactgaatatggggtcgaatattatttttggaacgatatccttctttactttctccacagcggctattttgcagctggcggtatcgatggactattctattttcctgcttcatacctttacagcattgaaaaacaggggcatggaaatccatgaggcgatggtggaggcgatcagggaatcctgcagttcgattctcgccagcggggtgaccaccattgtgggatttatcgttatcgcgtttatgcggtttaccataggaaaggacgtgggatttgtactcgcaaagggaatcatatgcagccttttaacggtgcttctgctgatgcccacactgattctccggtttgacgataagattgtgaaaacggcgcataagccgcttatcgcttctttcgatggatttgcacgggccatgtaccggatcaggattccggtgttccttttggcggcgctcttagcagtgccctgttatttcgggcagggtatgaatcacttcctgtacggcgacgatgcgatcggtgcgggaccgggaacgcgggtttacgaagacacgcaggagattgaccgtctgtttaaaaagtccaacatgacgatctgcatcgtgccgaacggttccggcgtgacggaaaaggaactgtcaaaggaactggagaacctggattttgtcaattatgtgatttccatgtcaggaaccatgcctgacggaataccggaaagcttccttcctgatgatttgacgagccagctgcggggcgatgtttatgccagaatgctgatttccatgaataccttacaggagagcgactatgcgtttgagtgcagtgccagactggaggagattgtacataagtattatcctgacaattcctacgtgatcgggatgacgcccacaaccattgacatcagggatattctgacagaggattacaatcatgtatctctgctgtctctggctggtgtggcacttgtcgtatttctgacattccgctcggtcctggtgccgattctggtgattgtgccgatcgaagttgccatctatttaaacatgacgctgccctatgtgatgggggacaccatgatctatatcggctatatcatcgtcagctgtctgcagctgggggctaccatcgattactcgattctgatgacaaacaactacctggcgtttcgaaaggaaaagggacgccgcgaggctgccgttgccgctgtcaataagagtacgctttcaatcatgacatcgggcggtattctgatggtggtaggatatctgctgtattttacttcgtccatacaggcgatttcccaggtagggcgtctggtgggacgcggggctttcctgagcgtgacactggtactgtctctgcttccggcgctcttatccgcatttgataagcagatcaaacggcagcaggagcgggcggatgcacggaaagagagaaggcggaaccgtctggcggcagcaaaaaacctgacaacagggaaaagtctgccgggagcgaagcgtgtgacggaagagaaggaactgacggaagagaaggagttatcggaagagaaggagttatcggaagagaaggagttatcggaagagaaggagttaccggaagaggcaggtcttacgacagatgtgagcccgacatttgcagatggaaaatgcgggcagaaagaaggttccgcgcaggcggaggcagaagagccggagcagaaggaaaagggagatgacagccatgagaaagagtaa

SEQ ID NO: 40 - DNA, 2247 bp, Clostridium hathewayi
atgccaacgatcaaagatattgccgccaaagcaggggtatcccacggcacagtttccaatgtgttgaacaagaggggaaacgtcagcgccgaaaaaatccagctggtagagcggattgccaaagagatgggatataaaatgaatgtccaggcccagcagctgcgggccggtacggcacggagagtctgcgtcattgtgcctaagatcagcttaaaatgctacaacgatttatataacgggctggaacagtacctgcgggagtacgagatcagcatagaactcatatccaccaataacctggagtgcgacgaggaaaaagcagtaaagaaggctctctccttaaatcccatggcggtggtggtggtcagctcgcttcttaagaacaggggattatacacttcagataccaggtttttctttgccgaaagaaaggtaaagggaatgccggacgcgtctgtctacgtatcctttggatttgagcaggcgggacgggatatcgcggttaagtgtatcgaggatggccatcagaatgtggctttgctctgtgagaacagcatctattccaacaataaaagctttattaatggtgtggtggatgtgctggaggacgataattgctcctgcaaaatatttcccagcgacgacagcatgtggtttaacaaggcctttgatatcctgggatcgaaagaggattttgacgcggtgattgccatgagccaggaggacgccgattatttgagggtggcccatcagtataatccggataagaaaatgccggttatatatgcgctgaccagcaagagcatcggaatcgatccggccgtgtgccgatatgagctgaattataagctgatgggaagaaacatagcggaacagatcgtaaatgccggcggggaagaggcggagacggcgcctgcgcagaaacagcagatcatcatggaaaatgacggattctacgataatccccttccggccgcagggaagaaagacagcatctgttttttgaccattcagaatctgaccagcaaggccatcggcatgctgcttccttcctttaccagggagaccggtatcaaggtcaatatgatcgaggtttcctacgatgagcattacaagatggcgcaggcctgcgtgcagaacagcccctatgatctggtccgcatcgatatggcgtggatgacggagctgggcgataagatttatcagcccttcgacagctccagctcttcggtcaggtggctgcggcagcagattcttccctcactctcggaaaactattccatggttcatggtgtccagtacgcgtttccgttggatgcctgcgtgcagatgctgttctaccggaaggatctattcgaggatgagctgatcaagagggaatttttcgaaaaatacaaacggcgtctggagattcctaagacgtttgaagaatacaatgaagtggccagattctttacgagaaaagagaatcccgattccaggacgaggtatggagccgttaccgcttatggaagaacattcctggcggcgtgcgattttctgccgcgttttagggaactgaagaaggatatcttcgatgcacggggaaatgtaaatatcctgatccccgagatgaaacaggcgatccgcaattatctggatacctgcaagtatgcgggcagtgatatctatcagtggtggggggaacccacccgccagttctcggaggggaatacggcgatgcatatcgtgttttccaactatgcctccgagatgatacacaatccggaatcgaaggtgctggggcgaatcgcctgcgacaccgttccgggcgggcagccattgtcgggcggaggctcggtgggaatctccagattcagcaaaaagtatgacgcgtgcatgagcttcttaaagtggctgtaccggaaggatatcgcggagaccatcacgtatcttggcggatacgtctgcaaccgccagatcagcaggaacatggatatcctggaacgctatccgtggctcgagaacatggaaaaatccttcgaacccggctggaggctttataaacatgacagaaatcctgatttcaatgagttcctgtttgaggatattctgggtaaggcgatccggtccatcgcatcgggaatcgaagagatggatgacgcgctggagaaggcgcaggaggaatgtgatcgggcatttaacgaaacaagcgggaattcttccatctcaataggcggagggctgaatcgccaaaaacaagtttag

SEQ ID NO: 41 - DNA, 2127 bp, Clostridium hathewayi
atgagaaatagaagaaaaatcagatataaaattaccgccgccgcattgatcagctcgatgctcggcatgtccatggcaggcagcgcccttgcgggaccgcccgcggttgccacggatgaggcgctgtatgtgaacctggattattacggaaatcaggtggacagcagtgtggtgaagggagtttccttaaacggccttcgaacatttacggattatggaacttatacagatgtaacaaatatgtctaattacgcggaaccggtgatcagcggggacggagtcacctggcagctgccggaggactcaaaggagcggttttactacgagtgccagctgaacaacgacgaggtggttctcccgtggaattttgacgtgtcctataaactaaatggtattccaaaggaagcaaaggacctggtccatgccaatggactggtggaaatggaggtccactgcattccgaatgagaatgcaaaggagtactaccgcaacaacatgcttcttcaggtggcgaccatggttaatatggaagacgtaaacgctgtggaggcgccaggctctcagacacaggcattaggaacgtataaggttgtgatttttgccgcggtcccaggggaggagaagacctttcacatcgggatcagcacgacgaatttcgagtccatgggcctgatcatgatgatgattcccggaacgctggaccagatgagcgagatcaccgatatcaaagaggtaaaggacacagtgggggattccaccgataagctgctggatggtatgaatgaaatcctggataccctggaccggatcagcggcggtatgaatgtggcacaggcgggcctggaggatctgcagaaggcgagatcgggtctggacgcgtcaaaggacgaaatcatagccaacgcggataacagcctggacagtctggaagctgtcaatgaaaaaatcagccagctggctccggatatcaatacgaataagcagtctctggatgaaatcaacacgagaatcaacgccatcgtgaagactctgagaagctccggcaatgacttctttgatctggcaggaaaactcagtgatctggaggactctctgggggatttgcgggatgatttgaataattccaacagggacgagattctggatcatctgcagattgtagatgaccagctggaacagatcaatgaagtgcttcagaatatcatacagacggccggaggtatccctgcggaactggatgaggaagatctggcggagcagcaggagacgctgagcaatttgctggaggagacgtatggtattctggatgacatggagtccgttgtcggctccgatgccgtggaccgcctgcgcagccagctggatgcgattaacggaaatggcctgggagacgcggccagcctttcgaagctggcggcagcggccaaggcgcttctccctgtggtttccggccttcagggcatggtgagcgatctggagcgcacactgtctggaatccgcctggatgacggccttgagagcggccaggacgcggccggggagatcagctccatcatgggccggatcgagaccttgatcggcgacgtcaatgatttaaacaggactgtcaatgaagataaagccggttttgacctgatgcttgatgacatggccgcctccctcgatcagatgagttccggcacaagtcaggtgattgctctcttgagaagtgtgcagaacacggccaggaccaaccggagcgcggtggaaaacggtacgaagcagacccttgacggcctgatcgatattctggaaaaggctgcggataccaagggcaccagcgacaaattaaaggatgccaacgaggacttgagagccagtgtaaaggatgagctggataagatcgaggacgatacgaatctgctggaaatggacccgtctcagtccatgatttccttcacctcggataagaatccgtctccggccagcattcagattattctgcgcacagaggagatcagcgaagaagatgtgaatacgaacgcggttgatatcgaaccggttccgcagaatgtcgggctgtggcagagaattgtaaatgtgtttgtgaagatatgggatacggtaacgggattttttaagaaatag

SEQ ID NO: 42 - DNA, 2076 bp, Clostridium hathewayi
gtgtatacaaaaaagaaaacagctgagaggcgggagaggggaattacgatgaagtttacagtagaaaatccggatgagaaacggagtccctatacgggaatgacaagagaacactggatcagtatcagtcattttttcctggaaggaatttttgagcatgtggagaagatcgaggatccgatcgtagtcggacgccatgagacaaaggtcagctatccacagccggatgggccgaaatggagaattgcggcggagcggtttgagggacttgccaggagctttctgattgcggcaccgctgcttcataatgagccggaggcagcggcgggtggctactctcttaaggagtattattcaaaacagatcctgctctccgtcacacccgggacgcccaattatctgcttcgggtggaggagatatttccggaggcgcaggaaggggagatggcgtttcagcacacgtgtgagtgcgcttctcttgttatcggcctgtccatgtgccgggaggtgatctgggagaattatgcgaaggaggagcgggaccgcattgcagattacctgtcgaattttggccattcctatacgggccaccacaactggcgcctgtttaatatgctgattctggcctttctggaccgggagggatacccggtggatcatgggatgatgcgggatcacgcggccgccattctctcctattacgcaggggacggctggtaccgcgacgggcatttgtttgattactactgcccttgggccttccatgtgtacggacctctctggaaccagtggtacggctatgaaaaggagccgtacatggccgcaaagatcgaagaatactccaaccgtctggtggagacattccatcgcatgttcgatgaagagggccatgtgaccatgtgggggagaagcggtatctacagaagcgcggcttccgctccgctggcggctaattttctgttaaagaatccggctgcggacccggggctggccagaagaatcgcctcaggtgccgtactccagtttgcgacccgggaagagtgtttctatgagggagtgccgtgccttggcttctacggaccgtttcagccgttaattcagacctacagctgcgcggccagcccattctggattgccaacgcatttgtctgtctcgcccttccgaaggatcatccgttctggaccgatacggagagaaacggggtctgggaggagatgaaggaaagggaagtaaggactacggtgctcgatggtccggggatcgtggtggataaccacaaagatacgggaattacagaattcaggacggcaaaggtcctgatgaagaaagataatccctccctcaatacctattccagactgtcctttaacagccagtttctatgggaggacttcgattttaaggggattgaggccatgcagtacagtgtgacctatgacggcagaccgaagagcctgatcccgaatatcctgatgtacggcggcgtgaaggacggagtgctctaccggaaggaatactttgaatttgaatttaccttccagaaccaggcgtcgatcgatctggccgatttcccggtggcggacggcatcgtgcgcgtggacaggaccagaattccggataagccatataccctgacactgggttcctatggaatgccggacgtggaccgctcgggtgtggacgtgagaatccgcacggatcaggtgacgggggccaaggcaatccttttgaagtcttccgagggacagatggcgatggtcatctacggcggcttcgatgatattgaaatcatgtcgagacagggcgtgagcgctgtgacgaagcagagctgtattatgtatggcgtcagccgcaggaggaaatactatgaataccttccgtatgcgatgatcagcgtgattctgacaaagaaaagccaggaagagtggcgggacgaggaccttttcccgatccggagcatctcctatgcggataaagaaaaatgcggggcatacggtcccattgttctggagatgaaggatggcaggacggtcacggtggattatgagggactggaaggaaggctccatatttaa

SEQ ID NO: 43 - DNA, 1956 bp, Clostridium hathewayi
atggcgctttatgactattcaggtgctttgaaaaaaggaagaaaacagtatcaggtttccgtggcaaagggagagtatccttatcttcctgtgctggacgatatcctttcctacacggatatcatttcagaagtgaatctgggactgatggatgtcccgctggataagatcgttggaacaaaaacaaaaggcagaacgagtgcctttgccaataattttatgcctctgctggcagagaagtcagagtttggggcgaaatgggcgtatttatacgaccatcagatagaagaggggatccatgatcccatcgttgcgtatgaatttatgaatcaatattacgtgcaggagggcaataagcgtgtcagcgtgctcaaatatgtgggtgcattcagcatcacggcctcggtgacccgtctgatcccgaagagaacggatgatctcgacaatcgcctctattatgaattcctggagttttaccaggtgtcctttaactgtgatgtctggttcagccaggagggctgctacgaccgcctgttaaaggctatgggaaaggccccggaagaggtgtggagcgaggacgacaggatctatttcaaatccgcctacgaccagttttccaaggcgttccgcgcatttggagggagttcctatgagatgacgtgctctgacgccttccttgtctatgtcgaactgttcggctatgatgtggtgaagttaaagactgaaggggagatcacaaaggatctggcgaagattaaggatgaacccctgctggcatccagaggcagcaagattgccctggtagagcagccggaagaggtggaagagcaggataacggcccgttaaagatcattaactggctccgcccatcccagaacatcgaacctgagatgctgaagattgcatttatccatgcgaagaccgctgagacgtccagctggacctacggccatgagctgggacgcatgtatctggagcaggcctttgagggccggttaaagacggttgcgttcttcgaggccgacacggatgcagagattgcgaacgccatcgacctggcgatagcggccaggtgcaacatgatctttacgacggcctcccagatgatcggtttaagcgtcaaggctgccatcgagcatccagaggtgaagattttcaactgttccgtcaacatgtcgtattcatctgtctgcacctattatgccagaatgtatgagtcgaaattcctgatgggcgcgctggccgcttccatggcgcagtgtgataagctgggatatattgcggattatccgatctacggaaccatcgccaatatcaacgcatttgccctgggcgcgcgtatgatcaacccatacgtcaaggttcatttggagtgggcgagggtaaaaggcaggaatgcccgggaggaactggagaaggaaggaatcgcgtttatctccggagaagacatgatcacgccgaagaccgcgtcgagagagtacggtttatataaaatagagtctgacggagaattccggaatctggcgacgccgatctggcactggggaaaattctacgagagaatcgtgaatatcacctgccgcggcggctccgatgtgaaggagatgaagggaaagcaggccatcaactactggtggggaatgtcggcggatgtgatcgatgtcatctgttcccagaatctgcctcacggcaccaaccggctgattacgttcctgaagaattcgatccgaagcggaagcttccagccgtttgtaggaaccatctactcacaggatgggacgattcagtgtgaggaggaacagaggctttctccggaagagatcatcacgatgaactggctggctgacaacgtggtgggaaagcttcctgaatttgatgaactgacagaggaggcacagtcgctggtaaggcttcagggactgacgatatacgacaatgcggtgatggaggaataa

SEQ ID NO: 44 - DNA, 1947 bp, Clostridium hathewayi
atggttgaggcaagaaccagatatgttatcatgataaaaacaatgttaggcaggaaaacgtacgtgacctcggctgctctcgcagaagcagccggggtttctgtgcgcacggtaaagtatgacttaaaggagcttcagagcttcttaaaggagtatggcgtggagatcgaatcgaaacgttcttacggctaccgcctgctggtgggagacggctccgacatggaggggctgtcgaaggcgcttcgggccaatctgcggaaacataagggagaggtgttccgctataattttcagagggtgatctatatcatcaacaagctgctgatcggaaagccgtactataaggcggaggagctgatggatacgttttacatcagccgttcgacgctcacccaggacttaaaccgcgcccggacccttcttgcaaagttccgcctggaaattgacgtgaacctgcgccggggaatcggcgtcaccggtgatgagctggataagcgcctctgtatagcagaatacttcttccggtacgatgataagctgcaggttatggtgcagaggcgggctgacggcgggaagtatgactgggatgcccagagggacactcttgtccgtatcgtctgggaggcatgccgtgccaataagatccggctgtcgccgtttctggccgtggatctggccagtcacatgtatgtcagtgtgctgcgcatgaaggcaggctgcggcatcggggagctgccgggccataccatgacagtggaatatgtgagggagcggtacgcggcaggggaggtcgcggatcagctggaaaaactctattccgtatcgatttcagagaaagagcgggagtattttgccctccatatactgagtaagaaaatgccggacagcgggcctgtgggctccggagagcacgccacgttaaagcagtgtgtgacggaaatcatgcgggaggtaaaggataactttgaactggattttaccaatgatcccgtgtttctcgattttttatattccagcattgaacctatggtcttaaggctcagaacgcatctgattgtcagaaatccgcttctgtttgagaatctgcgccgttatttatttgccaccaaggtggcccactcggccagcggaatcatagaaaagctgtttggcgttcagatggacaataatgagtttgcctatctggtgcctgcattcaacatgatcatcagtacccatgagaagcggaagaagtttaagatcggattctgcggtgacttggggctctcggaggctctgatctactataatgagctttcggagagtcttcccagggatggctatgaactggtgtggctggacagataccacaataccggttatttaaaccagctccagtatctgatctacgtcagtgactaccgtcttccgtcagagctgccgtattatgagatacaggacggggattccaccagtgaggtctgcagtgcaattgcggaatataagctggagcaggtacagatagaacagtatttaaagccggaattcggcatattcggtctggaggggaaaagccgggaagaggtcatggagaacttataccgctgtctggccgcccgcggcctgattgccacggagctggactggaaaaatgcattccgggccaatgaggtgggcaatgggatcgcccatattcaggacctgggaaggattcttaagaatgccggctgttacgtctgcatcttaaaaacacctatcctgtgggagcaggatatcataaaagtactggtgatgatcaagacaaagcgggatggagacaagaatttgtccctgctctgccgcatcgtctccaattgggcatcatcgccggaaaaggtggaacattttctgaaatcgcagagctatgatgtgttctgcggggatattaagtcggaatgcctgaacatatgcttccattccatcatctga

SEQ ID NO: 45 - DNA, 1944 bp, Clostridium hathewayi
atgaaggcatatgggaaacggctggggaagattgtgattctggcagctgttttaaattttttgatcgagtttatcagcaggaagtcgcttgcagtgcttttggcctacgtgttggaaagtccgctggtcttccttttgaatacatgcattatcgctctgccgtttacggtgctgtttcttacgaggcgcagggtgtttggggcaatcgtgctgtcgattgtctggctgggaatgggagtcgtgaatgggatactcctgattttccggacgactccgtttacggcggcggatttcaggctgatcaagtacgcggccaatattgcgaccacgtatttcacctggatgcagctggttatgatagcagcggctctggtggtggtggcggtcttctgcgtgtttgtgtggcggattgcgccggtgagccgggaaaaggtcaattacgtcaagggcacggcggttgtggggatcagcgcggcggtggtcctgggactgacgacagctgccatgaacaccgggctggtggcggtgcgtttcggcaatatcggagcggcgtttttagcgtacgggttcccctactgctttgccaattccatgttcaacacgggaatctccaagccggaggactatggtacggagacgatcgaggtgattaaggcggaggagctggttccggaaaatacatatgcggtctcggccagtacgaagccgaatgtcattatgatccagctggagtcctttttcgacccgctcctgtggaagaagaatccggtgatgggcaatccggaatccggtgggacggaaaactatgatcccatcccatttttccaccagctgcagaaaaattatccccatggatatttgaatgtgccttccgtgggcgcggggacggccaatacggaatttgaagccatcacgggcatgaatctggatttcttcggaccgggcgagtatccttataaaaccgtgctgaaaaagacctcctgcgagagtgtggcctttgatttaaagaatctgggctactcggcccacgccatccacaacaacgaggcgaccttctatgacaggaacaatgtattcgcgcagatcgggttcgatacgtttacgcccattgaatatatgaacaatattgagagaaatccggccggatggtgcaaggacaagatcctggtgaaggagattatagggacgctggattccacagaggggcctgattttatctataccatatcggtgcagggccatggaaagtatccggattttaagtattactgtgaacagatcggtgagatggatgatttcatccgttcgcttgtcaatactcttcgcacgagggaggagcccatcgtacttgtaatgtacggagaccaccttcccagctttgaatggacggaggatgagatgatcaacaaatccctgtaccagacggagtatgtggtctggaacaatatgaatcttccgaagaagaaggtggatgtggaggcgtatcagctggccgcccacgtgctggatatgctggggattcatgagggaaccatgatgcggttccatcagaactatctggatggcggcatggaggatgaggagacgtatctggccgatatgaaggcgctggaatacgatatcctgtacggagacagggaggtctacggcggggaaaatccctaccagaccacggatttacagatgggaatcgatcccatcaccattgatgatattgtgtataacgattctaatattctggtgtatggtgagaattttacaccatattccaaaatctgcctggacggaaaggcggtggagaccacatttgtgtggccggaactgatcattgccaggaatattccggagaaaaaggtcacggatgccgatattacggtgtggcagatcggaagggacaagattccgctgggagagggagtcagagaaaaggggaaaggatcatga

SEQ ID NO: 46 - DNA, 1845 bp, Clostridium hathewayi
gtggagcgtcagtatcagaacgaagaagctatgagaaaggagcttgaacgcgggaactatacctcagagcatccttatatcgtggtaaatccttatctcgtaaatccgctgacggccatgattttatttaaaacagaaaaagaagaggcagtgactctgactgtaaaggggaaagaagctgccggtgatattacccatacatttccgaaggcaaaggagcagatccttccggtgcttgggctctatccggagtatgataatacggttgtgattgcgctggaggacggaacggcttacgaagtaactgtgaccacggaacagattgaaaatatgccgtaccaggcggattatatcaacacaacaagtgattatatgaatgggcagctgatgttcgtgacacctgccggggattcactggccggaggctatgactatcggggagactgccgctggcatctggtggagccgtttatatttgacatgaagcctgccgcaaacggccgcattctcattggctccaaccggcttttaaacatgccttactacacggcgggcgtctgtgaaatggacctggtgggaaaaatatatacggagtactgcattccgggcggctaccatcacgaccagttcgagatggaggacggaaatctgctgatcctgactcaggagaaaaatgcagccacagcagaggacatgtgcgtgctggtggaccggaaaagcggaaaaatcatcaaatcatgggattacaaaaaggttcttccccagcaggcggcgaagtccgggagctggtcggaacacgactggttccacaacaacgcggtgtggtatgacaggcggacgaattccctgacgctctcaggcagacatcaggatgcggtcatcaatatcgattttgagacgggagaactcaactggatcatcggagacccggaggggtggccggaagatctggtaagccgttatttctttaccccggcaggcggcggtgactttgactggcagtatgaacagcacgcctgcatgatgcttccggatggcgatattatgatgtttgacaacggccactggagggcaaagaataaggagcagtacaggctcaaccgggataatttctccagaggagtccgctaccacattgatacggagaggatgacgattgagcaggtatggcagtttggaaaagagcggaagaatgacttcttctcatcctatatttccaatgtggaatattatcgtgacggctactatctggtacattccggcggaatggggtataatcatggtgttacttgtgaggaacttccggtctatatgaatctggaggatccggaatgcgtattaaagagcattaccgtagaaatcatggacggagaactggtgtatgagatgcatctgccatccaattattaccgtgccgagaagatgagcctgtaccgggaaggagccaatttagacctgggaaagggcagagtcgtaggaaatctgggagtgacaggcgagtttgatacggaggttccggcagagaacacaggggaactgcttccggaagcctgtgaggcggtgctgacggaagaggacgaccgcatcatttttaaggcgaagtttaagaagggacagctggtaatgttccagctggaaaaggaagatgatccggaggagatccatcggtatttcatctccaccagtgcacagaagtttctggcgatgtgttccggcaccttcctgcccaaggatgacagggaagtgacgttaaacgtcgacaaagagggcctgaacggcacctttgatgtgcgtgtcatcattgacgacagcaagtatgagaccgggctgaagctgaagttctaa

SEQ ID NO: 47 - DNA, 1746 bp, Clostridium hathewayi
atgaaagaaatgagtcggaattttatgaaaaagatctggaaaatggggcgctatcgtgacgcgtccattcagaaaaaacttacgctgtcgacatgggtggtggcaattataccgattatgattatatttgccattgtttttttcgtgttcacaaatgtcagtgtggagaattcaaaacgccagtcacagatgcttttagataagacagtggaggaactggatgcgtatttcgcgcaggcgcaggaaggcatgaatctgatggtgacggatattaatgtgcagaatgccatcgataattacgtgaccgggacctataaggaaaaactggatttaagggattttatcagaaaccgtctgaccaatatgagtacggtgggcagacgaacaggtacgatatccatttatatcaaggatgccaatcagaccttttccagagacttttccgaccaggatttagggctggcctgctccggtgctccctggtttgaagcgctgctgtcaggggaggcgtcctttgtccgcgaggatgggaactccctgcaggacgggcggcctgtctggattctggcgtccaatattgtcagcgtcaaaaacggagaggtccaggggctggtctatgtggagctggataaaaagaagatgattcagccgttttacgatctggtggagggcagcggagatgagatcatctgtaatggacaggagattgtatccgatgcctgcagggagggcggccattttgttccgctgtactcttattccacggcgctggggcagaatgtggagttcagactgcagttaaaggaactgcagagaggctatggcgcagccctggtttactttctgatcggtatggtggttctcattatcctgatctatctcattgacaagctgctggcagactggttttccaggagaatcatcacgctgcgtgatgcgacgagggagatcgccaaggggaatttagacgtggttgtctgtgatgaccatcccgatgagatcggggaactggtacagagcttaaataccatggtaaaggatatgaagcgtctgattgaaagcgaatatctggttaaaatcgagagccagcaggccaccttaagggcgcttcagagtcagattaaccctcattttatctacaatacgctggaaagcatctccatgctggccctgattcgggatcattatgagattgtagatatggcacaggcgttttccctgatgatgcggtattccatggagccgtccactcttgtggcggtcagagaagaggtcgagaatgtgcggaattttgtgaccatacagaaaatccgtttcccggaccgttttctggtggagtacgccatcgatgaggagtgcatggcggaaaagataccgaggctgaccatgcagccgctggtggaaaatgcatttaagcatggattcgaggacacgccggagcacaagcgtctcctggtttctgttctgaaacggcggggatttctcgttatcagaatttttaacgatggtatggcggttccggcggagcgaattgccagaatacgggagctgctgatgccggataaccaggaggagacgctggactgttttgctctcaggaacttaagcaggcgtcttaagcttctgtttggggaaaacagccgggtgacgctgcgctcgggaaaaggcattggaacgattgtttcattgagaattccactgcgagaagagggggaagaggacgatgagaaagattttgatctgtga

SEQ ID NO: 48 - DNA, 1740 bp, Clostridium hathewayi
atggaaagagaaaaaccacgcagcagaaagaaaaagcggctgggcgtaaagttctgggcagctgtctgcggcggtatcgcagtggcggcggctgccacggttaccgtgttgtacatacagacgggaaagcagtatcgtactgtgtttttcccaaatacgactattaacggcattgatgcgtcgaagaagactgtggatgaagtgaagcagctgatcgcttcgggcatcgacggatatacgttgaccatcaaggagcggggcggcgcagaggaagtgatatcgggcgatgagatcggcctggaatcggtgtttgacggcagccttgagaggcttctggaggaacaggagcccaacgactggttccgccatcggaaggcgactcagacttttgagatcgatactatgatccagtttagtgatgagaagcttacgggcgtggtggatgcgctgaactgctttgatgagacgcaggtggtgaaaccacaggatgcggtgatgtcagagtatgtgtcaggccagggatatagtgtgattcctgcagtagagggaagcgaactggatagagagaaggtgatggccggtatcgcggaggcggtaaacggcttacagagagagctgtccctggaggaactggaggcctacgtgaagccgggagttcccagtgacgacgcagagctcctcgcccgcgtgcaggcgcttaataaatttgtgaatgtcagagtgacatatacctttggagacagtcgggaggtgctgagcggcgatactatcaaggactggatcggcatcggtgacgatggaaacgcttatgtcagcagcggagcggtcacggagtatgtgaagagtctggcctccaaatacgatacctataataaggcaaaaactcttaatacctcctacggaaagaccgttaggattacgggtggaagctatggctggagaatcgaccagtccgcggaggcggatgaactggcagctataatccgttcaggcgagagtcagacgagagaaccggtctacaagcagaaggcggtcagccatggggccaatgattatggcagcacctatgtggagatcaacttgacggcgcagcaccttttctattataaggacggcagtcttgtggtggaatctgactttgtgtcgggtaatgaagccaagggctgggcgactccggcgggagtttatcccctgacctataagcagaaggacgcggttttaaagggcgaagattataagactccggtggattactggatgccgtttaacggcgggatcggtctccatgatgcgacatggcgttccagctttggaggcacgctgtataagaacggcggatctcacggctgcgtcaacctgccgcattccgtagcacagaagatatttgagaacatctcggcgggtactccggtactctgttaccatctggagggaaccgagtcaaagaccacctcaacaccggcgggcaagccaatacagccgacgaccgcggcaccggagacaacggcggccaccactccggcggctactgccccggcagctacaacggcgtctcccgagaccacggccccgtctgaagctcctgcgcccaagccaacagagagccagactgcggcccctacaaaggccccggagacggaagcctcgactacggcggcttcaccggagagcggagagaagggacctggagtaccaactgggagttcagggaataaagagattggaccgggcgtctcatga

SEQ ID NO: 49 - DNA, 2154 bp, Dorea longicatena
atggattttaaggaagaatggaattggttgaattcctatcagatggaagcagtgacagatgaaaatgatgcatgtattgtaaatgccaatgtaggaagtgggaagacgaccgtactgatcgcgaaaattttatatttgcattatgaaaagaagattccgcttgagaagatggtggtgctgacatttacgaataaggcagcaggagagattattgaacgtctgaagaaaaaagaaccgggacttacggaagaacaggtgcagttttttggaacattccacagtgttgccatgcggatgctgaaaaatacactgttacagacaaaagcagagaatggagaaatagctcatacagtggaaaatagcagcatggcaccggaagaatggacttcggagtttgaaattatagatccggacgaggaacaggaactggcgctttatctgattgcagaatatagtctgaaagtaaagtataaaaaccgtttgaaaaaaagactggagcaggaatatccaaattataaggctggaaaagtaaccagccgctataaggatgaactgtttcggttatatcctcttttaaagaaggaaaagaagaaagagaataaaatgagcttttccgatctgctggaagaggggacaagacttctgaaaatggggaaaaattctcggccagaatggattattgtggatgaagtacaggacagtgaccggtcacagctggaatttctggaagcattaaaaggaccggagacgaaaatctttgcagtaggagatccaaatcaggtgatctatagtttccgcgggacaactcagaatatgtttttcctgttaaagaacaggtttcaggcaaaagaactttcacttccggttaattaccgatcgaatgcatccattctggaggcggcaaaccgtttccttcaatttggcggaaagattcaaggcagtaatgaatgcggggagaagattcagataaggaatcattatgatccgtttcaggaagcaatgtatctggcagacaagatctggacacttcatcaggaagggaaggaatacagggatattgcagtattttacaggctgcaaaaacaggcagaaatcctggaaaagatgtttgcagaacagaatattccatatgaagtatcggtgaaaaagtcgtggaaagatattcctgtattgaactggcttatgtatgtcttaagatttgcgacgcatccggacgatatacaggcgggaatgcaggtattgatggataaaaggttcggagacaaatgcacaaaaaagaaagcagaagacattataaagaatcacaagacagagaaatctgatatatataagaatatgatgctgttttatacagagaaagaagtattgtcaggagaagatatatttgattcgcttggattgaaagaagcactgcaccctacctctgcagattatcagcaagatgcaaagcaggtattggattttctgaatcagatctgtacatatagcagggaaaagaagctgaatatgtcagacggaatccgggaattcctaaatgggatggcactcggaacaatagaaagtccagaggatacgcaagagtctgcggagaaggaagaagcaggcggcagagtaaaactcatgacattacatgcatcgaaggggctggaatttgatacggtattcattatcggagtaaatccgggactgctgccgatcagatgcagtagctttgatcaggaagaggaagaacggagattattctttgtagggatcacgcgtgcaagaaatcacctggaactttcttattacacgaatccgggagaaccgggggtattgggcagttacagtaattatctgaaaatgatcccggaggaattacttgagtggaaagaaatacgcagtgatgaagaaaagcggacaaatcttaaagaactaacgagaagggcaaaagaagaaatccgaaaagcagaagcacagaaagcagaaaatgttcaggaacaaaaaacggaatccgagaaaacagaaaatgttcaggaacaaaaagcgatacatcccaaatatggaaccggtattgtgacatcggaagacgatatgatggtagaagtagaatttccaaattacggaaagaaacaatttatcaaggcatttcaggaggtcgagatgatcaggtaa

SEQ ID NO: 50 - DNA, 2112 bp, Dorea longicatena
atgggtaggaagataaaaaaagtaataatgatagcagcgtttggtatggtgaccggaggacagattgctgatctgttaccggaaggaaatgtgatgcaggtagaagcgggaagtcgaaagcagattataaaagtaaaaaataaagtaaaagacagtaagaaagaatttgacaaggacaaagataacgccaaagataatgaaaaggatctggtagaagagggagaaaaagaggacagaaaagattcggaggaagatagagagaaagacgataagaaagatgacgggaaagatccggagaaggatgatgaaaaagatgacgggaaagactcagagaaggatgacgagaaagaggatggaaaagatccggagaaggatgacgagaaagaggatgggaaagactcggagaaagatgacgagaaagatgacgagaaagatgacgggaaagacttagagaaagacgatgaaaaagagaatggaaaagatccggaggaagaagagataaaaatgtatcatgcggaatatgaggatccggatggtcagaatggctattatatcagtgctccgaccggaaagatcacacatctgagtaagaatggcgtgaccagatacctttttgagaatggagatggggaaaggcaggaaggtacgctggaaaaattaaatgaatcctgccggttgaaacaattgaattttgcagatggaaggaatgaactggaagtatggatggaagatgaagaacatcatcagattgaaaattcagaaagcagaaaggaattctggatagacagtgtaagaccggtgatcggtctggaagtgtccggaggagcagatatttggcacaaagaggcagcagaggtagtggtagaagcttctgacgggagcaatggaagccagatcgcggaaattatctgtaaaacaggagaaaaaatagttgggaaaagcagtaaaggagcagaaaaatttgtcattacagaaagttcacagaatggggaaagtaccccggtaacaattattgctacagactatgcgggaaatcagacggtggtaacggatcgggtttttgttgacagagatgcaccgaaagcattgatacaaggagtggaggattatacgattaccagtaaacctgtacaagtcagctatctggcagaagaagagaatgtaattcagacggtgcgggcaaatattttaaaagaagatatcgatgggaaaaaggaagaaacagaaatcacagaatggaaaacaaaaagcaggaatgagtctggtgatacaaaaaaagaaagtgtgcagacacttgcagaggacgggctgtataaactccgaatgaatgtaacagatatggcagggaatgtcagtcatgccgagagacagctgattatagataaagaaaatcccgttattgcacatgtagatgagttggatggaaagtatttaaagaagtttagctggaattattctatcgaggaatcgattaaggattttacgaattatacatatgtaatgaaagtggacgatgcattttatcggccaggagaaaaaattgaaaaagaaggggtacatgtactgacaattgaagcttttgattcagcaggaaataaaggagaagcaaaagcgaggtttaccatcgatcatacaccgccggtgatcgagtttgaggggatagaagatggagaaaaatatgaaaaagaaaaaacattttatgtcagaacagagaatctggaagatcagattgaatacattaaaattaatgggaaaaaacaaaacaggaaaaaacagaagaagggatatgaaattcagctaaatgaggcaaaaaattatgaaatagaggtaaaagcaaaagattttgcgggaaatgaaaaagtttcacagataggatttgaaatatacgaggaaaagagtttgtggcagaaaattgtggaaccggtcagaaaatatattttttatggaaatgaaaaggtaatacaggatgaaaaaatggtcaaggaagataaaaaggaaggaaaaaagaagaacataattttatgggagagagctgttttatttggcgcattgattgttgtaggaatatggaaacgggaaaaagtgaaagaaatctggaaaaatctttcataa

SEQ ID NO: 51 - DNA, 1995 bp, Dorea longicatena
atgaaaagtatgttgaaaaaaatattttttaaactgctgggagaaaggaaaaaggattacataagagttattttaagtggaatcttctgtatatcggtcgtatttttttctacgtctgttggcagcagtcttgtttatatatcaacgggacgacgggcaactatgacagaattagtaatggaagttgaaaagaattttattttgccgtatgtgttactgatctttctcatgattttaattatactcggatatattcgtaaacgatccagcgattatgcaatgctcaatatactgggaatcaaaaggaaacacagatatatgtatattggctgtgaatatctcggaatcattttaggatcaattgcaggaggattgattcttggaatattggaagcaatgatcgtaaaaaagatactggaaaatatttttcagaattatgtaagcaatatatatttgggaatatcaccgttaattctcacactaattatcagcgtaatcatgtttggaatcggcttcgccttttgtgatcagtatattgcctgtatcggaattgaccatatagtatcgggaggaagtaatcataacagaacaagtaagaatacattgctattttgtcttataggagttgcagtatttattcttacattagtttctattgttacatattggggacaaatcggatatacgattccgacagctctgggaatcataacggcagttatttttactttatttggctgtagattatatcttgaaaaattaagaaaacaaaagaataaatattataaaaaaatcctttggctcgataactggtacgatcagtttttcagtcatgctaatatcagttatattgtcagtgcttttctgattgttattctgtttggatttaatattgtattggtagacaatcttcctgtaaagcagccggaaaattatccgtatgacatagtctggggtgccaatacaaaagataaagcatttatcgaaaagttaaaagaaaagtataatgttcagacagaattcattccatctatcagagtgacttcaggaaactgtgcagaacatactggaatttctgcaacagaatataaacgccttacaggaaagcaggttcatttaaaaaataatgaaatatacgttatataccaatgggaccgaagcgaatatggaacaattggtctggatttcggaaagctgaaaccaagattatacaccggatgcgctactgcagatatctggatttatactgcgagaacattaccaggtaataaatttacaagaaaatatacaattaagggaaatgacagaagaatcattaccgggaattttaaaacaagggttttgagtaccagcaatatgaatacggatgtgtttgaagatataattgtattttcggatcatgaatatgataagatcagtcaaaaagccaaagggtcaaaccttacagtattaatgaacgtagcacagaattatgatgctgttgtaaataaaatagctaattatgcagcaaaacattcacagattaatttctttgattatcatgacggaaatctgatttatgataaaaaaccgtgcacaatagaaaatcaggaaaaccgaatgttaaatgtaagtgcgatgttgattgatatgcttgtgttatttatcagcataatctttatcttactagagaaaatatccagtgattacgaagcactggaatggaagtatttattctattaccgtacaggaatgccggagaaaaaacgaagagaaagtatttataaagaaataaccatgacatccaaagttgccttgataacaggaatatttatagcagcagtaatgatattggtgaaaatattatataagaaaatgccggtatattggacaaagatttatctggcagaagccgcagtaatgattataggtatgaccgctattatcatagtaatcgtaagaattgcagcatggcgttcatttaagcgcagtgagaggagaaataaggatgaataa

SEQ ID NO: 52 - DNA, 1974 bp, Dorea longicatena
atgctgcataaaataatttacaaaaattttaaaagcaatatacggaaatatattttattttttgtcagtaacattatagccgtagcagaattatttatcttttggggattgaatgatgttgtagtgcgggcagttacagaaccttcgattatgatgggaataaaaagtgattttatgatagcggttggattaataactgttgttacaatacttttgatggtattttctatgcgctattatattaaactccgggcaaaagattatggaacttttattatgcttgggatgaaaaagaagatgtcttatatgcttctttttgcggaatacattataggatgtataggttcacttttaattggtattttgttaggaaatctgctcctatatggaattttatattgcttaaatcaatacaatcctcagattattacattacaaaaagtggatccggtcgtatataaaaatacaattcttttgtgtctgggagttatgcttggaatctttataattctcctggtgtggatggacggaagaaatttaagctctttaatgatgaaagaggaaataaaggaaaaacgtcccgtcagttcaaaatggctgttgtttacagtgttagggattgtatttataatacttgcaattaaacaatataagccaggaacatggggatattattttgcacatatatattttctgataggcggaattcttattatcactttcagtggtgcatttattcttgaacaggcgaaaaaagaacctttttactttcggtatgcattgaaaatcaatcaacttgatagtaaatatcaaagtaatatattaattattctgatgttatttgtaatacatttttttgttctttcttatatcggtacacaaatagtagagattctgcctcttgacaagacaaatagtaattatccttatgatataatctggatggcacgccagaacgatgaaaaatacagtgaaaaaatagctgaaaaatataatgggacagttaaacatattccgatgatccgggcaacaatgttttattcacaggaagaaattggaatatctgaatccacatataaagaactaacagggaaggcttatggtttgtctgggaaagaaattgttataggaattgaggaccagaattatcaaagggaagaaaaagtaactgataaggttctttatgatttatttggatggctgtatattggtaaatttaatccgaataaaaaggaatttgaatcttccaatattttaaaagatgcgaattatcagtataggataaaagaaattcatacacaaaacgtatttggaaaattcgtaccagaagatgccggtgaaggttgtgaagatacagttatattttcggatgaatattttgataaacaatgggaaaaacaggcagcagatgatgaagaagtttcaatgttagaagcattttcttttccaaaaacaaaagagcagatggcctggaaagagataaaagatcatgcagataaagagggaattactgtatttcaaccagatgacagtcattcgccacatgctatatgctatgataagactgtgtttttaaaagagcagaaagcaagtaatatatttttactttttagcaagctgtttattctgataacacttttgattagtggtacttttattatggttgttaaaaatctggccgaaatgtcttcttatcaaagacgttatgaattttttcattctatgggcatgaaacaaaaagagcaaaagaagatcttaagttttgagatttgcagcgtagcaaatatagcattaggtacaggtatttgtttagctcttttatatgtaatgacttatttacattggtatgatgcgatgggtgaaaaaatatcaaccactttttggagctactggcttaagctcgttggaatttatataattattcagatagttgtgcagaaattatttgtaaggtatgtgaacaaaagaatttag

SEQ ID NO: 53 - DNA, 1917 bp, Dorea longicatena
atgcttatttcgtataataaaatatggaaagataaagtacaatcgccatgggctgttatgaaggtagaggattcaccgaattatttggggagtaaagacattattgaattgcaaaatggaaaagatgtttctcaaaaaatacaaatggttagtgaaaacttaactggtgtagcaataaaattcgcaaatgtggataaaaaagcaacaggtattattgagattgaattattggatccgaatagtaaattagttgaaagatggaagttggattgtgcgatccttcaaacagacggatattgtaatgtacaattgaaaaaagatataaaggtcaaagtcggcgaaaaatatgagttaattattagacctagattacaagatggaaaaggattagcacttgaattatcaagaccatcagtgataacaggtcatgccaatgtaaaaggtgaaaaaaatatatcgttgtctttggcgtataagttgtacgatggcgacggaagtgcattaaaatatttaattgtcgcaattattattacagcacttgtagcaatgcttggaagctttttgatgatgaaaaagggaaaaatcgcaagtacatttgtcgtaatgacattttttattggatgcatttatatttttgtattaccaccgtttgctgtaccggatgaaagtgcccattttgttacggtatattctaaaagtaataaattgctaggaaaagaagttgctgataaagagggaaaagtaattgctgattctaatatgggattatattttattagagaagagtatcctacaaaagagtcttatattagatttgtaaaaggagcattaggaaaaaattcagatactattactactaaagaaggattggcgaatcctttaaatgtaaaagcgataggttatattcctcagattataggagtgagtattgcaagaatactgggaggatctggagaacaaattttattgataggaagattatttgctcttttgtggtattgttttgttatgtattttgcaatacgaatatttccgtttaataaaatgattatttttgcagtaggattattgccaatgacaatacaacaagtgtgttcgtttagttatgattcgattttattaggtttatgctttttcttaatatcatacattttatggttaatttatactaaggagagtgtggagataaaggatgttctaatattagtttgtgctattagtggaattgtaatgattaaatatatatatataccaataatagggctgcttttatttgtcccaaaacaaaagtttaattttagagttaacagaaaaaaaatagcattgtatatgtttggaatgctttcaatagttgaaatagtttcaaaagtgacattgattacagaagcagcagaaaaaaatatgcaaattagatcggatggattatacaaatattcaataggatatataatgagtaatttgggtgatacattggtagtagttgttcgaacaatttttgaaaagctctctttttttgttgagtcgatgattgccaatccattaggttgggtagatatacaggtcccgaacattattgttatggggttcgctattgttttgatttttagtgcaattccaaatcatatatcaaaaaaaacgactaaaaagctaatgataatgtcaggggttatagttatattagttagtggattggtcttggctgcgatgttaattagttatacctatgttggatcagatattattcttggggtacaaggaagatatttccttcccgttttaccgttgatattgttaattattcaaggaagtaagaatattgttgtaaaagatagtatagagacagaattgatacttgctattacgggattgcagttatatacaatttggtcaatagtatcagttgtgattacaagatag

SEQ ID NO: 54 - DNA, 1752 bp, Dorea longicatena
atggacaaagaaaaagtgatcaaaaaaataaaacagggtgcaccggctacctcggcgattgtagttgcagcctgtatcggggtgtcattaagcggctatcaggcaccggtttatgaagctcaggcacagacgaaagagacaaagacaacggatgccgaggaagcgaagaagacagaaagcaaggcaaaaggttcttttgatctggcggacggaatctataaaggaacaggaaccggttatgccggcgaggtgactgttgcggtaacgatcaaagataaacagattacggcaatcgatatcttaagttcttcggacgatgcagcgttctttaaccgtgcaaaagcagtgatagacaggatcattgcaggacagacgctggatgtggatgtggtgtctggcgcaacatttagctctaatggcattatcagtgcggtgaagaatgcattgacaggagaaaaagacagtggagagacgggagagtcccagtccggaaatgcagcggcacagggaagtgcactgtcactggctgatgtacaggatgcggcagcgtataaagatggaacctattatggaacaggaaccggattcgggggaactttgaaagtcaaggttgtgatcagcggaggaaagattgcgtctattgaggttgtggagaatcatgatgacagcagttatctgaatcgtgcaaaagcattgatcggcaatattatttcgtcgcagagtacaaatgtagatgtaatctccggggcgacttacagttcgaacggaattaagagtgcagtaagagatgcactccgtcaggctgcagtaagcggtaattcacagtctgtgaatgcgaagacggaagatacttctaagacagaagacaatacgactgtcaaaggcaatttcccgtataaagaaggtatttattacggaacggcagaagggtataacggtgagatagaagtagcggtggttcttcaggataaatcaatcaaggcagtactcgtaacaaagaatcatgatgatgaaaaattctttaaccgtgcaatggatgtagtaaaaaatattatgaaaaaacagagtacggatgtggacgtagtatccggagcaacttacagttcaaatggtctcataaatgcagtgaagaatgcattaaaagaagcagaaaaggtaacaaacggacagacaacggagccggataaggaagaagctgatacttcagaacttgaaaaagcgatgaaagaagcagaagaactgaaacaagaggattatacagaagcaacctatgcggttcttaagaccagaatggaagacgcacagaagctgcttgatgcagataagacagagatcagtcaggaagatgtggatcaggctcttgagaatctgaaccaggcactggcactgctggagaaaaaagatgatggcgaagatgatactacagtatataaaaatggtatctatgaaggacgtgcgctgtgcagaccagatgaagatgaagatttcacggcttataatctgacattgaaagtgacagtgcgggatgacaagattgttgctgttactgatgtaaaaggggacggagattcatcgaatgacagatatatccttcgcgctgcaaacggaacaccgaataaaaaaggtgtgacaagccagctgatcgagaaaggtaatacagaaggaattgatgcagtatcgggtgcaacctgtacttcaaaagcaatcctggatgcatgtgagaacgccttgctttctgcaaaaagacagtaa

SEQ ID NO: 55 - DNA, 1671 bp, Dorea longicatena
atgtctgaacaacgtaaaaaaaatgagaagaatttcctcgtacagggatcgattctggcgatagcaggagttatcacaaagctgatcggagcattttaccgcattccgctgcttaatattatcggaacggaaggaaacggatactattccgtagcgttctcaatctattccgtggctttgatgttgacttcttacagcctccctttggcagtatcaaaactggtatccgcaagagtcgccgtaggagaatacaaaaatgcacataagatttttcgtggagccataacatttgcattgctcgccggtggttttgtagctctgcttgtattctttggagctgattttattgcaacgacgatcatgcatctggatatgagtgcatatgcgctccgtgtattggcaccgtgtattctgatcgttgcattacttggagttttgagaggattttttcagggaatcggttccatggtcccgactgcaatttcacaggttattgaacagatcataaatgcagttgtatctattgcgggagcctatgtattattaaatgcaggaaaagccgtaggaaaaacgagaggtgacaaatctttcggtccggcatttgccgcagccggaggaacacttggtactgttcttggagcattcagtgcattagtatttgttggtcttgtatttcttgcatataacaaagtcttcaaacgcaaaatgagacgtgaccattcgaaaaaacgcgaaagctataagacggtatacaaagttctgtttgtaacgatcgcaccggttattttaagtgcaactgtatataatatcagtgacttcgtagatacggcgctttttaataacgtaatggctgcacaggggttcagtaaaaaagaatatgcaagtcttttgggaatctttcagggacagtacagtacaatgatcaatgtaccgctttctatttccagtgcactggcggcatctctggtgccaagtctggttgcaacagtacagactggtagcagaaaacaggtacataataagatcaatacggtaagccgttttaatatggtgatcgcaattccatgtgcggttggttttattacgctggcaaaaccaatcctgaatatgttatattttactcaggataatacaacggctgcactgatgcttcagatgggagctctttcggttgtattcttctgtctgtcaactgttaccaactctgtattacagggccttgatgacatgatgactccggtaaagaatgctgcaatttccctggtgatccatattgtgacattgttcctgatgctggtagtattgaaatggaatatctatgccgtagtattaagtaagattattttctccggagcaatctgtgtattgaacgcaaaagcactgcgtgacaggattggatatgtgcaggaaaagaagaagacttttgtaatccctgcactggcttcactgatcatgggtgtgatcgctgttttggtccacctgattttcgaattgttcgcaggcccatatattgcgacgatcatcgcacttcttgcagcagtggtaacttatggtgtggctattgttgtacttggaggaattacagaagaagaattacttggcatgccaaaaggagctacccttgtgacattatgccgtagattacatttgataaaaggggaatacaggtaa

SEQ ID NO: 56 - DNA, 1659 bp, Dorea longicatena
atgactgcaggaatgttggctatgatacttgcgatgggaatgacagcgtgtgcaaatgcagacacgaaagagaagagcacaacgaagaaagaacaggtttcagagtctgatgaaaaaaaagaacagaaaatgtcagataatgaagcaaatgtaatgaatgaaaaacagaaaaaaatctatgagaagatcaaaaaaacatacaatgcagaagagcagcagaaaatagcggacgaactggaaaagaaaaaagaatctcaggagtatacactgagtaatatgctgatcgaatacaatccttttggaaccaatacacagtcattgtatgtttattttgagacagattcggcggtgaaagtttcttatacgattcatgtaaaggaggatgatattgccgactttagcagaaatgtatatcaggatgaagagtatcagaaagagcatgaatttcaggtgatcggtctgatcccggatacggagaatacgattacattctatataacgaatgaagacggttctacggatacgaaggaaatcgtatatgagatgggaagtctgtatggagaagaggcagtacagcttgatacggatgtaaaacaaagtgcggacaagttagaagacgggctgtatgtggtacttggaaatgacagtccttctatggattttatgtattattatgacaataacggagtcttaagaggagaagttcctcttctgggataccgaagtcacaggcttatctttgacgagaattcgatgtattacagtatttccgaaaagaagatggcacaggtgaaccgtcttgggcaggtaacaaaggtatatgatcttggcaattacaaattgcaccatgattatgtgtttgatgaaaatggaaatatgttgattcttgcaactgatacgacgcaggacagcgtggaagatatcgtgttgaaactggatgtaaattccggtgaggtgacagaggtactggatctgggagatctgtttggcgaatataaaaagacctgtgtgaaaaattcttccgatgaactggactggatgcatatcaacacgattcagtatataggaaatgggtcagtacttttaagttcaagagagacgtcaacaatcatcaaagtagataatatctatgacgggccggtggtttcttatatgatcggtgaaaaagatttctggaaagatacttcttatgtaagtcttctgctgaataagaaaggagattttacaatacagggtggccagcatacgatcacatatgagacagatgaaagccttgcggacgggcagtattatctgtatatgtttgataataatattggaatcagtgagacaagaccggattatgactggtcgtcgataggtctgaaagtaagttctgcggttgacggaaagaattccaagtattacaaatatctggtggatgaaaatgaaggtacatttgaacttgtagattcgtttaaagtaccttattccggatatgtcagcagtgcgcaggaaacaggagataatgtacttgtagattcgggattaaaggggacttttacagagtatgatgcagatcataaagcaattgtaacttataagatggattatgagaaatttatttatcgtgtattcaaatacaagtttgatggattttattttgaaaaaagtgaataa

SEQ ID NO: 57 - DNA, 1632 bp, Dorea longicatena
atgagaaaggggcttttctggcattatctggagaaaagtgaattaagaccggtggtaagggaagaatataaagaaccttgcagcagcctgtatgtacgggataaaaagacacttttatttgaagtgacatattataaaaaacggatcaattttgaagtattccatgcgctgacagatggaaccggtgcaacagaattcctaagagaactggtgaagaattatctgtatctgatccacgaagaagatctggagccggtggagctgtcaaaccagtatctgacggtaaaagatcaggaagatgacagtttcagccgatattatgatccggattttccaagaaagaaaaagaaaaagatcagggcggttcagatcaaaaagggtggaaaaggatatgaagagctacagatcaatgaagcttccatgtcggtaaaagaactgctggggattgccagagaaaagaaagtttccatgtcggtgctcctgacggctgcatttatctgtgcaatccatgaagaaatgagccggatgcaggagaagaagccggttatcctgatggttccggtgaatttaagaaagatttttccatcggattcgatgctgaatttcttcggttatatagagccggggtatcagttcggagggggaaaagattcttttgaagatgtactggaggcagtaaagttatattttcaggagaatctgtccaaagagcatatggcaggacggatgaatgaactgattgcaatagaaaagcataagatcttaaaatgggcaccgctggaactgaaaaaccgctgtatccgtgcgggtgccaagatggcggagcaggaagtaaccgccgtgctttcgaacatgagtgtggtaaagatgccggaagattatgcgcaatatattgaaaagtttggcgtgtatacaagtacgaaccgaacagaattatgtatctgttcttttcaagatacgttatcacttggctttacatcgagatacgacagcacgaatatccagcggaatttctaccggatattgaaagaactgggggcttcggtcaaagtggcagaaccggatttcccggaggatgcaagaccaaattatgaaggaaagaaagtattacagatctttacattttgctgtattgcagcgatcgtgatcagtatgatgacggatatcattatatcgcccggcgtgcactggtcggtgttcgtggcagctgggtgtgcgacgatgtggcttacaatggcagtcggttatgtgaaacggttcaatctgctgaagaatgcggcatggcagcttctgatcatgtcagggatctgtgtattgtgggatctcggaaccggatggagaggctggtctgtgaatatcggaattccggatatctgcctgctgatccaggttgtaatgttgatcatatcaggaatacgttccctgtcaccgagagaatatatgatctattatgtgatggccgctgtctattcgatgattcttccattgattcttttagtgacaggagtaatccattacaagactccatcggttatctgtatcgggtgcagttttctgctgttgatcggattaattttattcaaacgaaaagaatttaaagaagaaatgcataaaaaattccacgttggctga

SEQ ID NO: 58 - DNA, 1623 bp, Dorea longicatena
atggtattaataaaaggtatgaggtgtactatggggttgttaaaactggtgatcgtagatgatgagccgatcctgctggagggtctggtaaagacgtatgactggaacggtatgggatatgaggtggttggttttgcgcagagcggagagcaggcgttaaaggtaatacgtgaaaaaaaaccacacgtagtgctgacagacatcaggatgaaacagatttccggacttatggtaatggaagaaatcaagaaagagaacccggaatgtcagttcgtggtattaagtgcatacagggattttgaatatgcgaagaaggcatgtgatctgggggcattcgcatatcttctgaagccgattgaagatgaaaaattacaggcgacgatgacagatgtcggtaaaatctgtgaagatcagatcagaaatgaggaaaagtatgaccgctgggagagacttctgaaaaaggacggagatggatttttgcaggttgtcgtgcaaaaatatgtccagaaccggctgccggaagaaaaagtagatgaagtcttccatacgctgcaggatgtcatgaaggaaggagaccggtttattacagtatatgcagatcttgatctggcctataagattaccaatgaactggaatatgaagcctcgagattttccatggtcagaatgattgaagaaaagatcgcagagagattcacatactggaaattcgaaagtgaagaaggacatcgtacatttattgtaaagacgcaggagaacacagcggtacatgagctgaaagaactactggaagaggtaaaaaaagaagagaacagcccggttattgcagcaatatccaaaccatataaagggatccgcggaatcagaagaagtttcgaagaagcgcagagattgttcgctgttacaaatgcatccggagcgggagtatttacaatcccggagactgttgaagaaaaagaggaaagcccatatccggcggaggcagagatgatggtggtcaacagcgtgcggaagaacgacgccgtacagttaaagcaggcatttgtacattttatttaccaactgccacacagagaagaactgcaatgccagtatatgcacaagatcatggtaaagacagaattcatgttaaaagacagttacgggatggacgaatcactgaatcagcaatttgaaaattattattcgaatatgagaaacttaaaggcggcaaaagcagtggatgtctgttacaagattctgggaactgctattgaaaaaagactggaaaatgcagaaaagaaagagaataagggatcaaaagaatacattgcagcggctgtggcatatatagatgaacatctggataatgaagatctttcgattgtatcagtggcgacacatgtatatctgaatccggtatattttggacgggtattcaagaatacctttcatatgacattcaaacaatatctgctgcagcgtagaatggagctggcaaagagactgctggaagacggaagaaccagcatcggtaatatctgcgagcaggtcggaatcagtaatccatcctatttttcgcatttgtttaaagaatatacaggacagcttccgagagattacaaaagggaatatgaagtatga

SEQ ID NO: 59 - DNA, 1542 bp, Dorea longicatena
atggatagtcgttcacgtacagaatattcgatactaaatataatagcaggagttgggggatatattgtaaatactattcttggttttatatgcagaatggtgtttgtaaagtgtttggcagcggattatttaggagtaaacgggttgtttacaaatattcttacaatgctttctttggcagagctaggaataggcggtgcaatagtttatgcactgtataaaccattagcagaaaatgatgaaagaaaaatagcatcattggtaaaggtatatggaacggcatataaagttataggttgtgttattgggataataggaatatgtctaatgccgtttttaaatataattattacggaacagccaaatatttctgaaagtatttatttattgtatatttttaatttgttcaacacagtaataacatatttctatagttatagaagttcgttgctaatagctgctcaacaaaattatattgtggttgcaacgaattatatagtaactattttacaaagcattttgcaaatggtggcattattagcgacgcataattatttggtgtatcttactattcagacgataggaacattggcatacaattttggggtgtcgcatatagcaacaaagcgtttcccatgtattatgtcaaaagatattgaaccgttgccagttgatgaaaaaaaggcattatttaaaaatataaaggatcttacatattacaagatttctggattattagttaatagcactgataatatattaattactttttttaagggattggctacaactggagtcgcatcaaattacacattgttaacaaatacaataaattccttattaggtcaaatttttaatagtttaactgcaagtattggaaaccataatgcaactgaaacggagaaaaaaaaatatgagatgttcagcttcatgaatttaatgaatttctggatttttggctgggcgacattaggaattattttttgttcttcagatgttgtaagattgtgctttggcgagaaatacgttttgtcaaaagaaattccatttgtattagcattaaatttttatactgtagggatgatgaatgccgtatggacgtataaacatacaatgggcttatttagatatggaagatttttgcagattattacaggagtgcttaatattattttctcaatagtattaggacactattggggattgtttggaattttatttgccacatttatagcgcgagctatgacaaatttatggtatgatccgtatgcaatatttattcatggatttcataaatcaccattacagtatttaaaaaagtatatttattttattattgtgttattaatatctgcgggtggatgttggctttcatttaaacttattaaaggtggaattctagcacgtgtaatggaagaaatagtattgtgtagtgtagttacgaatttagttttttatatattttttagaaaatcagaagaatttattacattaagaaagattattaaaaatataataaatttgataattaaaaaatcgtga

SEQ ID NO: 60 - DNA, 1542 bp, Dorea longicatena
atgttgcaacaaaaagaaagttatgatgtgttgcggctgattgagcatggacaattatgctatatcagttccgaaaatgtgcaggggaaaaccctggacagatacttaaaatatcatccggtaataaaaaaacgggagatatttttattattaaaagagatagcaggacaactggcgtcatttcacaggtgcaggggaaatccttgttatcaatatgtaaatccatatagtattgtcaggtctgaagatggaagaatttattttctggatatgcagtcggaagcaaacagaagcaagatgatatttatgcaaagaagagatatccgtgaatattttcttccgccggacgaaaagtattatcaacatgccagtaaggaactggatatgtatgggctgggaaaaacatttcaatatattctggcatctgtggaggcagaaccacgttttaacagacgagaagaatatcgtcttcagagaattatttcaaaagcaatggggataagatcaccccattatctaaatgtatcagaaatccaaaagcaaatcccaaggtatgaagaaaaagacagagataaaattttgaataataaggggaaaagaagaaaaaaagtgtgtataacagtagttttgtctattgttttcgggggatatttgttcataaatgcatgggaaaatgctgaaaaagcaaaccagagagagatgaaaagaacggaatcttccaaatcagaagagaaaaaaagtgaaaaatcggatgaccggataaaaaagaaaatatatgaaagagatgaagagtatctggaattggcactggcatatttcctgaatgtgggagatatgaaaaaaagtctgaaatgtctgaatcaaatggagaatcagacgctggcagttaatctgaaaaggcttatcaaagcgtatgaaaaacaaaaagtgccggaagaggcagaaaaatttgcagcaagtcttgcttacctggagaatgaatggaaagaaagaagtatgcagtcggaagagaagaaaaaacaggcaatacagtgcctgataagagggtatggattactggatgataaagaaagttcagaaaaagtgttgaatctggtagaagaaggattaaagacagattatctgaatgattctgcgaagagagaactattgcagtatcaggcgtctgcattggaaaaagaagaaaagaaagaggaggcagcaaacatatatgcagagatattggaggatgagacggaaccgggtaagagagaagagctgtataaaaagatggtacagttgtatgaaactgcaggaagacgggatatggcaagcgatacatgcattcaggggataaaagagcttggagaatcagaagagttgaaattaacacatataagactgatatgtgcagatccggttgtcaatagagatacgtgtgcactcaagattaaagaatatgtaacagaagatactgaacttttggaaaatgcagaatttaagaaattacaaaaagaatatggaattaaggcagaaggaggaaatatatgggtaggaagataa

SEQ ID NO: 61 - DNA, 4359 bp, Eubacterium siraeum
atgacaaatgtaaagaaatttacagcaaaagtgacagctttactgctggcgctttcactggcactgctgtcagtaccgcaggtgagctttactgtatttgccgatgatgacctcggaagcgtccgtgttattgtagaaaacacaacgtttaccgaagcggtcagcggcggtaacgctcctgcgtggacaggtaccaaggtcgacaagtgggtatcgcttgacaagacctcaagtgcaatgacctgcataaaggacgctatcgaaagctccggctttactcagaagggcgcagacgatggctacataagcgagatcgcaggccttgcggcgtttgacggcggctcgatgagcggctggatgggtacgctcaacgactggtttacaaacgaaggcttcacagcctataccgttgctaacggcaagcttgcaagcggcgatgagatccgtatgcagtacactatggactggggtgctgacctcggcagtgactggagcggtacagatacatcgcttaaagcgataagcagcgattacggcacactttcccccgaattcagtgcaaagacctataattatactcttacagttcctttcggcacaaagagcatcaatttccgtcctaccgcactgaacaagaatttcaagacggtaagcaaaatcggcgacaagacgctgagccttacaaaaccgactgaaataaaggacggcgatattatcaccgttactgtaggcgagggtgcaacagcaagcacttataaggtaacaataaaggagggtgcaagacccgccgcacgttttgacagctttgcactttcggctttctcgcttgacggctgggacaatgacgctttcgaccctgaaaagctcgaatatgatgtaaagataaagtcttacagcacatcatctttctatatcaacagcggaaccaagttcaacaaggacctgctgaagtgctatgcggtatacaccgatataaacggagttgcacagagaaacgagataaagtccggcagcttcaacagcatttctaatattcctttcggcttgactaagctgattttagagctttgctacattgacgatgaaagcataaagacgcagtatgtgttcaacataacacgtccctatgactacactgcggaaatcgcaagcacaagcggcatcacgcttgttcctgccggcagagagctgtatgcgacaaagtacaacggctttgcagagggaacggttttcagaaatgacgaaaatgacaatgtgaccgatacgacaggcacaaacgcagaatgccacagctacacagcctatgttttgggaggcaccgacagcgttgcacttactctcaagggcaaaaccgcaaacgttcatttcagagcgaaggctgacggcgaatatacagagcttaaaagcggcgaaacaactcccgcatattccttcggcaaggacggcactgttacagtatcaatagatgctgtttcggacggcgattatcttacagacaagtttgatgatgcagacaagataacaagctacaaaataaagcttgtaaaggctgacgtttctataaagaacgtacactttacagagcttaaaagcgaacacggcgatatgtatcccgcattcgacccgtcacttctcagctataatatagttatagcaaatgacgcagaattccccacagtatatttcaaggttgccaacggttgcacagttaagataggcaacgatgccgcaacagcagacgaaaacggcgtttacagccttgttaccaagagcgcaaacactactgtaacggtaacagacggcactctttcagaaagctatactgtcaaggctacaaagagaagcaagtatgacgtacccgacaaggtcgttgattatctttgcatcaacagccagtacaccaacgtttcctacggtgtaggccccgagcagacgctcgcaggcactataaaatcactcggtaacttcggcggttatatcacatattactatgaaaaccccgtaacagacgacccctcaaacccctacggccttgacttctacgcttacggcaacagctttgtaagcggcggaagtgcggctgaaagcggacaggtatatgtttctgaggacggcaaaacatggtatgcgctcgcaggaagtgagcattttgaagatacgaccatcaccgattacgaagtgacatacaaaaagacagccgacggtaaaacaagctggacagacaatcagggcaactcaaacgacggctcaaagcagacaggcagatgggtttcacccagcgtttattatatgaacgatcttgcaaagggcgatactgtcacactcagaggcgttgttatccccggtgttcagggcagtatacagggcgacagctctacagcttcctttgtaggcacgacaaggttcggctatgttgactacttcaagaacggcacgataggcactaatgtaaacgcatacagcgaaaatgccgaatcaaacggtttcgacttaaagtgggcggtagatgaaaacggcaaccccgttacattcaaaaacggcgttcactatataaagatacagacggcaagcaacatctgggcaggcatattcaacgagaaatcgacagaggtttcttatgttgtaagaacagctgcaaacgagcaagaggtcggcacgacagcgcttcccggaaaaatagtcttaacagacgcaaacggcaagacaataaaggaaatcactcccgatgataacggtgtttacgagataagcacaggcatcgaggaaagcgtgaacgtttccgtatccggcgctgacgatgataacatttatatcaacaatcagcgtgtagcatccggcacagaggctaaaatcgcacttaatcagtctgaaataaaggttgtcagaataatcgttcagaacggtgaaaaacagcccgtatacgcttacttaaagctcgttcccgatgatgtaaaggcggctgagcaggtcgaagaacttattgacgctataggcgatgtaacgctcgacagttatgacagcatcacagcggcaagagcggcttatgacaagctcagcgacaacgcaaagacgcttgtaggaaactacgaaaccttaacagccgcagaagaagctctcgctaaggctgaggctgacgttataagcaatgcgataaaggcaatagacgcaatcggcaaggtgaccgctgacagcaaggataagattgaaaatgcaaaggacgcttactcggcagttcccgagcgtttaagagataaagtcacaaattcggatactcttgacaaggcaacagaaagatttgccgttattaacacgataaagcaggcaggcacaaagagtaaggagcacttcgacactgttctcggtactcttgcggataacaatatctaccccgttcagtctatcggcggtgaatggtcggttatcgcactcgcaagagcaggaaagctctctgccgacaaggcggcaaaatactacagcgagctttgtgaagcagtaaaggctaacggttcagacagactttcggacagaaagcctacggagaacgcaagagttataatcgctctgtcctcactcggaaagaattccgcagacatcgcaggccataacctgctgagcggtcttgacgatatggactatatcacatcgcagggtatcaatgcggttatattctcactcatagcattcgacactacagattacagcgcaaagacgcacgatgagcttatcgcttatattgttgacaatatgacgggcaagggctgggcgctcgccggcgataccgcagatgttgaccttacggctatggctatacaggctctcgctccctatgcggctgacgagaaggtaaatgcggctatagacagcggtcttgagttccttgcagaatctcttgacgagaacgcaagatatgcaaacggcagtgaaagcacctcgcaggtacttatcgcacttgccgctctcggcatcgacccgcttacagattcaagattcatcgttgacggcatcacgcttatcgacgcacttgaaagctacgctacagaaaacggctacagccacacactcggcggcgaagaaaactatatggctaccgagcaggcggcactcgctcttacagcttatgagctttcaaaggacggctcttcactttacgaaatgtctgcgaaggctgagccgacagaacccgaaaatcccgatacgcccgcacagcccggcgattctgtaaagcccggcgactgctcgggcaagcccgaagataaaaacgatcccataaatcccggtacaggcgtacttgtaacaggcggtatggcagttctcatctcaggcgcagttatgcttatttcgaagaaaaagcgcaaataa

SEQ ID NO: 62 - DNA, 3681 bp, Eubacterium siraeum
atgaacttcatgcaacttcgtgaaagacagccgaaattccccgttaccgtaaagacgggagagggagtagtagagcttatctggaataaaattgaatatgctgacggctaccgtgtgtttgcgtcgcctgtcggcaagaatcattttgtcggtgtaattaacgtcaaaggcactactgccgttatgaaaaaacgtgcaaacggcgttcctatgcagtataaggtcaaggcgttcagaattgcggacggtccggataattttttcggagagtccgaaattgtcatagcgtgtccgcttgaaactccacgcagacttaccgcaatagtcggaagcgacggtatatgcacattgtcatggagatacaactcgcagtgtgacggattcaagatctatgccgattcgaatgaaagcggaaaatactcttttgtgtgctacagcggaaagaattcctgcaggcttgacagcttcacaaaaagcggtaaggtttcgtttgttgtacgcagttttataatgaccgggcatatggaaaagctgggcgtttcttctgctcccgccgaagccgttattcccaaatccaaaggcgctaaggcggtgcagttcgaccattcgatgataagaaaaacggcaggtgattacaatgcaaggcgctttgccggcaaggacggaaggctttgcaacgatcaccataaatgcaccgtgatgataggcggcgatattaccgtttcggctgaaatgcagaaaaatgcggcaaagggaatgcctgtttttgacgagactttttcatcgctcggcggaatattcggttcgtttgatttttccgttgcgatgcttgatacggatattaacgataaaaaggcgtatacattcgaggacagccgtgtcatcaactgcccgtcaacgatcgccgacgctgtatgcaagagcggaatagacgcacttgctgtcaacgcaggacttctgcagagagcgccgcagtcgctcgaaaagtatccgcttacggttataaccgagaacgactgcacacagggcggagaaaagttcagcattgtaaatatcaacaatataaatgtcggattcatttctgcgacagtgaacaaggatatatcgcagtatgtgtcacagctcagaaaagcgggggcagagtacatattcttcttctgctcgtggaatgaacgtcatacgcctgcggtaaagcctaagtggagaaatcaggcggtaaaggctgcggagagcggagcggatataattatcggcaacggacttaacgccattgccgaatatgatgttatagagtgcgcagacggaagacgtgttcctgtggcttattcgctcggctcgcttattcctgccgatcctgcgacacgctttgaaaagataggagcgttactttgcgtaaggctcaagcgtgataccgcaacgggcaaggtgaataccgacctttgcggatacattccttatgcgttcaaggattacggcacggaacacagagcggtgcttttgtccgatgataatgcacgttatttcgggctgtcggtatacgatacgcttaaaaagcaggtggcaacggcactcggcagtaaaatagagcttgcgagatatgcagagaagcccgaacagcaatcgtttgcacttctcggctcggcactgatttcggagcttttcaaggacgataacgatgtagaaaccgaccgttcacatctgttcatatcacagcttactatgaacggaacacactgcgatgttgatgagaaatacttccgtgacggtgttgtgcctctttactacaacctttccaaaggctatgacgaataccttgcagaaaacaaggctgatgcgcttataacggacctttattacgctgtttccacgcctgtttacaggctaggagattcgctttattcgggcggaaaagcgtttatacaatcacgtttctacgaggaaaacaaaagtcggctgaaacggctcgatataaaggatgaagcggtgtggaagcctctgcttgacaagttcattgattcggttaccgctgtgtacgacagggagaagattatacttgtacgcataacggatcccaagctgtactatgtcaacggacgatatgtacgctcgacagaccgctcgtgcaacttcaggctgcttcttgatatggagaactactttataagacgtgtttctccgaaggtcatcgacatatcacggttctatcccggtgtgataaacaaaaggggaagaagctatgcggtatgccgtgacgagcatttccgcaataacatttcgttgattgccaaaagtatatgctccggcaagaaggcaaactatgtcaactcgcttgcttacgaccctgaaatatggctcacggaagtggctgaaaactttgatataataaaggcaggcaaggcggacagcttcttcttcggcacaaacaatgccgtagactactttataagcaggctgagccgtgactttatctgtgcggaattcaaggatattctcaggctgaaaaccagtgagcttatcacgttcaatgagataagggcttgctatgatttcggcagaaacgcagtgctgaagcgggtttataacggcatctgcgctatacgcaagggcgatattacgaatgcggatattgatgagatcataaggctcggattatatgcacaaagcgatcttgctaagacgttggaatcattttacaacaaaaacgggattatcagaaactgtgtgctttcgactaagaatcttagcttctatctcaagtgtgcaaggctgtggatggcaggcacagacaaggatgcggtggcacagcttgcccgtagatattacgaaaaacacagacctgtgattcttgatgtttttggcagggcagacggcggtgacatttcagagcttgcggacggtacggtaaagggcagtgtgataagcggttattcggctctgacggtgtgttcggagaaacctgcggatattgatttgagctatattgacgataagtcggctgtttttaccgagcttacacgctcatactttgcgaatgcgcacggcgactggcttttagtcgatttttcggatattgtaaagccgatttacaggcataggtcggcgtatgtcgcatcaattgatgaattatgctgttctatggcttacagagcatttatgacggacgatgaggttttcgagccgttcaaggaaaatgctgacagcaaatttatcgaaaaagcgatttccgattttgcaagaaccgtaaaagcaaaatatgggaaaaatataatattaaggaaaacatatcttccgcttaacagattggatattacaggaagaatccgtccttttgacgatacggaatttatatccgagaaagaaaatctgataagcagagcagaggagatatttgtaaaatgcacagactgctatataattgactatgaaagccggtatctgcctgtgtgcgccgataaaaacgccgatatttccgagcgtatgcttgaaagcgacttctataaggaggcggcagctgccgttgaccgcataatttcgggaacaagcaaaaagacggtaaacaatgtggatatagtcggctatcttgagcggtgcgagcgtatcagaaaggataaccccgatatgtctgccgagctttcccgtgagatattcggcggtgcgtcggagatattcatgacagaatga

SEQ ID NO: 63 - DNA, 3456 bp, Eubacterium siraeum
atgctgaaagctccgcaaaacttgttcgctaccgcttatgacggatctgtgcgatccgactggcagacggtagagggcgcagacggctatatattgcagttctataatgcagatgaaccggaaaagtgcattaaaacacgctatgcacagaataattcaaagctgatacttgggtttcgcaacggcagaaagtatgttgtacgggtaaaagcgttcagctatcgtgacgggaaagaggtatgcggtgaactgtcacagccggcagaatttacgccgatgtgccatcaccttaaagctcagaatgtaattacgatgaacaagggtgaaacgtcgcagatagtatgggaatgcagaaataaagtgcctgccgttacttttgaatgcgatgacagcgatgtggcgaccgtaacaaagggcggacaggttaccgctgtttcggacggcgcggctgagataaagctgacggctgatgacggtcagacttttactgttaagatagttgtcggcagggatatgtcacgttatccggctacgggaagaatcatgctctgcggcgatataatgtgttcgcttgagcatcagcggaaagccgctttgcgttcgcttgattttacagacgcattcggaacgcttaaagatacggtcagttcagccgattatgctgtagcggtgcttgaaaccacctgctttgacggagcaccgtttgaatatgaaaagatacgcacagacagcggaagccccaattgcaattctccgtccaccttcatagacgcagtgaaaaactgcggattcaatgcactggtaaccgctaataatcataactgtgatacagggcttgaagggcttcacgctaccgtacaacgtatcagaaacagcggtatggcaaatatcggtacgcttgacgatgaaactcatattgccgatataaacggcataaaggtaggatttgtcgcagtaaattcaatatcaaacgggcttgagaaaaatataccgcccgaaattatcgggaaatatgagcctgagcatttcagacagcttgttgaaacgctaaaaaatgaaggtgcagagtatataatcgcatatcagcactggggtgttatgaattccgtcactgtccgcaattctcagataaagacagctgaatatatggcacagtgcggcgtggatcttattatcggttctcatccgcacgttatgcagagggtcggtaaaatacacacatccgccggcagagatgtgacgtgcttctattctttaggcaatcttttgtcatcaatgaaagagcttcgtgaaaaccgtgagagtgtaattgtaaatctgattctcacaaggaccgaaagcggagtaaagtctgatatatcgtgcattccgacgctttgcaaggatacatccgacggatatacggtaagcgttcttgacgggttgctgacacaaacagaacagatttccgaagatcgcataagagatatactcggcaaggagggcgttatacgaaaacaccctaaattcttgctgcaaggctcagccgtgctgagaaatattttccgtgacagcggcttttcttatgacgataccgctcttattctgtcgcccttatcgcttgtaagcaaaaaaagtaatctttcgggaaaagccggcagccaaagaaataaaattgatataaataaaaatttcaaatcgtttttagacggctcagacagcgattatatcgtaatcgacctttatacagcggcggctgtttcgtgctacaagtacggcgacagcttctatacggcatcaggcagttttatttcttccgatttttacaattccaataaagacaggcttgaaaaaatttctccgccttttgacgaaaaaacagtaaaatctgcacttaaagaatatgcgaaaattgtcttgtcaaaatatgataaggataaaatcatattagtgcgtttaaaattcagcaatatctgcgtaaaagaaaatcagctcagaaacggtaaaagcagaaatgcgttgaataagcggttgaggctgtatgaggattatctgatttcgcttttacagccggtggttattgatgtttcctgcaattattttatggcgtcaaaaagtgacaatatgatgtcctttgagccgcttttctacgatgatgtaagaatcaagctgaactcagcggtaaaacgtatccgcaaggatacatatttttctgcaccggaaataaggctgcagcttatgcgtgtcataaaatattatgataatatgacggcaagagcctatcaacctgaactgcttgacagaaattttgtatcggacagaatggcagagcttacatcaaagcggtttgtcgcagagaatttcgagtattttgtatatctgcgtgaaaatgagatccgtacctatgatgatgcaaaaatcctgctttccgctaaagccggtgcagaaaggcttgtttcggcgataaaagccgctgagtgtattgacggcgaccttggcgattgcagttacgataatataaggattgttttcgatgagaacttccttatgaaaaaacaactatcccgtaaactttctgaggtttacaaatatactgttcccgataactgcgaacatattttccttatcagaaacgaccgcaaattgcttgaagactacaaagcacagcacaaacctgtattggttgacatctggggcagctgtatttcccgtgaatccgttaaccgtaattcatcaggtatctatgtcgataagtacattttcaagcagccgtttttgcttgcggacgagcctgaaatatcgtttgacaacgatttgtcggctgataaattctgcggcagtaagtggcgaaggcgcactgttaaagaggcgtttttgcacgaaggaaaacgcattctatctgatagtaatgccgaatggctgattattgatatgtacgaccttatctgcaatatgcgtaagtgcggcgattcgcttttcgaggtggatgatttcatacttcgcaccgctttttacaaatcgatttccgataaatgtgaaagcacatatttatttaacgaaagaagccgtgaatatctcgaaagagtgcttgaaaatttctgcaaatttgtcactgagcgctatggaaaaaacattattttaattaaagccgatcttaaagaccgttatatttcgcttgacaatcggttagaaatgttatctgacagcgataacacattcaaaaccaaaaaagcatttataaacggatttgaagaagaattcgcacgtcttaccgattgctgtgtaattgatatttctaaaaggttttatgccgatgaccgctttgcacttggcggtgcgcatatcgtccattatgaagatgagttctacagtcaatgctgtaagcatataacggctttcctcggcggttcggagagccgctataccgataaagtcgatgaggagtatatcgctctgagagatatgaaaattaaataa

SEQ ID NO: 64 - DNA, 3345 bp, Eubacterium siraeum
atgaagataagtaaggcgattgttgccgctgtaggtgcggcggctgccgtaggtgcggctgtatacgccaagaaaaagctggaggaaacacagactccgctcagaaagaaaagcctgaccgtatggaaaaacggcggggtaactcataaggagataatcagaaagcctataagcgaggaagaacagaccgatgcgataaacagccgcattgatgaggctgtacgccggtataagcctatgtccgaaagggatagcggcgaaaccgaaaccgagcctgaaatatcgcctgtcaattttacatttactcagagtgaagatgacgacgataccggtgtgagctttgagcgtgtattcgaccatttcaacaggcttgaatcgtccgtcggtaatgaaggcgaggatgtaggcgaaagcggcaaaaaagctgaggatacagccgaagaagccttatccgcagtaacggcaacggcagttgaggaaaattttgacgagcaagccggaatgccgaagcagatgctgcttgaaaatgggataatggcatccgctccgatagcaaatgcggttcaggagcttgcagaaatgccgtctgttatacaggataatgaagaaattgaagacgtaagactgcctgttgatgagagcattttcgatttatatgcaagcgagcctgtcgaggacgcagtaaaggcttttgaagaaatagccgagcaggaagaaaccgccgacagcgaaactgaaattgacagcgaacaaaatgacattgctaccgaagaagccgtaagcgagcctgtcgaggacgcagtaaaggcttttgaggaaatcgcagagcagaaagaaactgccgacattgaaactgaaattgacagcgaacaaaatgaaaccgccaccgaagaagccgtaagcgagcctgtcgaggatgcggtaaaggcttttgaggaaatagcacagcaggacgaaaccgccgacagcgaagctgaaagcgaacaaaatgaaactgctaccgaagaagccgtaagcgagcctgtcgaggacgcagtaaaggcatttgaagaaatcgccgagcaggaagaaactgctgacatcgaaactgaaattgacgatgaacaaaatgacactgctaccgaagaagccgtaagcgagcctgttgaggaggcagtaaaggcttttgaagaaatagccgagcaggaagaaaccgccgacattgaaactgaaagcgaacaaaacgacaccgctaccgaagaaccggtaagcgagccagtcgaggacgcagtaaaggcttttgaagaaatcgccgagcaggaagaaaccgccgacagcaaaactgaaattgacagcgaacaaaatgacactgccgtcgaagaagccgcaagcgagcctgtcgaggacgcagtaaaggctcttgaagaaatcgccgagcaggaagaaaccgccgacagcgaagctgaaagcgaacaaaatgacattgccgccgaagaagctgtaagcgagcctgttgaggacgcagtaaaggcttttgaagaaatagccgagcaggaagaaaccgccgacagcgaaactgaaagcaaacaaaatgacactgccgccgaagaaccgataagcgagcctgtcgaggatgcggtaaaggcttttgaagaaatcgccgagcaggaagaaactgccgacagcgaaactgaaatcgacagcgaacaaaatgacactgctaccgaagaagccgcaagcgagcctgtcgaggacgcagtaaaggcttttgaagaaatagctgagcaggaagaaactgctgacagtgaagctgtaattgacgatgaacaaaatgacactgccaccgaagaagccgtaagcgagcctgtcgaggatgcggtaaaggctttcgaagaaatcgccgagcaggaagaaactgccgacagcgaaactgaaatcgacagcgaacaaaatgacactgccaccgaagaagccgtaagcgagcctgtcgaggacgcagtaaaggcttttgaagaaatagccgagcaggaagaaaccgccgacagcgaagaaaagtcgctcgaagaacagttccacgctataatggaggaggaaaccgcaagcgagcctgtttcttctattcgtacagccgagtctgtagaggatgcattgaaagaattcggcgactttataggattatccgaaaccgctgacagcaccggtagcatcggtagctccgaagatatttcggatgacgatcttgaacagacaagcggtatttttgaggaaagtacattatccgatgagctgtccgaaactccggacgagccgattgacgctgacgaaaagccgagaactatggactttttcgatttgccggacgaagtatatacgcctgtacagcttaccgaagaaaagcacactgagaatgttgccgaggtagaggatctgttcggaaatctgcttatggatgacgagcctgaggtaaagaaaacatttaacgatccctcagaggtattttcactgttcgatacggctgacggcggacaggacgatttcgacaagtacagcgatgaaaagattgaggaagaaagcgagaaaaagaagaccagcgatacaagaaagtacatagcgcaggatattgcggataatatcgcatcgtttgcacagctgcttgaaccgctcaatgccatcaaggagaacaagatacgcagtaagagcggtatactgttcgactgggaaatgagaatacaggcgcttataggcgatttgccgataaagacgtactggagaaacaacttccgcaattatgagatatggagcgatgaaaagtgcatggaaaaggcaggcgagctgctctctatgcttgagcttgtcggaatagtgcgtgataaggcaaaagaggtcgtgatagacaaggatacgcttgatttctattcggcacagagcgagcatctcaacaacgatttccatataggtgaaactgtcgttgttacacggccgtgctggaaaataaacggacaccctgcaagaaagggcgaaattgccaagaaagcaccgtttgcggaattcagccgtaagaaagtatcaccgcttgaaactatgctgagagaaaacagctgttctgacggggatgttaatattcccgttacggaggacaatttctgtacatacgaccgtgatataccttatgtaaagagggcaatcgccgaaggcttctgcaagtgcgcagtaagacgtatggaggacggaggcgctctggcattcttctatgaggttattgcggagggcgaaaatgttcactattcgccgtgtacgctgagattcgaggtaaacattgacaagaatgcaaatgttgtcggaagattcagaagcgaaaaagtgtaa

SEQ ID NO: 65 - DNA, 3141 bp, Eubacterium siraeum
atggcggcaacggcaaaaagcagatatatgacggcggtaaaatggtttacggcatttgtatgcgctctgctttgtgcggctgccgtctgctgttttacgggaagcagtgcagacgctgcggcggtaacaaactgcaaggtttcggggctgacaacaaagacctatacgggtaaggcacagacgcagtcgatcacggtaaaatacgggaataaaacgctgaaaaacggcaaggattacacggtaagttatcagaataatataaacgcaggaacagcttatgttattataaaaggcaagggcagttacagcggaacagtaaagcgttcgttcaagataaaccctgcgttgatatacaagcagtgtactttttataaaatcgcctcgcagtattataccggctcacagataaagcctgttccgaaaatcaagaacggaacaacgacactgaaaaacggaacggacttcacgcttacatatcagaataacgtaaacaagggtactgcgaaggtatatataaaaggtaagggcaactacatcggaagctgttcgctgacattcagcataacggcaaggcctgtttctacgctgaaaatcaccgtgccgtcagtgacttataacgggaaggcacaaaagcctgccgttacggtaaagtataataactatacgtttaaaaacggtactgattatacgctgagttataaaaataacacgaaaatcggtacagcaaccgttacggttaagggcaagggaaagctcagcggaacaagaagcgttacattcaagataaacgcaaagccgataaaaaacgcagttattacatataacaactcgctcacatacaacggctcggcgctaagccctgcggttactgtaaaatacggaaacgcaacgcttaaaaagaataccgactataccgtcgcctactcgaataacgtaaatgccggcacgggaacaatcacgataacaggaaaaggcatatacggcggaagtgtaaaaaagacctttacaataaagaagctcggaatatcggccacagccgtatcgggaacaggaaacaaggtctatacgggaagtgcgataaagcctgtacctgcggttaaagtcggcggcaggatgctgaaaaacggaacggactttaccgtaagctataaaaacaacaccgagccgggaacggcaactctcaaagtgacaggcaagggaaactattcgggcagtgtatcaaagaccttcaaaatcaccgcaagagcgataaacgatgttgaggtaaccgtacccgatacggtatttaccggtgaacaggtaagacccgatgttgttgtaagctacggcaactatcaatttataaataacagcgactataccctgtcattcaaggacaacgtcaatatcggtacggcaagcgtggtggtcacaggcaaaaaacatctcagcggaagcaggacggtaacattccctatagaaaaggcggatatttcaagtgcggagatagccgtgaagaacgcaacatttacgggaagtgcggtaaaatccgacgttgatgtaaggctcggtaatgtgacgcttaaggaaggcactcactacacgctttcctataaaaacaacgtcaatgcaggtacggctcaggtgacagtcagcggcaagggaagccttgagggcgctgtaacaaaggatttcactattgcaaaggcggatatttcgaaagcctcgatttctgcaagcggaacgtatgctccggacggtgtaaagatcggcataaacgctaaactcggcaattacacgcttaaaagcagtgactacagttttaccgctccgaccgctgcgggagagcagacgctcacaataagcggaaacgacaacttcagcggcaaggccacagtgaaatgcaatgtggcaaaagcggatatagcaaatgccaaatcgtctttatcgctgtcaaccgacggcaagggctataccgtaacggtaatttatgacggtgtgcttttaacgcagaacaaagattataaggtagctgtaacagaatcaggcacaggcgtcagtgcggttattacaggcatcggcaattacggcggaacagcgactctcagcggcataagcaacgagcttgaagcgtttgaaaatgctgttgtcacaataggtaaagtcacatacaacggcacggcacagcttccctcggtaacagtgaagataggctctgtcacgctgaaaagcggaacggactatattctgagcgcttatgataacactaatgcaggaacagctacggcagttatcacaggcaagggaaaatatgccggtgcggaaaagaaaacgcagttcacgatagcgcctgccgccatatcatctgcaagcataagctgtgaggatcagatatatacgggacatggcgtcaccgcacagcccattgttacattcaacggcaaaacgcttgctctcggtattgactactatatatcgggatattcaaacatagtgaatgtcggaacagctaccgttactgtaaagggcaaaggcaatttcacaggcactgcaaaaggcactttcagaatcgtcaagcaggacaatatggaagcgcttgtcaagaagcgccttgatgagatgatggaaggcaagtgggacaggaagatatatgactactggcacagctatcagattggcaagtattacaacacgctccttacctctccttgtacctgccactcctactgtgaaacgggcaacgaggcaggctgtacctgtcttataggaagaagtcacgttctgaataattccggcatacagtgtgcgggatttaccatcgaggtgttcgagtatcttttcggcaaaacaaacggaacgggcgaaaataccctcacgataaggaatcgttccgacggaaactggacagaggcggcactgaagaagtggatgaccgatacgttccgtccgggcgactatctcgcatatgacaacataaagtacggctatccgcactatgtcacgatatactctgttgataccgacggtatatgggtgtacgaggcaaattacggcggaaggtgcaaaatcaatttccgtaagtttacgtttaaggagatttacgaagaaacggacggtttatggcacaggacaccgaacaattatgagttgtcggagtattga

SEQ ID NO: 66 - DNA, 2898 bp, Eubacterium siraeum
atgaaaataaaatttaaacgcattacagctttgtttgcggcacttgctattatgataaccgcactgcctctgacaatcatacctatcagtgccgcaggcaccgatggtgaaagcacagagtatgcaagtgacggataccttatcgtccgtagttaccggcagctgagattggcatacaacggcagtgaggagtctaagataaggcttggcgcagatattgactgcgaccctgaggaatataagcctaactatctgacgagattgtgtccgcctatagaaagtgacaagacgctggaccttgccggatatacgcttaaaaagacaggtaacagtattgactcgaaggatcatctgttaagcgtcgaatacagtaagctgaccattgaggattcggtgggaacgggtaaaatgtatttctatgccaaggatgtagcccagaatctgtttttggctgagaacagaagtacgatcgttataaacggaggtacattctgctacacgggtaccaatgcgatgtattgtgaaatgatcaagctgagtgcatcggatcttgtaatcaacgatggttattttgacgcacagatcggtactccgataaagctggataacggttttgccggcaaacaaagaacgcttaattctactgctctgataaacggaggtactatagtaactacctccagtatagcgctctcctcgatagacggttgtgattattacgcatcgctggttatgacgggcggaaccatcacaaacaagagcaagggcagagtgaccgataaaacgggaacgataatttccgatccgtattttgtccgtgttacaagtgacgaggcgttacagaaaaagtattacaacataacgctcctgggcggaaccatgccgcttagcctaaatgatatagaggtatattatcctgccgagaaggcggtacttacttctaaagcaggtacgatcacaaattctgcagaaaaggtagagtacacgactctgcttaccgcaccgcaggccggcattgacgaaaagaaggctatggcagcaagaggcgcagacgaaatctgcaggctgaagacagacagaaataattatgtgctgagcaataacaaacgcacacgttttaccgtcaacagcaacagcgtaggtaagattgacctgctcactcaggctcccaatccgtacaacacgggcgatccgataaaaacggtagattggtatgtgtccaagaatttcggctcgttcacatcaattcccgaagctataaacgatctgtcgtatacgccgccggaggttacggaaaaatgcacaatgctgtataaggctgttataaattacggcaatgtgctgagaatcaacgagataataataattgattatgattttgaagccgtaacggaaatcaaggcggtcgtgtcaggctttcacggaggttcgacgttaagcgacgtcagcgttgcgtcgggtgaacccgaaaaatacagtctgacgataaacaatatccgtgatgtttacggaaacaatatagtaaacgatcgtcagctgtgcaaaggcttcaaatacaacatatttgtaaaagtaaagctgaaaagcggatacgttgcagcgtatacaacaggcacagtaaagatgcgcaggtttgaggatcccgcaaatgaatggcaagcggcagaccatatttacatcggccttaacgagattgcatttaagagcgttcttgtttgcgacgaaggaatcaggacggtcggggtcgaaatcagcaacttcctgccttacagaaaggtaaacgatctgcagcttactgaatcggaacctgataaatatacggtaactcttgtcacgccgcttttaaacacatgggaatataacgaagaggtttacgacgatgacgagcttatagtagataactgttatgcggtcaaattcaaggtaacgcctaagtcgggatatgcgctttctcccggttatatattccgatgcaggcttgatacttacaaagaaggattctggctgacatccgaagacaaggaactgttcacggtttccaatgacggaacggtagtgattaacagtctgagggtgccgtttgaagaatatgatcagaatatatatgtacagataacacctccgaaggcaggaggaactccggcaaagagtttaatctcacataatcttcctgagcatatgagccttataagtattgactggtatgacgatgaagagcggaaaacaccgactgtatttgagaagggcaagacgtactggtgctatatatacatcaatgccgactgctatgagtataatctcaaaaaagcaaaattctatctgaacggaactcaggtcagacaggattacagttacaattcaaaagagaactactactatattctcggttatacggaaatcaagatcgacaatgatgttgcaactcctacaggctttgcggctggatcggcgacttcatcgagtgtttcgctgaagtgggataagaacgcaaatgcgagcggctatgagatagagcagtacaaaggcggaaagtggacacagattgcaaagataaataacaactccacggtttcggacaaagtaagcagacttgccgccgatacaacgtacacgttcaggatgagggcatataagactttatcgtcgggtacggcatacagcgactatgtaaggcttgcggcaaaaacgcagcttacaaataccgacaaatttgtcggcaccgcaatatctcctacagctgtaaagctggactggaacaggaatgataaggttacaggctacataatcgaacagtacaagggcggaaagtggacgcagatagcggtaacaaagaacaacacaacgcttacctttacggtaaaggggctggcggacgcaacaccttattcatccgcataa

SEQ ID NO: 67 - DNA, 2556 bp, Eubacterium siraeum
gtgcagttaaacaccaacggtcagaagtttataaatataataatcggcttttcacgggattttccctttaccgtaaatccgggcgaacattccgagaaaacctacccttctcttttagagctgataaatcccgatgatattcctccgataaccgaaatgttcaccgatgtatcacaggacgaggaaaagcgttttgaggcgcattgtcgttttatggtgaacgatgaatatcactggtttttcctttcgtgcaaggcggtatatgcagagtacggcaggcctgtgcgttttgagggaacgatgtgcgatgtatcgacctaccttgaaacagcgggtgacgaccttgtatataacgaattccgcaaaaagcacaatataaagctgtccgaacttaaaaaaggcgcaccgggtcttgccgatgtgcttgatgtcgactacctcacaagcatacagcgtccttttgccgtgccacagctttattccgccatatttgacgaaaaaggaaagctgatatgtgcgccgaaaacacagcataaatctctttctcccgatgattttgcatatcagaagaaaaagaatatccgcataaatcaccttgtcagcggaacgtggatactgggagcgaaaacgcaggaattgctcgatgacaacattcagctgtgggaaacgcttgtacagacagtttcccgtatggcaaacgcatttgttgtagttctttcggagatggacaattcgcagaatgcaaacaaactgctcggtcagaatgtcgaggagcagatactgctgaataatatctacgctatcataatgcagagcaaaagcgcagatattgcgttaaactccgttacagagcttataggcgattattttcaccttgacaggataaccataatcgaccgtgatgattttactcaggagctgtgctggtgcaaggattacaagtaccgccacctccctcttgaaatagacggcgataccgcacttgactgcgcctcgatacgtgaggatctgagccttacgtcatcggctttttcggatacggataccaacgaccttgcaaagttcggtatcaagtcgtatgctatcttcaagctgataaattctggcacttttgacagccttataatgttccagacgattgaaaaggaacataactggacacagcgtgagcgtaaacagctccgcaacatttcacagataatctcctcgcttatgatgcgtaaggaaacgcaggataagctggagcagtcgcagaagcgtatgcgtcagcttgccttttatgacgctatctacaatattccgaaccgtgcaaggctgaacaaggatcttgacaagataatgaagcgtaatacaaaaggctcgcttatcgctttcaaagtcaccaacacacgcactctgtccgcagtttacggtcacacctattcggatatgctgctgcgcagtatcgctcagtatcttaaggacctgcccgtaaaggatattggtgtatattatttcacaaatgcgatttttatgcttaatctaccggattgtaccgacaatgaagctaaaaatcttgtcgaaatgctgatacaccgtttttcaaagccgtggaaattcggtgaggatgagcattcaatccattgcagtctcggcatagcgttctatcccgaaaacggcgaggatgcagaggagctttgcaaggcggcaagcacggcaatgtaccgtgcaagagaattcaaacagaacagttatgctttctattcaggctcgcttgagcgtacaagaatgtttgcggcaagccttgaacagcatataagagaatgtataaacgacggtatgaggggcttttcactgcgttttcagccgtcattcagtgcggtcgacggcagtataatcggctgtgaaagctttgtacgctggcacgacgagcagtacggcaatattcctaactcaactttgttccctatggctgaaaatctcggcttatcccacgtcatagacggctgggtaatggaacgttcgtgcgaattctgcaaggagatacaggacgcaggctttgagaattttaccgtcagcgtaaatcttaccgcaggcgaaccgcaatctgccgaaatcgtaactcaggtacgtcacgctcttgaagaaagcgcactccctccgtcctcgctgatactcgaaattcctgtaaaggccaacattttctacagcgacagcacccatatcctgcacgatctgcgtactctcggtgtaaatattgccatagataaatacggcacggggaatatttcgttaaaggtcctcaaaaactcatacgtcaaccttgtgaatcttccggcaaagctgtttatgaatcacgaggacgaatttgacactgagcttgtaagctctgtcatccatctggcaaaatgccgtaagcttaccgtatgtgtaaagggcattgaggacaaggaacagcttgataccgtgcagaagttcgatattgacaggatacagggctactactgttcacgtccgctgtcgctgtcggaagcaaagacagtatttaccgaaagtataagaataaagggatactga

SEQ ID NO: 68 - DNA, 2256 bp, Eubacterium siraeum
atggacttaaagctcacgcaaggcatgaaaaaacgcatactggttattctggtggcattgtgtataggtgtcaccggcattgtcagtggtgtgctgttcaaggtttcggtcattgacagcaaggaactgtctgcaatggctaccgatcagcaacagagcagctttgacataaaggcaaagcgtggaacgatatacgaccgcaacaacaaggtgctggcgcaaagcgctaccgtgtgggatgttatcatttcgccgggcgacattgaaaaaaacgagcctgagaaccgtgagtttatatgcaagggaataagcgggatactcggcactaaatatgaaacgctgacggaagcgtgcaaggacacttcttcacgctattatgtggtcaagaagaaggtggaccgcagtacagttgaaaaaatcaacaacttcgtactgaagaacaaccttaaccgttattccgtttacactgttgaaaacagtgagaggagctatcctaacggaactcttgcggcaagcgttctgggatttgtaaacgagaatgaagagggctacggcatcgaggcatactacaattcgtatcttaagggtacggacggcagagttatcacaacaacagacgctcacggaaacgcaatgccttatgactattccgcacgctattcggcaaaggacggcaacagccttgtgctgactattgacgaaacgcttcagtattatcttgaaaagaatcttgaaatcacggtttcacagcataagctggcgaaccgcagtacgggaattattatgaatgcgaaaacgggcgctattgtggcaatggcgacatcacccggattcgatccgaacgatccgtcatatgtttactttgaaagcgacaggctgacgcttgccaagatgtcggcggacaagaagaccgaagaggaaatacttgctaaaaagcaggagatatggggaaagcagtggcagaacaaggcagtaagcgaactgtatatcccgggttctgtattcaagatgttcacctgcgcttcggcacttgaggaggaagtcgtatcgcttgacagcacattcgaatgctcgggcattgcagatgttgcgggaacgaagataagatgctggaacataggcggtcacggtgtatcgaatcttacagaagcgatgatccgctcgtgcaaccctgcatttataaagataggtcagcttctcggtgtggagaagttcagcaaatatttcgaggcattcggctttaccgaaaagacgggaatagatctgccgggcgaagcggattcgctgtatgtgaaagaatcggacatgggaatagttgagctttccagctcgtccttcggtcagacgacaaaggttacgcccatacagatggttacagcggcggctgctgtcgtaaacggcggtaagcttgtcacaccctatgttgtggataagataatagacagtgacggaaatgtcgtgaagtctgcacagacggtggtaagacgtcaggtaataagcgaagaaacaagcgcaacgatgcgtaagatacttgaggacgttgtaaccgcaaacggcggcggtaacgcatatatgagcggctatcgcataggcggcaagagcggtacttcggagaagatagacgactacaacagcggaaagacaccggaactcagatatgttgcgacattctgcgccatagtgccgatagatgaccccgaatatgttatgcttgtcgtatgcgacgagcctacatcgggatatatctacggcagtgctattgcggcgcccgtagtatcggctgtgttcaaggaaggccttgaatatatgggaatatatcctcagtatacggctgacgagcttgcacagcaggatgttactgttccgtgggtcggaggatataacagtataagagcggaggcacagcttacagccgcaggacttaaagcagagtacataggcagtacggacggtacagaggtaacaggtcaggtgccgtcggcaggtacggttatgccgagcggaagcacggtaatgctgtatatgggagacattccgttatcggattacagaatgtctactgtgccgaatgtaataggaatgacggtcgaagaagcaaacaaggcactgagcgaggcaggactcaacataagtattaccggtgcggcaacgggaagcgaagcaaaggcggtaagccagagcgttaattccggactggtggtatacagaggatctgttatagaggtcaatttccttgtaaacaacgaaacgggctga

SEQ ID NO: 69 - DNA, 2205 bp, Eubacterium siraeum
atgtcagaagtcagagctgttcagaaaaccgaaatgcccgagataaatgctcaggcggcaatcgttgttactcagcatgagggtcgcatactgcttgaaaagaatgccagaatgaaactgtcgcctgcttttcttattaaaataatggcatctataatagctctggaaaaatgtaatcctaatgataccgtaacagtatcggacagcgtcataaagcagatttcgaactggaaaggctcggcgtctatcaatcttgaagcaggagaaaaaatatctgtacttgatttaatttattcgatgatgctggtttcagccaatgactctttatttgctcttgcggaattcatatgcggaagccttgacaagtttgccgcaatgatgcaggagaaggctaaatctatcggtgcggcggatacaactgtgactaccgctgacggcagatttacagcggagcagtattcaaacgcatacgaccttgccatcatctgccgctactgcatgaccaacagaatgttcagaacaatagcggctaccgataaatatacaatcccggcaacgaataaaaacggctcaagggatctgcagaatacgaatcttcttattaacagcggtaacagaagatacagatatgaaacggctatcggcataaaaagcggatatacggctcgctcaaaatcgtgccttgcctgctctgccctgccgcccgcaaacaaattcggagaagaagtgcttgcaataatactcggagcagaaaacacaaagcagatgaaatacgttttctatgacgcaataacactgctcgacttcacgttcaacaattatgaagcgctcagcggtaaaaaaccggaacagcagaattccgaagcggaaaaatccattaccacagtaggaaagctgtgtgaaattcttaatgctgagcttcgcaatgccgcagacgttccaattacatcatttgccttcggtaaacagaaaataaaacccggatgtgcatattttgccgccgataaggaaacggctgtcacggcatttgaaaagggtgcggctgttattatcacaactcagccgatagagaagattccgaatatcgttgtggcaaatcttgataccgctctcagcaggaccgcagtatttataaagtcggcactgggaatgtggactgtagctgttatggacagtcccgaaaagataaatcccctttcgatgatagaacaaatgctttcgagcaagatggaaaccgtgcattcaatttccgttacaaacaactacaattcaatgctccatgcaatgtttgcttctacacctaaaaccgagacggctgtcatcaatgtttcgtgcgtaaacggaggaaacgttgaacgtgtttcgcagacagccaactttgatgttgcgatacttacaagcacggtcgtatccaaaaatccgagggaactgacaaagcctgagcttattgaagaaaaactcaaggtatgcggcggaatgaacgaatcgggtgcggtcatcataaatattgacgataagaatctcgcaggcatattcaccataccgcaggatattatcaccatcggcgttgataacagaatggctgattattttgccgataacatagagctttcccataataaaatctcgtttgatataatacacggtgcggataattatcatatcgagctttattccgatgataagcacagcgtatatcaggctctggcaacatttgcactgggcgagattatgggcataccgccaaagcagattataccggcaatcgaaaaataccgcccgtcaacaggacttacaacagtacgcaacgaaagaggtatttatgtaatatccgattttgaaaacgaggctgttgaaagcgtaggtgcggctcttaaggaactctgcaccatgcagcttcctcccgattcaagaagaatagcggtattgtctgaagtaggtgacggtgacgagcatgaacttgaaatatacaggaaggtcggcaatatcgtcaataaagcaagcgtaaatattacggtttgctacggtgaaaccgccgcagaactgatgaaaaccgccgatttaaaaagcaaattcgtaataaagctgaacacaagacaggctcttacagaatttttaaagctgaatctgcgtgataatgacgctgtacttttcaaaggctcgacggtgaccgagcttgacgaaattatgacggacgtcacataa

SEQ ID NO: 70 - DNA, 2019 bp, Eubacterium siraeum
atgaaaaaatggcttgtcagaaatacggacaatgcacttgcaatgaaactcaagaccgacacgggactgccgatgcttttgtgcagtctgcttgtcagcagaggaatatacacagccgagcaggcacagcagtatttcaacggtacggagctttccgaccccttgcttattgcggatatggataaagctgtgcaggcgatagaagaagcggttgacaatgaagtaaagataaccgtatacggcgattacgattgcgacggcgttacatctaccgttatgcttttcacacatcttgatgcaataggtgctgacgtaaactggtacatacccacacgtgaagaaggctacgggctgaatgaaaatgcgatacgcaaactgcacgaggacggtacgggtcttataataacggttgacaacggcgtttcagccgtcaacgaggcggagcttatatatgaacttggaatgaagcttgttgttaccgaccaccatcagctccctgagattctgcctaaagcggaggctatcgtaaatccgcacagacaagatgacaactctccctataaagaacttgcaggctgcggcgttgcgctaaagctcattatggctctggaacgtgacgttgaaggtgttcttgagcagtatgccgaccttgcggctatcggcactataggcgatgttgtcgcactgacgggagaaaaccgcataatagtaaagcgtggacttcttgaaatgcagtacagcgaaaatcagggacttcaggcgcttatcaatgcggcaggacttgatgccgaaagtattacttctacaggcatagcgttcggcttatgcccccgtataaatgccgcaggacgttatgacagtccgaaagcggcggcagagcttcttatggctcagaccggacagatagccgagataaaagcgcaggaactgaatgaactgaacgctaagagaaaacagatcgaaagcgatattctcgaaatggcaaaggctcagcttattgccgaccctaaagcgttcaactcccgtgtgcttattgtttgcggcgagggttggaatcacggaattataggtatagtcagcgcaagacttcttgaactttacgaaaaaccctgtatcgtcataggaatagagggcgatgaggcaagaggctcagcgagaagcatcgaaggcttttcactttataccgcacttgatgcgtgcagtgagcatcttacacgtttcggaggtcatacgaaggcggctggcttttcgcttccgaaagacaaggtagatgattttatagctcagctgagaagctatgcggatgaaaaattcccttcaatgccggttatgacaacggaggctgatattgagccggagctgtccgaccttgaaatatcttcaatcgagaatcttcgtcatttacagccttacggcgaagaaaacaacgctccgctgtttttgatgagaaactgcacgatcatatcatcaagaccgctaaaagacggtaaatatacatcgtttagcgcagagtataaaggctcacagtttaaatttctctgcttcggaacatcgtttgataagttcggatattatcccggagataaggtcgatgtgctgagccatatcgaaataaacgaatataatgataaaaaaagcgtcagcgtaagagtaaaggacatacgcagaagtgattttacgcaggataagtattttgccgcaagaaatttctatgaaaaaatcctcagaggcgaaaaaaccgattcaagacttcttaaacgtatcctgcccgataaggagaacatgaagctcccgttcgaccttgcaagaaagctgacctctatagattcagccgcacagattgcaatgtcgcacggtatgaattactgcctttttatgatgtgccttcatgtttttgcggaattcggtcatcttgagctggacagaataaacggtacgatgaatttcataaaaggcggcagacgtatagaacttgaaaactcggcagtgataagaagaataatgaaatcctgcagctga

SEQ ID NO: 71 - DNA, 1977 bp, Eubacterium siraeum
atggcagtatatcttatacttatggcacttgtgcttgtgctagcttatccgctcatcgagcataagccgaatgtggtgaagaagctctgttatgttatcgtgacattcggggcaatgtatcttataagcgtattcagatacggactgggaaacgattattattcgtatatctatattttctggaatatcaagaatgcacccggactttcgatattcaactacgggtatgagccgggctttacaatcgtcacaaagctgatctcgatgtttaccgcagatgtgaatataatgtatgcggtgtacgcactgctgatacttatacctacggcgtatgcgatattccgttacagtgaaaatatatggatgtcaacgatgatgttcatatcgctgacgttcttctactgctcgctgagctttatccgtcagtcgatagcgtttgcaatcatactctgcgcttacagatttatgaaggaacgcaatcatttcatggtgctgttgtttattttcttagcgtgtctgttccacagtacagtaatagtgctgataccgctgtatctgattgcggcgttcataaagcccacaaagataaccgtaccgatatatgcgatattgacagcgcttgtatatctgctttcgtggccgatactgcggtttgcggttgtgcttcttccgcagtacaagggctaccttgaacttaactttatcacgcagggctattcacctgtttatattatagtgcctgcgataatcacggcacttgcgcttatcgcacatttcacgggatacggaaaggcatatccgaaagagtcggcactgttcacgaactttgcgatattcaacttcataatatggtttatagcgacaaagcactttgttatcgagcgtttctcgatgtatctgtacattatgatgataatgttcataccgtcaatagcaaggtactatatgaactgcgcaaaggtttatcttgcacgcaggaaaaatcccgatgctgtggttgaattcgataaaacggtagatgaggtcatacgttccaagcatcccgaaaaatatgccaagaagtatgccgccgaacccaaaaaggaaaaagcggtttcgcagcccgtacccgaaaaggcggagcctgaactgagcgatatagaaaaggaaaagcagagaattttagccgaaatcatggctgaggacggcggcgacagcaatatagtgacaaagccgattgaagctgtggaaaacaaaaagcccgaaaagcagaagaagtattcgtctgtattcggagagcagtttaatgctgacgaaagatatatgccgaagaacagggtattcaaaaagagaaggaacggttttgtgaacttcgttacacgtcctgttacgatatttgcggctttccttgttgtagtggtgggcgctaacctgtggtacaactatttcggccttacggtatcgaagaagggcttccacggagttatgccgtacaagagcattgctccgcagtatacagaatttgtgctttcaaaagaaagcaaggacgaaaagaacactaacctcagaagcgaggataatttccttaactatatgtacaggctgaaagagggcgagaatttcactgccataatctcggcaagaggagatgtgacgggcggatataacgacggtgctttatcggctgtaaaggatctggggcttgaaaagctgcttacggctcagaaaaaccagcgttatattgcgataatagaaggcggcaaggttgtccgtgaggaactgtcggatgacaggatcgatacaggcgttattgatgtgctgggctataagacacagataatcagcgacgcagatgaatcgattgtcaaaatgggcaacaagaactactcgctaaacgagcgtggaatgaatatcgtggtgcttgacaacacaacgagaaacattgttgacaaggtacgtttcaagacgtattacgttatgctgtcggcaacaagataa

SEQ ID NO: 72 - DNA, 1881 bp, Eubacterium siraeum
atgaaaatatttgtatatgagatgaaaaagatactgataaaacagtacgcaataataattctggcagctgtagtaatagtaagactgctatcttctctgccgcttgcaaagcagacatacggatttgactctgctacagagagagagaaatattttgagataatctctccgtttataggagcagtgaccgaagaaaaaactgaccgtgcagacgagcttgaaaagcagcttgaaacggcaagtcaacaatacgataagctgattgatcagcgtctggaacacaaaatatcggatattgaatattacgagcagatgaagctgtacgaaccgaccctcaatatcaaaaagcagattgaaaaaactgtcgaacaggtacggcaggcgcaagaacgccaatgcgatattctgcctgtaagctatatccctataatatgcgaagcgtcggccgattacctttttgtgcttgcaatctgtcttatatgcagtctgagtgtaatcacagagtatacaagcaagacaagatatatcctgtgtactactccagcaggacagtcacgcagtatggcggcaaaaacgacagttctgctcttttcggtcgcagtggcatcggttttgctctcggcggttgagggatactgtctttcaaaacagcttccctttgaatactgggcgtattccgcaagaggtatagtgataatgacgaattgtacggcggagctttctataggcagtctgtttattcagacccagcttattaaactggtgggaagtattttcatcgcctcggttgcaattcttatttccgagctttttaaaagctattccgcaagcgtattttcgcttgtaaccgtgcagatagttgtcgactatgtcggcaatcgctcaaatctcagctatcttctgccgacaggggctatgcgtggctacggttatttttacggcgatgtcacgccgaccgccgaaaacaattatatgcagttttcgggagtgcctctttggtatactgcagtgcttatgtgcggtttgctgattttttctgtggcagcttgtgcaggaacgattctttcctgcaataaccgactgaaaagaaaaaggaaaaagatacgcaaggcggcacttttgtcaacgatgtgcattgtcacttcactgcttctgtcctcgtgcagtgttgcgaataaccgctacgaccccgaagatacaatgaagcttgtaggcggctcatataccttgatcggcgaatataacatcccttttacagaaggactgaaaacaagcaaatatgaaatcgttcttgagaccaatcagtcttccggtggattttcaatatcgctgatcgatcttgcaagcaatgaaaagctcgatattccgcagagctatttttcggacgaaactttcattcattgctttataaccgagcattacattttagtcgagtatatcgccaaagacggaaccgaagcaatgcggtactatgacctgaatgacttttcgacacaaacaattgctcagaacacccgaggagtagaaaaaaatctgttcggacttacctttaaggacagcgaaagcatatttacgacaagctccttggttttcaccgatgacagagattttttctttgttacagacagcggtttgtataaggtaggcgtaaataaaaatgcgtcactgataatagacgagcctgtaactgaaggcttgatttacgatgctcacagcatctattttatcagcgaaaaggacagcatcaagcgttacgacctttcaacaggcattctcagcgaaattgtaagcggtgaaaaaataatcccacgttcgctgtggggagattacgattatatttattacacaagcgagaacggcgaacaaaagttagcaaaatag

SEQ ID NO: 73 - DNA, 20 bp, Alistipes senegalensis
gcggaaggtaaggtcgaaca

SEQ ID NO: 74 - DNA, 20 bp, Alistipes senegalensis
aatacttttccgcctcggca

SEQ ID NO: 75 - DNA, 20 bp, Alistipes senegalensis
gtttcggtcgaagccggata

SEQ ID NO: 76 - DNA, 20 bp, Alistipes senegalensis
atcgtgcagatgcatggtga

SEQ ID NO: 77 - DNA, 20 bp, Alistipes senegalensis
ttcgagcaggccaatgctaa

SEQ ID NO: 78 - DNA, 20 bp, Alistipes senegalensis
gtattcagttgtccgcccca

SEQ ID NO: 79 - DNA, 20 bp, Alistipes senegalensis
gtgaccgtctggctgaaaga

SEQ ID NO: 80 - DNA, 20 bp, Alistipes senegalensis
cgatgccgcggattttgaat

SEQ ID NO: 81 - DNA, 20 bp, Alistipes senegalensis
cgacgatccggaagatgagg

SEQ ID NO: 82 - DNA, 20 bp, Alistipes senegalensis
acctcccgaacagaggatga

SEQ ID NO: 83 - DNA, 20 bp, Alistipes senegalensis
gctacacgttcgacaatcgc

SEQ ID NO: 84 - DNA, 20 bp, Alistipes senegalensis
cgaaatgccgtaagaagcgg

SEQ ID NO: 85 - DNA, 20 bp, Alistipes senegalensis
tcagatcagcggtgatgacg

SEQ ID NO: 86 - DNA, 20 bp, Alistipes senegalensis
gcaccttgtagcttttgccc

SEQ ID NO: 87 - DNA, 20 bp, Alistipes senegalensis
ttcctgaatcggttgctggc

SEQ ID NO: 88 - DNA, 20 bp, Alistipes senegalensis
cctcggcgaaatagtccgaa

SEQ ID NO: 89 - DNA, 20 bp, Alistipes senegalensis
cgtgccgctgaagaaaaaca

SEQ ID NO: 90 - DNA, 20 bp, Alistipes senegalensis
cgtaggttcccgaatagggc

SEQ ID NO: 91 - DNA, 20 bp, Alistipes senegalensis
aggtcgaaagccgaacttcc

SEQ ID NO: 92 - DNA, 20 bp, Alistipes senegalensis
tgcgtatatgggcgttctct

SEQ ID NO: 93 - DNA, 20 bp, Alistipes senegalensis
cgtcagtcgaagaggtacgg

SEQ ID NO: 94 - DNA, 20 bp, Alistipes senegalensis
cgacggcctccatctgtatc

SEQ ID NO: 95 - DNA, 20 bp, Clostridium boltae
gaggcataggcggaagtacc

SEQ ID NO: 96 - DNA, 20 bp, Clostridium boltae
accccgccggaattaatgtt

SEQ ID NO: 97 - DNA, 21 bp, Clostridium boltae
gtccggcgaaaacaggtctga

SEQ ID NO: 98 - DNA, 20 bp, Clostridium boltae
cctgcaccatgtcccctttt

SEQ ID NO: 99 - DNA, 20 bp, Clostridium boltae
cgggacatttgcatgaacgg

SEQ ID NO: 100 - DNA, 20 bp, Clostridium boltae
ctatgcgctccgctagcaat

SEQ ID NO: 101 - DNA, 20 bp, Clostridium boltae
ccggaccttttggctcagat

SEQ ID NO: 102 - DNA, 20 bp, Clostridium boltae
tccgcagcctcgatgtattc

SEQ ID NO: 103 - DNA, 20 bp, Clostridium boltae
gggcagtattcgcggtatca

SEQ ID NO: 104 - DNA, 20 bp, Clostridium boltae
ttcggcagcaccatcagaat

SEQ ID NO: 105 - DNA, 20 bp, Clostridium boltae
ggcgataacctgtgtgtgga

SEQ ID NO: 106 - DNA, 20 bp, Clostridium boltae
cccgctgtaaaatccccctg

SEQ ID NO: 107 - DNA, 20 bp, Clostridium boltae
gacaggccataaggtggctt

SEQ ID NO: 108 - DNA, 20 bp, Clostridium boltae
agcctgtagttgggaatggc

SEQ ID NO: 109 - DNA, 20 bp, Clostridium boltae
gggggacacatggactgttt

SEQ ID NO: 110 - DNA, 20 bp, Clostridium boltae
gttcccttcatgtctggcga

SEQ ID NO: 111 - DNA, 20 bp, Clostridium boltae
tattccagcccctacggaca

SEQ ID NO: 112 - DNA, 20 bp, Clostridium boltae
tcaacggcctcgcatatctc

SEQ ID NO: 113 - DNA, 22 bp, Clostridium boltae
attctccggtatttgcccaatg

SEQ ID NO: 114 - DNA, 20 bp, Clostridium boltae
taccagtgtaaggcggtcat

SEQ ID NO: 115 - DNA, 20 bp, Clostridium boltae
ccgcgctaaagattcatggc

SEQ ID NO: 116 - DNA, 20 bp, Clostridium boltae
gcttgcaaggctgtggtttt

SEQ ID NO: 117 - DNA, 20 bp, Clostridium boltae
ctgtgtaccctctgtgcctg

SEQ ID NO: 118 - DNA, 20 bp, Clostridium boltae
agattccgtttcagcccctg

SEQ ID NO: 119 - DNA, 20 bp, Clostridium clostridioforme
tgcatggatgataccgaccg

SEQ ID NO: 120 - DNA, 20 bp, Clostridium clostridioforme
ccgcgtttgtggtttccaat

SEQ ID NO: 121 - DNA, 20 bp, Clostridium clostridioforme
tcaaagatgcggcagaggag

SEQ ID NO: 122 - DNA, 20 bp, Clostridium clostridioforme
caactcctgatacgcctccc

SEQ ID NO: 123 - DNA, 20 bp, Clostridium clostridioforme
gggacgcccttctgattgaa

SEQ ID NO: 124 - DNA, 20 bp, Clostridium clostridioforme
agtgcaaacaaggccggata

SEQ ID NO: 125 - DNA, 20 bp, Clostridium clostridioforme
ccatcggatgtctggttgct

SEQ ID NO: 126 - DNA, 20 bp, Clostridium clostridioforme
tcctccaatagccaaacgca

SEQ ID NO: 127 - DNA, 20 bp, Clostridium clostridioforme
gcccagtgcagacatggata

SEQ ID NO: 128 - DNA, 20 bp, Clostridium clostridioforme
agccaatgcaccatagacgg

SEQ ID NO: 129 - DNA, 20 bp, Clostridium clostridioforme
tgtgccaggaacgggataac

SEQ ID NO: 130 - DNA, 20 bp, Clostridium clostridioforme
cagattcagctgcccaggaa

SEQ ID NO: 131 - DNA, 20 bp, Clostridium clostridioforme
gccgtggttaatgcatcgtt

SEQ ID NO: 132 - DNA, 20 bp, Clostridium clostridioforme
tgccggttgccttcgattat

SEQ ID NO: 133 - DNA, 20 bp, Clostridium clostridioforme
gctggcaggagtagtttcgt

SEQ ID NO: 134 - DNA, 20 bp, Clostridium clostridioforme
tggcggcaattgtttccttg

SEQ ID NO: 135 - DNA, 20 bp, Clostridium clostridioforme
gccgtcaggcgtattatgga

SEQ ID NO: 136 - DNA, 20 bp, Clostridium clostridioforme
cccttttggcgtcttcctct

SEQ ID NO: 137 - DNA, 20 bp, Clostridium clostridioforme
ccgttacgttgaggctctgt

SEQ ID NO: 138 - DNA, 20 bp, Clostridium clostridioforme
gtgcatacggtcatgggtga

SEQ ID NO: 139 - DNA, 20 bp, Clostridium clostridioforme
tagcggctgcaaatagcctt

SEQ ID NO: 140 - DNA, 20 bp, Clostridium clostridioforme
tgggctggatgaaaccacaa

SEQ ID NO: 141 - DNA, 20 bp, Clostridium hathewayi
aaggcggtaaatggcggtta

SEQ ID NO: 142 - DNA, 20 bp, Clostridium hathewayi
cgtctgcttcatcaatggcg

SEQ ID NO: 143 - DNA, 20 bp, Clostridium hathewayi
tatttaccgtcagcggcagg

SEQ ID NO: 144 - DNA, 20 bp, Clostridium hathewayi
gttgctgaattccactccgc

SEQ ID NO: 145 - DNA, 20 bp, Clostridium hathewayi
accacaattctctgtgccgt

SEQ ID NO: 146 - DNA, 20 bp, Clostridium hathewayi
tgccgggataaccaaactcc

SEQ ID NO: 147 - DNA, 20 bp, Clostridium hathewayi
cgcatcgggaatcgaagaga

SEQ ID NO: 148 - DNA, 20 bp, Clostridium hathewayi
attcagccctccgcctattg

SEQ ID NO: 149 - DNA, 20 bp, Clostridium hathewayi
ttctggaaaaggctgcggat

SEQ ID NO: 150 - DNA, 20 bp, Clostridium hathewayi
cactggctctcaagtcctcg

SEQ ID NO: 151 - DNA, 20 bp, Clostridium hathewayi
ggcttctacggaccgtttca

SEQ ID NO: 152 - DNA, 20 bp, Clostridium hathewayi
ttggcaatccagaatgggct

SEQ ID NO: 153 - DNA, 20 bp, Clostridium hathewayi
accaaccggctgattacgtt

SEQ ID NO: 154 - DNA, 20 bp, Clostridium hathewayi
gcctctgttcctcctcacac

SEQ ID NO: 155 - DNA, 20 bp, Clostridium hathewayi
tcacccaggacttaaaccgc

SEQ ID NO: 156 - DNA, 20 bp, Clostridium hathewayi
gaggcgcttatccagctcat

SEQ ID NO: 157 - DNA, 20 bp, Clostridium hathewayi
cggctggggaagattgtgat

SEQ ID NO: 158 - DNA, 20 bp, Clostridium hathewayi
caaaagcactgcaagcgact

SEQ ID NO: 159 - DNA, 20 bp, Clostridium hathewayi
gccggaggctatgactatcg

SEQ ID NO: 160 - DNA, 20 bp, Clostridium hathewayi
aatgagaatgcggccgtttg

SEQ ID NO: 161 - DNA, 20 bp, Clostridium hathewayi
ggccctgattcgggatcatt

SEQ ID NO: 162 - DNA, 20 bp, Clostridium hathewayi
ttccgcacattctcgacctc

SEQ ID NO: 163 - DNA, 20 bp, Clostridium hathewayi
caagccaacagagagccaga

SEQ ID NO: 164 - DNA, 20 bp, Clostridium hathewayi
actccaggtcccttctctcc

SEQ ID NO: 165 - DNA, 20 bp, Dorea longicatena
accggaagaatggacttcgg

SEQ ID NO: 166 - DNA, 20 bp, Dorea longicatena
agcggctggttacttttcca

SEQ ID NO: 167 - DNA, 20 bp, Dorea longicatena
agcttctgacgggagcaatg

SEQ ID NO: 168 - DNA, 20 bp, Dorea longicatena
caccgtctgatttcccgcat

SEQ ID NO: 169 - DNA, 20 bp, Dorea longicatena
tttatctggcagaagccgca

SEQ ID NO: 170 - DNA, 20 bp, Dorea longicatena
tgaacgccatgctgcaattc

SEQ ID NO: 171 - DNA, 20 bp, Dorea longicatena
cgatgatccgggcaacaatg

SEQ ID NO: 172 - DNA, 20 bp, Dorea longicatena
ccggcatcttctggtacgaa

SEQ ID NO: 173 - DNA, 20 bp, Dorea longicatena
atggcgacggaagtgcatta

SEQ ID NO: 174 - DNA, 20 bp, Dorea longicatena
cggtacagcaaacggtggta

SEQ ID NO: 175 - DNA, 20 bp, Dorea longicatena
aagctcaggcacagacgaaa

SEQ ID NO: 176 - DNA, 20 bp, Dorea longicatena
ttccgtccgccagatcaaaa

SEQ ID NO: 177 - DNA, 20 bp, Dorea longicatena
tcgattctggcgatagcagg

SEQ ID NO: 178 - DNA, 20 bp, Dorea longicatena
tgccaaagggaggctgtaag

SEQ ID NO: 179 - DNA, 20 bp, Dorea longicatena
tgcggacgggcagtattatc

SEQ ID NO: 180 - DNA, 20 bp, Dorea longicatena
tctttccgtcaaccgcagaa

SEQ ID NO: 181 - DNA, 20 bp, Dorea longicatena
ggccgctgtctattcgatga

SEQ ID NO: 182 - DNA, 20 bp, Dorea longicatena
agcagaaaactgcacccgat

SEQ ID NO: 183 - DNA, 20 bp, Dorea longicatena
tctgggggcattcgcatatc

SEQ ID NO: 184 - DNA, 20 bp, Dorea longicatena
accgacatctgtcatcgtcg

SEQ ID NO: 185 - DNA, 19 bp, Dorea longicatena
ttggctgggcgacattagg

SEQ ID NO: 186 - DNA, 21 bp, Dorea longicatena
acgtatttctcgccaaagcac

SEQ ID NO: 187 - DNA, 20 bp, Dorea longicatena
tccgaaaatgtgcaggggaa

SEQ ID NO: 188 - DNA, 20 bp, Dorea longicatena
acgccagttgtcctgctatc

SEQ ID NO: 189 - DNA, 20 bp, Eubacterium siraeum
taggcgatgtaacgctcgac

SEQ ID NO: 190 - DNA, 20 bp, Eubacterium siraeum
acaagcgtctttgcgttgtc

SEQ ID NO: 191 - DNA, 23 bp, Eubacterium siraeum
gagatatgcagagaagcccgaac

SEQ ID NO: 192 - DNA, 21 bp, Eubacterium siraeum
aggcgtggaaacagcgtaata

SEQ ID NO: 193 - DNA, 20 bp, Eubacterium siraeum
catcaaagcggtttgtcgca

SEQ ID NO: 194 - DNA, 20 bp, Eubacterium siraeum
cactcagcggcttttatcgc

SEQ ID NO: 195 - DNA, 20 bp, Eubacterium siraeum
atggaggaggaaaccgcaag

SEQ ID NO: 196 - DNA, 20 bp, Eubacterium siraeum
taccgatgctaccggtgctg

SEQ ID NO: 197 - DNA, 20 bp, Eubacterium siraeum
gctgccgtctgctgttttac

SEQ ID NO: 198 - DNA, 20 bp, Eubacterium siraeum
aggtctttgttgtcagcccc

SEQ ID NO: 199 - DNA, 20 bp, Eubacterium siraeum
aggctcccaatccgtacaac

SEQ ID NO: 200 - DNA, 21 bp, Eubacterium siraeum
cttaacgtcgaacctccgtga

SEQ ID NO: 201 - DNA, 25 bp, Eubacterium siraeum
gagatggacaattcgcagaatgcaa

SEQ ID NO: 202 - DNA, 20 bp, Eubacterium siraeum
gccgatgacgtaaggctcag

SEQ ID NO: 203 - DNA, 20 bp, Eubacterium siraeum
gcggacaagaagaccgaaga

SEQ ID NO: 204 - DNA, 19 bp, Eubacterium siraeum
caccgtgaccgcctatgtt

SEQ ID NO: 205 - DNA, 22 bp, Eubacterium siraeum
catttgaaaagggtgcggctgt

SEQ ID NO: 206 - DNA, 19 bp, Eubacterium siraeum
cacattcccagtgccgact

SEQ ID NO: 207 - DNA, 22 bp, Eubacterium siraeum
ttttgtgcagtctgcttgtcag

SEQ ID NO: 208 - DNA, 18 bp, Eubacterium siraeum
gccttcttcacgtgtggg

SEQ ID NO: 209 - DNA, 20 bp, Eubacterium siraeum
ttgtccgtgaggaactgtcg

SEQ ID NO: 210 - DNA, 20 bp, Eubacterium siraeum
cattccacgctcgtttagcg

SEQ ID NO: 211 - DNA, 20 bp, Eubacterium siraeum
cttctgtcctcgtgcagtgt

SEQ ID NO: 212 - DNA, 23 bp, Eubacterium siraeum
agggatgttatattcgccgatca

SEQ ID NO: 213 - DNA, 20 bp, Clostridium boltae
atgcctccagaacctccgcc

SEQ ID NO: 214 - DNA, 20 bp, Clostridium boltae
cagctgctgcttccggaata

SEQ ID NO: 215 - DNA, 20 bp, Clostridium boltae
aattcatcagtatttacggc

SEQ ID NO: 216 - DNA, 20 bp, Clostridium boltae
tccgcatctgctcatcatat

SEQ ID NO: 217 - DNA, 20 bp, Clostridium boltae
gtatttcacactgtcactgc

SEQ ID NO: 218 - DNA, 20 bp, Clostridium boltae
ctggagccgcatgttatcaa

SEQ ID NO: 219 - DNA, 20 bp, Clostridium boltae
gaggaagcggccagggaggc

SEQ ID NO: 220 - DNA, 20 bp, Clostridium boltae
cagacgaggaatattctgta

SEQ ID NO: 221 - DNA, 20 bp, Clostridium boltae
acggtctggaacaagaggaa

SEQ ID NO: 222 - DNA, 20 bp, Clostridium boltae
caggtacagagtcagttacc

SEQ ID NO: 223 - DNA, 20 bp, Clostridium boltae
agcccgccgcccaattaccg

SEQ ID NO: 224 - DNA, 20 bp, Clostridium boltae
agcctacttgctggcaggac

SEQ ID NO: 225 - DNA, 20 bp, Clostridium clostridioforme
cgcatcaacagcgaaccgga

SEQ ID NO: 226 - DNA, 20 bp, Clostridium clostridioforme
cgattcaagcagcatctgac

SEQ ID NO: 227 - DNA, 20 bp, Clostridium clostridioforme
cctaagctccgtctcatcta

SEQ ID NO: 228 - DNA, 20 bp, Clostridium clostridioforme
catgctgctgcaaactccga

SEQ ID NO: 229 - DNA, 20 bp, Clostridium clostridioforme
gcttatttatggaagatatc

SEQ ID NO: 230 - DNA, 20 bp, Clostridium clostridioforme
cagtgacggctattcctata

SEQ ID NO: 231 - DNA, 20 bp, Clostridium clostridioforme
gaacgggattggaaacagtg

SEQ ID NO: 232 - DNA, 20 bp, Clostridium clostridioforme
gcaaccggcaacaggtaaac

SEQ ID NO: 233 - DNA, 20 bp, Clostridium clostridioforme
gtacacgaagccccggaaca

SEQ ID NO: 234 - DNA, 20 bp, Clostridium clostridioforme
gccccagtccaggcggattg

SEQ ID NO: 235 - DNA, 20 bp, Clostridium clostridioforme
cagcttaaaccgttacgttg

SEQ ID NO: 236 - DNA, 20 bp, Clostridium clostridioforme
aattggacttggaagtcatc

SEQ ID NO: 237 - DNA, 20 bp, Clostridium hathewayi
cggattatcaggcggaacta

SEQ ID NO: 238 - DNA, 20 bp, Clostridium hathewayi
tttcatatgatccgtcatac

SEQ ID NO: 239 - DNA, 20 bp, Clostridium hathewayi
cttctttcgatggatttgca

SEQ ID NO: 240 - DNA, 20 bp, Clostridium hathewayi
agctgcgggccggtacggca

SEQ ID NO: 241 - DNA, 20 bp, Clostridium hathewayi
tcagcggggacggagtcacc

SEQ ID NO: 242 - DNA, 20 bp, Clostridium hathewayi
aagcggtatctacagaagcg

SEQ ID NO: 243 - DNA, 20 bp, Clostridium hathewayi
gtcccgctggataagatcgt

SEQ ID NO: 244 - DNA, 20 bp, Clostridium hathewayi
cggccagaaacggcgacagc

SEQ ID NO: 245 - DNA, 20 bp, Clostridium hathewayi
tccgtacattacaagtacga

SEQ ID NO: 246 - DNA, 20 bp, Clostridium hathewayi
acatgtgcgtgctggtggac

SEQ ID NO: 247 - DNA, 20 bp, Clostridium hathewayi
cagttaaaggaactgcagag

SEQ ID NO: 248 - DNA, 20 bp, Clostridium hathewayi
gattactggatgccgtttaa